European Patent Application EP 4 385 999 A1, published June 19, 2024. Title: Antibodies. Applicant: ModiQuest B.V. The sequence listing filed with the application follows.

SEQUENCE LISTING (2095 sequences)

SEQ ID NO: 1 - protein, 126 aa, synthetic construct
QVQLVQSGAEVKKPGASVKVSCKASEYTFTDYYMHWVRQAPGRGLEWMGIINPSGGSTTYAPKFQGRVTMTRDTSTSRVYLEMSSLRSEDTAVYYCVRGLGDTGMEPNYYYGMDVWGQGTTVTVSS

SEQ ID NO: 2 - protein, 8 aa, synthetic construct
EYTFTDYY

SEQ ID NO: 3 - protein, 8 aa, synthetic construct
INPSGGST

SEQ ID NO: 4 - protein, 19 aa, synthetic construct
VRGLGDTGMEPNYYYGMDV

SEQ ID NO: 5 - protein, 109 aa, synthetic construct
QTVVTQEPSLTVSPGGTVTLTCASSSGAVTSGDYPNWFQQKPGQAPRALIYRTNNKHSWTPARFSGSLLGGKAALTLSGVQPEDEAEYYCLLYSGGVWVFGGGTKLTVL

SEQ ID NO: 6 - protein, 9 aa, synthetic construct
SGAVTSGDY

SEQ ID NO: 7 - skipped

SEQ ID NO: 8 - protein, 9 aa, synthetic construct
LLYSGGVWV

SEQ ID NO: 9 - protein, 123 aa, synthetic construct
EVQLVESGGGLVQPGRSLRLSCVGSGFTFKEYAMHWVRQVPGKGLEWVSGISWNSGSIGYVDSVKGRFSISRDNAKKSLYLQMNSLRAEDTGLYYCAKDRREDIVVGGWLDPWGQGTLVTVSS

SEQ ID NO: 10 - protein, 8 aa, synthetic construct
GFTFKEYA

SEQ ID NO: 11 - protein, 8 aa, synthetic construct
ISWNSGSI

SEQ ID NO: 12 - protein, 16 aa, synthetic construct
AKDRREDIVVGGWLDP

SEQ ID NO: 13 - protein, 107 aa, synthetic construct
DIQMTQSPSSLSASVGDRVTITCQASQDINKYLNWYQQKPGKAPKLLIYDASNLEPGVPSRFSGTGSGTDFTFTISSLQPEDVATYYCQQYNSFSWTFGQGTKVEIK

SEQ ID NO: 14 - protein, 6 aa, synthetic construct
QDINKY

SEQ ID NO: 15 - skipped

SEQ ID NO: 16 - protein, 9 aa, synthetic construct
QQYNSFSWT

SEQ ID NO: 17 - protein, 123 aa, synthetic construct
EVHLVESGGGLVQPGRSLRLSCAASGFTFDDYAMHWVRQPPGKGLEWVSGINWNSGTIAYADSVKGRFTISRDNAKNSLSLQMNSLRAEDSAFYYCAKERVGELLPGYYFDYWGQGTLVTVSS

SEQ ID NO: 18 - protein, 8 aa, synthetic construct
GFTFDDYA

SEQ ID NO: 19 - protein, 8 aa, synthetic construct
INWNSGTI

SEQ ID NO: 20 - protein, 16 aa, synthetic construct
AKERVGELLPGYYFDY

SEQ ID NO: 21 - protein, 111 aa, synthetic construct
QSVLTQPPSVFGAPGQRVTISCTGSSSNIGAGIDVHWYQQLPGTAPKVLIYGNNKRPSGVPDRFSGSKSGTSASLAITGLQAEDEADYYCQSYDSSLTAWVFGGGTKLTVL

SEQ ID NO: 22 - protein, 9 aa, synthetic construct
SSNIGAGID

SEQ ID NO: 23 - skipped

SEQ ID NO: 24 - protein, 11 aa, synthetic construct
QSYDSSLTAWV

SEQ ID NO: 25 - protein, 123 aa, synthetic construct; identical to SEQ ID NO: 17

SEQ ID NO: 26 - protein, 8 aa, synthetic construct
GFTFDDYA

SEQ ID NO: 27 - protein, 8 aa, synthetic construct
INWNSGTI

SEQ ID NO: 28 - protein, 16 aa, synthetic construct
AKERVGELLPGYYFDY

SEQ ID NO: 29 - protein, 110 aa, synthetic construct
QSALTQPASVSGSPGQPITISCTGTSSDVGSYNLVSWYQQHPGKAPKLMIYEVSERPSGVSSRFSGSKSGNTASLTISGLQAEDEADYYCCSSAGSSNWVFGGGTKLTVL

SEQ ID NO: 30 - protein, 9 aa, synthetic construct
SSDVGSYNL

SEQ ID NO: 31 - skipped

SEQ ID NO: 32 - protein, 10 aa, synthetic construct
CSSAGSSNWV

SEQ ID NO: 33 - protein, 120 aa, synthetic construct
EVQLVESGGGLVQPGGSLRLSCAASGFTFNTYSMNWVRQAPGKGLEWVSYISSGSSTIYYADSVKGRFTISRDNAKNSLYLQMNSLRDEDTAFYYCARGFGLFRSSFDSWGQGTLVTVSS

SEQ ID NO: 34 - protein, 8 aa, synthetic construct
GFTFNTYS

SEQ ID NO: 35 - protein, 8 aa, synthetic construct
ISSGSSTI

SEQ ID NO: 36 - protein, 13 aa, synthetic construct
ARGFGLFRSSFDS

SEQ ID NO: 37 - protein, 111 aa, synthetic construct; identical to SEQ ID NO: 21

SEQ ID NO: 38 - protein, 9 aa, synthetic construct
SSNIGAGID

SEQ ID NO: 39 - skipped

SEQ ID NO: 40 - protein, 11 aa, synthetic construct
QSYDSSLTAWV

SEQ ID NO: 41 - protein, 120 aa, synthetic construct; identical to SEQ ID NO: 33

SEQ ID NO: 42 - protein, 8 aa, synthetic construct
GFTFNTYS

SEQ ID NO: 43 - protein, 8 aa, synthetic construct
ISSGSSTI

SEQ ID NO: 44 - protein, 13 aa, synthetic construct
ARGFGLFRSSFDS

SEQ ID NO: 45 - protein, 110 aa, synthetic construct; identical to SEQ ID NO: 29

SEQ ID NO: 46 - protein, 9 aa, synthetic construct
SSDVGSYNL

SEQ ID NO: 47 - skipped

SEQ ID NO: 48 - protein, 10 aa, synthetic construct
CSSAGSSNWV

SEQ ID NO: 49 - protein, 125 aa, synthetic construct
QVQLLQSGAEVKKPGSSVKVSCKASGGAFSIYAMTWVRQAPGQGFEWMGELIPMLGTPKYAQKFQGRVTITADESTTTAYMDLRSLRSDDTAVYYCAQKMRDCKGDSCHFYFDSWGQGTLVTVSS

SEQ ID NO: 50 - protein, 8 aa, synthetic construct
GGAFSIYA

SEQ ID NO: 51 - protein, 8 aa, synthetic construct
LIPMLGTP

SEQ ID NO: 52 - protein, 18 aa, synthetic construct
AQKMRDCKGDSCHFYFDS

SEQ ID NO: 53 - protein, 107 aa, synthetic construct
DIQMTQSPSSLSASVRDRVTITCRASQNITNYLNWYQQKPGKAPNLLIYAASSLHSGVPSRFSGSGSGSDFTLTISSLQPEDFGYYYCQQTYITPGTFGQGTKVEIK

SEQ ID NO: 54 - protein, 6 aa, synthetic construct
QNITNY

SEQ ID NO: 55 - skipped

SEQ ID NO: 56 - protein, 9 aa, synthetic construct
QQTYITPGT

SEQ ID NO: 57 - protein, 125 aa, synthetic construct; identical to SEQ ID NO: 49

SEQ ID NO: 58 - protein, 8 aa, synthetic construct
GGAFSIYA

SEQ ID NO: 59 - protein, 8 aa, synthetic construct
LIPMLGTP

SEQ ID NO: 60 - protein, 18 aa, synthetic construct
AQKMRDCKGDSCHFYFDS

SEQ ID NO: 61 - protein, 107 aa, synthetic construct
EIVLTQSPGTLSLSPGERATLSCRASQSVSSTYLAWYQQKSGQAPRLLIYGASSRATGIPDRFSGSGSGTDFTLTISRLEPEDFAVYFCQQYGSSSFFGGGTKVEIK

SEQ ID NO: 62 - protein, 7 aa, synthetic construct
QSVSSTY

SEQ ID NO: 63 - skipped

SEQ ID NO: 64 - protein, 8 aa, synthetic construct
QQYGSSSF

SEQ ID NO: 65 - protein, 129 aa, synthetic construct
QVQLVESGGGVVQPGRSLRLSCAASGFTFSNYGMHWVRQAPGKGLEWVAIIWYDGSNKNHADSVKDRFTISRDNSKNTLFLQMNSLRAEDTAVYYCARDPLGYCGGDSCNEHYYGMDVWGQGTTVTVSS

SEQ ID NO: 66 - protein, 8 aa, synthetic construct
GFTFSNYG

SEQ ID NO: 67 - protein, 8 aa, synthetic construct
IWYDGSNK

SEQ ID NO: 68 - protein, 22 aa, synthetic construct
ARDPLGYCGGDSCNEHYYGMDV

SEQ ID NO: 69 - protein, 107 aa, synthetic construct; identical to SEQ ID NO: 53

SEQ ID NO: 70 - protein, 6 aa, synthetic construct
QNITNY

SEQ ID NO: 71 - skipped

SEQ ID NO: 72 - protein, 9 aa, synthetic construct
QQTYITPGT

SEQ ID NO: 73 - protein, 129 aa, synthetic construct; identical to SEQ ID NO: 65

SEQ ID NO: 74 - protein, 8 aa, synthetic construct
GFTFSNYG

SEQ ID NO: 75 - protein, 8 aa, synthetic construct
IWYDGSNK

SEQ ID NO: 76 - protein, 22 aa, synthetic construct
ARDPLGYCGGDSCNEHYYGMDV

SEQ ID NO: 77 - protein, 107 aa, synthetic construct; identical to SEQ ID NO: 61

SEQ ID NO: 78 - protein, 7 aa, synthetic construct
QSVSSTY

SEQ ID NO: 79 - skipped

SEQ ID NO: 80 - protein, 8 aa, synthetic construct
QQYGSSSF

SEQ ID NO: 81 - protein, 127 aa, synthetic construct
QVQLVQSGAEVKKPGASVKVSCKASGYIFTSFDVIWVRQASGQGLEWMGRIRTNNGNTDYAQKFQGRVTMTTDTSTSTVYMELRSLRADDTAVYYCARVTGYFDRRGYYRLENFQYWGQGTTVTVSS

SEQ ID NO: 82 - protein, 8 aa, synthetic construct
GYIFTSFD

SEQ ID NO: 83 - protein, 8 aa, synthetic construct
IRTNNGNT

SEQ ID NO: 84 - protein, 20 aa, synthetic construct
ARVTGYFDRRGYYRLENFQY

SEQ ID NO: 85 - protein, 107 aa, synthetic construct
DIQMTQSPSSLSASVGDRVTITCQASQDISNYLNWYQQKPGKAPRLLISDASSLETGVPSRFSGSGSGTDFTFTISSLQPEDIATYYCQQYDSLALTFGGGTKLEIK

SEQ ID NO: 86 - protein, 6 aa, synthetic construct
QDISNY

SEQ ID NO: 87 - skipped

SEQ ID NO: 88 - protein, 9 aa, synthetic construct
QQYDSLALT

SEQ ID NO: 89 - protein, 123 aa, synthetic construct
QVQLVESGGGVVQPGRSLRLSCAASGFTFSSYAMHWVRQAPGKGLEWVAAILDDGTNKFYADSVKGRFTISRDNSKNTLYLQMNSLRVEDTAMYFCARDSVITMIVVSWPDYWGLGTLVTVSS

SEQ ID NO: 90 - protein, 8 aa, synthetic construct
GFTFSSYA

SEQ ID NO: 91 - protein, 8 aa, synthetic construct
ILDDGTNK

SEQ ID NO: 92 - protein, 16 aa, synthetic construct
ARDSVITMIVVSWPDY

SEQ ID NO: 93 - protein, 108 aa, synthetic construct
DIQMTQSPSSLSASVGDRVTITCRASQSISSYLNWFQQKPGKAPKLLIYAASSLQSGVPSRFSGSGSGTDFTLTISSLQYEDFATYYCQQSYSTPPWTFGQGTKVEIK

SEQ ID NO: 94 - protein, 6 aa, synthetic construct
QSISSY

SEQ ID NO: 95 - skipped

SEQ ID NO: 96 - protein, 10 aa, synthetic construct
QQSYSTPPWT

SEQ ID NO: 97 - protein, 128 aa, synthetic construct
QVQLGESGGGVVQPGRSLRLSCAASGFTFRSYGMHWVRQAPGKGLEWVAVIWYDGSNKYYADSVKGRFTISSDNSNNTLYLQMNTLRAEDTAVYYCARQLFYYDRSGYYRSDAGFDIWGQGTTVTVSS

SEQ ID NO: 98 - protein, 8 aa, synthetic construct
GFTFRSYG

SEQ ID NO: 99 - protein, 8 aa, synthetic construct
IWYDGSNK

SEQ ID NO: 100 - protein, 21 aa, synthetic construct
ARQLFYYDRSGYYRSDAGFDI

SEQ ID NO: 101 - protein, 108 aa, synthetic construct
EIVLTQSPGTLSLSPGERATLSCRASQSVSSSYLAWYQQKPGQAPRLLIDGASSRATGIPDRFSGSGSGTDFTLTISRLEPEDFAVYYCQQYGTSPYTFGQGTKLEIK

SEQ ID NO: 102 - protein, 7 aa, synthetic construct
QSVSSSY

SEQ ID NO: 103 - skipped

SEQ ID NO: 104 - protein, 9 aa, synthetic construct
QQYGTSPYT

SEQ ID NO: 105 - protein, 117 aa, synthetic construct
EVQLVESGGGLVQPGGSLRLSCAASGITVTSNYMNWVRQTPGKGLEWVSVIYPGGSTYYADSVKGRFTISRDNSKNTLNLQMISLRPEDTAIYYCARDRREQQLDDWGPGTLVTVSS

SEQ ID NO: 106 - protein, 8 aa, synthetic construct
GITVTSNY

SEQ ID NO: 107 - protein, 7 aa, synthetic construct
IYPGGST

SEQ ID NO: 108 - protein, 11 aa, synthetic construct
ARDRREQQLDD

SEQ ID NO: 109 - protein, 108 aa, synthetic construct
QSALTQPASVSGSPGQSITISCTGTRSDVGTYNLVSWYQQHPGKAPKLIIYEGNKRPAGVSHRFSGSESGNTASLTISGLQAEDEADYYCCSYAGTRVFGGGTKLTVL

SEQ ID NO: 110 - protein, 9 aa, synthetic construct
RSDVGTYNL

SEQ ID NO: 111 - skipped

SEQ ID NO: 112 - protein, 8 aa, synthetic construct
CSYAGTRV

SEQ ID NO: 113 - protein, 122 aa, synthetic construct
QVQVVQSGAEVKKPGASVKVSCKASGYTFTGYYMHWVRQAPGQGLEWMGWINPNSGATNYAQKFQGRVTMTRDTSISTAYMELSRLRSDDTAVYYCARDSQWSILVGYFQHWGQGTLVTVSS

SEQ ID NO: 114 - protein, 8 aa, synthetic construct
GYTFTGYY

SEQ ID NO: 115 - protein, 8 aa, synthetic construct
INPNSGAT

SEQ ID NO: 116 - protein, 15 aa, synthetic construct
ARDSQWSILVGYFQH

SEQ ID NO: 117 - protein, 110 aa, synthetic construct
QSALTQPPSASGSPGQSVTISCTGTSSDVGGYNYVSWYQQHPGKAPKLMIYEVSKRPSGVPDRFSGSKSGNTASLTVSGLQAEDEADYYCSSDAGSNNLEFGGGTKVTVL

SEQ ID NO: 118 - protein, 9 aa, synthetic construct
SSDVGGYNY

SEQ ID NO: 119 - skipped

SEQ ID NO: 120 - protein, 10 aa, synthetic construct
SSDAGSNNLE

SEQ ID NO: 121 - protein, 123 aa, synthetic construct
EVQLVESGGGLVQPGRSLRLSCAASGFIFDDYAMHWVRQAPGKGPEWVSGVYWNSGTIGYADSVKGQFIISRDNAKNSLYLQMNSLRPEDTALYYCAKDKGYGDPGYYTMDVWGQGTTVTVSS

SEQ ID NO: 122 - protein, 8 aa, synthetic construct
GFIFDDYA

SEQ ID NO: 123 - protein, 8 aa, synthetic construct
VYWNSGTI

SEQ ID NO: 124 - protein, 16 aa, synthetic construct
AKDKGYGDPGYYTMDV

SEQ ID NO: 125 - protein, 111 aa, synthetic construct
NFMLTQPHSVSESPGKTVSISCTRSSGSIASNYVQWYQQRPGSAPTTVIYEDNQRPSGVPDRFSGSIDSSSNSASLTISGLKTEDEADYYCQSYDSSNYVLFGGGTKVTVL

SEQ ID NO: 126 - protein, 8 aa, synthetic construct
SGSIASNY

SEQ ID NO: 127 - skipped

SEQ ID NO: 128 - protein, 10 aa, synthetic construct
QSYDSSNYVL

SEQ ID NO: 129 - protein, 130 aa, synthetic construct
EVQLVESGGGLVQPGRSLRLSCAASGFRFDDYAMHWVRQAPGKGLEWVSGMSWNSGTIGYADSVKGRFTISRDNAKNSLYLQMNRLRAEDTALYYCAKDVAAITMVRGVIREQSYGMDVWGQGTTVTVSS

SEQ ID NO: 130 - protein, 8 aa, synthetic construct
GFRFDDYA

SEQ ID NO: 131 - protein, 8 aa, synthetic construct
MSWNSGTI

SEQ ID NO: 132 - protein, 23 aa, synthetic construct
AKDVAAITMVRGVIREQSYGMDV

SEQ ID NO: 133 - protein, 107 aa, synthetic construct
DIQLTQSPSFLSASVGDRVTLTCRASQGISTYLAWYQQKPGKAPNLLIYGASTLQSGVPSRFSGSGSGTEFTLTISSLQPEDFATYYCQQLNSDPLTFGGGTKVEIK

SEQ ID NO: 134 - protein, 6 aa, synthetic construct
QGISTY

SEQ ID NO: 135 - skipped

SEQ ID NO: 136 - protein, 9 aa, synthetic construct
QQLNSDPLT

SEQ ID NO: 137 - protein, 130 aa, synthetic construct; identical to SEQ ID NO: 129

SEQ ID NO: 138 - protein, 8 aa, synthetic construct
GFRFDDYA

SEQ ID NO: 139 - protein, 8 aa, synthetic construct
MSWNSGTI

SEQ ID NO: 140 - protein, 23 aa, synthetic construct
AKDVAAITMVRGVIREQSYGMDV

SEQ ID NO: 141 - protein, 110 aa, synthetic construct
QSALTQPASVSGSPGQSITISCTGTTSDVGGYNYVSWYQQHPGKAPKLMIYEVSHRPSGVSNRFSGSKSGNTASLTISGLQAEDEADYYCTSYTSDSTVVFGGGTKVTVL

SEQ ID NO: 142 - protein, 9 aa, synthetic construct
TSDVGGYNY

SEQ ID NO: 143 - skipped

SEQ ID NO: 144 - protein, 10 aa, synthetic construct
TSYTSDSTVV

SEQ ID NO: 145 - protein, 124 aa, synthetic construct
QVQLVESGGGVVQPGRSLRLSCAASGFTFSRYGMHWVRQAPGKGLEWVAFISYDGSNKYYADSVKGRFTISRDNSKNTLYLQMNSLRVEDTAVYYCAKNQGSYGSGNYYTFDYWGQGILVTVSS

SEQ ID NO: 146 - protein, 8 aa, synthetic construct
GFTFSRYG

SEQ ID NO: 147 - protein, 8 aa, synthetic construct
ISYDGSNK

SEQ ID NO: 148 - protein, 17 aa, synthetic construct
AKNQGSYGSGNYYTFDY

SEQ ID NO: 149 - protein, 107 aa, synthetic construct; identical to SEQ ID NO: 133

SEQ ID NO: 150 - protein, 6 aa, synthetic construct
QGISTY

SEQ ID NO: 151 - skipped

SEQ ID NO: 152 - protein, 9 aa, synthetic construct
QQLNSDPLT

SEQ ID NO: 153 - protein, 124 aa, synthetic construct; identical to SEQ ID NO: 145

SEQ ID NO: 154 - protein, 8 aa, synthetic construct
GFTFSRYG

SEQ ID NO: 155 - protein, 8 aa, synthetic construct
ISYDGSNK

SEQ ID NO: 156 - protein, 17 aa, synthetic construct
AKNQGSYGSGNYYTFDY

SEQ ID NO: 157 - protein, 110 aa, synthetic construct; identical to SEQ ID NO: 141

SEQ ID NO: 158 - protein, 9 aa, synthetic construct
TSDVGGYNY

SEQ ID NO: 159 - skipped

SEQ ID NO: 160 - protein, 10 aa, synthetic construct
TSYTSDSTVV

SEQ ID NO: 161 - protein, 116 aa, synthetic construct
EVLLVESGGGLVQPGGSLRLSCAASGFAVSSNYMNWVRQAPGKGLEWVSVLYSDGNTDYGDSVKGRFTISRDKSKNTLSLQMNSLRAEDTAVYYCAREVSHAFDLWGQGTTVTVSS

SEQ ID NO: 162 - protein, 8 aa, synthetic construct
GFAVSSNY

SEQ ID NO: 163 - protein, 7 aa, synthetic construct
LYSDGNT

SEQ ID NO: 164 - protein, 10 aa, synthetic construct
AREVSHAFDL

SEQ ID NO: 165 - protein, 108 aa, synthetic construct
EMVMTQSPATLSVSPGERATLSCRASQSVNSNLAWYQQKNGQAPRLLIYGASTRATGIPARFSGSGSGTEFTLTISSLQSEDFAIYYCQQYNNWPTWTFGQGTKVEIK

SEQ ID NO: 166 - protein, 6 aa, synthetic construct
QSVNSN

SEQ ID NO: 167 - skipped

SEQ ID NO: 168 - protein, 10 aa, synthetic construct
QQYNNWPTWT

SEQ ID NO: 169 - protein, 123 aa, synthetic construct
QMQLVQSGPEVKKPGTSVKVSCKASGFTFSSSAVQWVRQARGQRLEWIGWIVVGSGNTNYAQMFQERVTITRDMSTSTAYMELSSLRSEDTAVYYCAAPYCTKTLCDDAFDIWGKGTTVTVSS

SEQ ID NO: 170 - protein, 8 aa, synthetic construct
GFTFSSSA

SEQ ID NO: 171 - protein, 8 aa, synthetic construct
IVVGSGNT

SEQ ID NO: 172 - protein, 16 aa, synthetic construct
AAPYCTKTLCDDAFDI

SEQ ID NO: 173 - protein, 108 aa, synthetic construct
EIVLTQSPGTLSLSPGERATLFCRASQSVSSSYLAWYQQKPGQAPRLLIYGASSRATGTPDRFSGSGSGTDFTLTISRLEPEDFAVYYCQQFGSSPWTFGQGTKVEIK

SEQ ID NO: 174 - protein, 7 aa, synthetic construct
QSVSSSY

SEQ ID NO: 175 - skipped

SEQ ID NO: 176 - protein, 9 aa, synthetic construct
QQFGSSPWT

SEQ ID NO: 177 - protein, 126 aa, synthetic construct
EVQLVESGGGLVKPGGSLRLSCVASGFTLSDAWMSWVRQAPGKGLEWVGRFKSEPDGGTTDYAAPVKGRFTISRDDSRNTLYLQMNSLKTEDTAVYYCTTDAPIYDFWNSYGVDYWGQGTLVTVSS

SEQ ID NO: 178 - protein, 8 aa, synthetic construct
GFTLSDAW

SEQ ID NO: 179 - protein, 10 aa, synthetic construct
FKSEPDGGTT

SEQ ID NO: 180 - protein, 17 aa, synthetic construct
TTDAPIYDFWNSYGVDY

SEQ ID NO: 181 - protein, 115 aa, synthetic construct
DVVMTQSPLSLPVTLGQPASISCRSSQSLVYSDGNTYLSWLQQRPGQSPRRLIYKVSNRDSGVPDRFSGSGSGTYFTLKISRVEAEDVGVYYCMQGSHWWGETITFGQGTRLEIK

SEQ ID NO: 182 - protein, 11 aa, synthetic construct
QSLVYSDGNTY

SEQ ID NO: 183 - skipped

SEQ ID NO: 184 - protein, 12 aa, synthetic construct
MQGSHWWGETIT

SEQ ID NO: 185 - protein, 129 aa, synthetic construct
EVQLLESGGGLVKPGGSLRLSCAASGFTFTNYAMGWVRQAPGKGLEWVSTINDSGGSTYYTESVRGRFTISRDNSKNTLFLQMGSLRAEDTAVYYCAKDDGGSRLPNCGGDCSRAFDYWGQGTLVTVSS

SEQ ID NO: 186 - protein, 8 aa, synthetic construct
GFTFTNYA

SEQ ID NO: 187 - protein, 8 aa, synthetic construct
INDSGGST

SEQ ID NO: 188 - protein, 22 aa, synthetic construct
AKDDGGSRLPNCGGDCSRAFDY

SEQ ID NO: 189 - protein, 108 aa, synthetic construct
DIQMTQSPSSLSASVGDRVTITCQASQDISNYLNWYQQKAGKAPKLLIYDASNLQIGVPSRFSGSGSGTDFTFSISSLQPEDIATYYCQQYDNLPPFTFGGGTKVEIK

SEQ ID NO: 190 - protein, 6 aa, synthetic construct
QDISNY

SEQ ID NO: 191 - skipped

SEQ ID NO: 192 - protein, 10 aa, synthetic construct
QQYDNLPPFT

SEQ ID NO: 193 - protein, 121 aa, synthetic construct
QVQLVESGGGVVQPGRSLRLSCAASGFTFSNSPMHWVRQAPGKGLEWVAVISYDGPNKYYADSVKGRFTISRDNSKNTLNLQMNSLKVEDTAVYYCARETPEQNSYYMDVWGKGTTVTVSS

SEQ ID NO: 194 - protein, 8 aa, synthetic construct
GFTFSNSP

SEQ ID NO: 195 - protein, 8 aa, synthetic construct
ISYDGPNK

SEQ ID NO: 196 - protein, 14 aa, synthetic construct
ARETPEQNSYYMDV

SEQ ID NO: 197 - protein, 110 aa, synthetic construct
QSALTQTASVSGSPGQSITISCTGTSSDVGGYNYVSWYQQHPGKAPKIMVFDVSKRPSGVSNRFSGSKSGNTASLTISGLQAEDDADYYCSSFTSSGTWVFGGGTKVTVL

SEQ ID NO: 198 - protein, 9 aa, synthetic construct
SSDVGGYNY

SEQ ID NO: 199 - skipped

SEQ ID NO: 200 - protein, 10 aa, synthetic construct
SSFTSSGTWV

SEQ ID NO: 201 - protein, 120 aa, synthetic construct
QVQLVESGGGVVQPGRSLRLSCEASGFTFSSYGMHWVRQAPGKGLEWVAVISYDGSNKYYADSVKGRFTISRDNSKNTLYLQMNSLRAEDTAVYYCARDYGDYGGFDYWWGQGTLVTVSS

SEQ ID NO: 202 - protein, 8 aa, synthetic construct
GFTFSSYG

SEQ ID NO: 203 - protein, 8 aa, synthetic construct
ISYDGSNK

SEQ ID NO: 204 - protein, 12 aa, synthetic construct
ARDYGDYGGFDY

SEQ ID NO: 205 - protein, 113 aa, synthetic construct
DIVMTQSPDSLAVSLGERATINCKSSQSVLYSSNNKNYLAWYQQKPGQPPKLLIYWASTRESGVSDRFSGSGSGTDFTLTISSLQAEDVAVYYCQQYYSTPLTFGGGTKVEIK

SEQ ID NO: 206 - protein, 12 aa, synthetic construct
QSVLYSSNNKNY

SEQ ID NO: 207 - skipped

SEQ ID NO: 208 - protein, 9 aa, synthetic construct
QQYYSTPLT

SEQ ID NO: 209 - protein, 122 aa, synthetic construct
EVQLVESGGGLVQPGGSLRLSCAASGFTFSSYEFNWVRQAPGMGLEWLSYISSRGHTIHYAASVKGRFTISRDNAKNSLYLQMNSLKGEDTGVYYCAREEGGAAGGWGLDLWGQGTLVTVSS

SEQ ID NO: 210 - protein, 8 aa, synthetic construct
GFTFSSYE

SEQ ID NO: 211 - protein, 8 aa, synthetic construct
ISSRGHTI

SEQ ID NO: 212 - protein, 15 aa, synthetic construct
AREEGGAAGGWGLDL

SEQ ID NO: 213 - protein, 110 aa, synthetic construct
QSVLTQPPSASGTPGQRVSISCSGSGSNIGSKYVEWYQQVPGTAPKLLICRNNQRPSGVPDRFSGSKSGTSASLAISGLRSEDEAYYYCSSWDDSLSGRVFGGGTKLTVL

SEQ ID NO: 214 - protein, 8 aa, synthetic construct
GSNIGSKY

SEQ ID NO: 215 - skipped

SEQ ID NO: 216 - protein, 11 aa, synthetic construct
SSWDDSLSGRV

SEQ ID NO: 217 - protein, 125 aa, synthetic construct
QVQLVESGGGLVKPGGSLRLSCAASGFTFSDFSMNWIRQAPGRGLEWISYISDSGSTMKYTDSVKGRFTISRDNAKKSLSLQMNSLRDEDTAVYYCARDRSTWERYTTSWCVDSWGQGTLVTVSS

SEQ ID NO: 218 - protein, 8 aa, synthetic construct
GFTFSDFS

SEQ ID NO: 219 - protein, 8 aa, synthetic construct
ISDSGSTM

SEQ ID NO: 220 - protein, 18 aa, synthetic construct
ARDRSTWERYTTSWCVDS

SEQ ID NO: 221 - protein, 110 aa, synthetic construct
QSVLTQPPSVSAAPGQKVTIACSGSSSNIGNNFVTWYQQLPGTAPKLLIYDNNKRPSGIPVRFSGSKSATSASLGITGLQTGDEADYYCVTWDDSLSVVVFGGGTKLTVL

SEQ ID NO: 222 - protein, 8 aa, synthetic construct
SSNIGNNF

SEQ ID NO: 223 - skipped

SEQ ID NO: 224 - protein, 11 aa, synthetic construct
VTWDDSLSVVV

SEQ ID NO: 225 - protein, 126 aa, synthetic construct
QEQLVESGGGLVKPGGSLRLSCAASGFSFRDYYMSWIRQAPGKGLEWISYISSTSGSTIDYADSVKGRFTISRDNAKNSVYLQMNSLRAEDTAVYYCARSRWSDSSGYYVGAFDIWGQGTTVTVSS

SEQ ID NO: 226 - protein, 8 aa, synthetic construct
GFSFRDYY

SEQ ID NO: 227 - protein, 9 aa, synthetic construct
ISSTSGSTI

SEQ ID NO: 228 - protein, 18 aa, synthetic construct
ARSRWSDSSGYYVGAFDI

SEQ ID NO: 229 - protein, 113 aa, synthetic construct
DIVMTQSPDSLAVSLGERATINCKSSQTVLYSSNSKNYLAWYQQKPGQPPKLLIYWASTRESGVPDRFSGSGSGTDFTLTISSLQAEDVAVYYCQQYYSSPPAFGQGTKVEIK

SEQ ID NO: 230 - protein, 12 aa, synthetic construct
QTVLYSSNSKNY

SEQ ID NO: 231 - skipped

SEQ ID NO: 232 - protein, 9 aa, synthetic construct
QQYYSSPPA

SEQ ID NO: 233 - protein, 131 aa, synthetic construct
EVELLESGGGLVQPGGSLRLFCAASGFTFSTAAMSWVRQAPGKGLEWVSVIDKSGGNTYYADSVKGRFTIARDNSKNTLYLQMDSLRAEDTAVYYCAKDRGPRDYDFRSGFIKYYYGMDVWGQGTTVTVSS

SEQ ID NO: 234 - protein, 8 aa, synthetic construct
GFTFSTAA

SEQ ID NO: 235 - protein, 8 aa, synthetic construct
IDKSGGNT

SEQ ID NO: 236 - protein, 24 aa, synthetic construct
AKDRGPRDYDFRSGFIKYYYGMDV

SEQ ID NO: 237 - protein, 107 aa, synthetic construct
GIQMTQSPSSLSASLGDRVTITCQASQDIYNYLNWYQQKPGKAPKLLIHGASNLETGVPSTFSGGGSGTHFTFTINSLQPEDVATYYCQQYENLPLTFGGGTKVEIK

SEQ ID NO: 238 - protein, 6 aa, synthetic construct
QDIYNY

SEQ ID NO: 239 - skipped

SEQ ID NO: 240 - protein, 9 aa, synthetic construct
QQYENLPLT

SEQ ID NO: 241 - protein, 128 aa, synthetic construct
EVQLVESGGSVVRPGGSLRLSCAASGFTFDDYGMSWVRQAPGKGLEWVSGINWIGGSTGYADSVKGRFTISRDNAKNSLYLQMNSLRAEDTALYHCARAYCGGDCYSLLSPRDAFDIWGQGTMVTVSS

SEQ ID NO: 242 - protein, 8 aa, synthetic construct
GFTFDDYG

SEQ ID NO: 243 - protein, 8 aa, synthetic construct
INWIGGST

SEQ ID NO: 244 - protein, 21 aa, synthetic construct
ARAYCGGDCYSLLSPRDAFDI

SEQ ID NO: 245 - protein, 111 aa, synthetic construct
QSVLTQPPSVSGAPGQRVTISCTGSGSNIGAGSDVHWYQHLPGTAPKLLIYGNSNRPSGVPDRFSGSQSGTSASLAITGLQAEDEADYYCQSYDSSLSLVVFGGGTKLTVL

SEQ ID NO: 246 - protein, 9 aa, synthetic construct
GSNIGAGSD

SEQ ID NO: 247 - skipped

SEQ ID NO: 248 - protein, 11 aa, synthetic construct
QSYDSSLSLVV

SEQ ID NO: 249 - protein, 127 aa, synthetic construct
QVQLVQSGAEVKKPGASVKVSCKVSGYPFTELSMHWVRQAPGEGLEWMGSFDPEDGDTMYSQKFQGRLTMTEDTSIDTVYMEMSSLRPEDTAIYYCATGVRFCTNAVCMRWHYFDSWGQGTTVTVSS

SEQ ID NO: 250 - protein, 8 aa, synthetic construct
GYPFTELS

SEQ ID NO: 251 - protein, 8 aa, synthetic construct
FDPEDGDT

SEQ ID NO: 252 - protein, 20 aa, synthetic construct
ATGVRFCTNAVCMRWHYFDS

SEQ ID NO: 253 - protein, 110 aa, synthetic construct
QSVLTQPPSVSAAPGQKVTISCSGSSSNIGRNFVSWYQQLPGTAPRLLIFDNQKRPSGIPDRISGSKSGTSATLGITGLQPGDEADYYCGTWDTSLSAWVFGGGTKLTVL

SEQ ID NO: 254 - protein, 8 aa, synthetic construct
SSNIGRNF

SEQ ID NO: 255 - skipped

SEQ ID NO: 256 - protein, 11 aa, synthetic construct
GTWDTSLSAWV

SEQ ID NO: 257 - protein, 120 aa, synthetic construct
QVQLVQSGAEVKKPGSSVKVSCKASGGTFSDYTFSWVRQAPGQGLEWMGGIIPIFGTPTYAQKVQDRVTITADKSTSTAYMELSSLRSEDTSVYYCARADSGSFGDFDSWGQGTLVTVSS

SEQ ID NO: 258 - protein, 8 aa, synthetic construct
GGTFSDYT

SEQ ID NO: 259 - protein, 8 aa, synthetic construct
IIPIFGTP

SEQ ID NO: 260 - protein, 13 aa, synthetic construct
ARADSGSFGDFDS

SEQ ID NO: 261 - protein, 107 aa, synthetic construct
AIQMTQSPSSLSASVGDRVTITCRASQGIRNDLAWYQQKPGKASKLLIYAASSLQSGVPSRFSGSGSGTDFTLTISSLQPEDFATYYCLQDYLYPLTFGGGTKVEIK

SEQ ID NO: 262 - protein, 6 aa, synthetic construct
QGIRND

SEQ ID NO: 263 - skipped

SEQ ID NO: 264 - protein, 9 aa, synthetic construct
LQDYLYPLT

SEQ ID NO: 265 - protein, 120 aa, synthetic construct; identical to SEQ ID NO: 257

SEQ ID NO: 266 - protein, 8 aa, synthetic construct
GGTFSDYT

SEQ ID NO: 267 - protein, 8 aa, synthetic construct
IIPIFGTP

SEQ ID NO: 268 - protein, 13 aa, synthetic construct
ARADSGSFGDFDS

SEQ ID NO: 269 - protein, 110 aa, synthetic construct
QTVVTQEPSFSVSPGGTITLTCGLSSGSVSTNYYPSWYQQTPGQPPRTLIYNTITRSSGVPDRFSGSIVGNKAALTITGAQADDESDYYCVLYMGNGIWVFGGGTKVTVL

SEQ ID NO: 270 - protein, 9 aa, synthetic construct
SGSVSTNYY

SEQ ID NO: 271 - skipped

SEQ ID NO: 272 - protein, 10 aa, synthetic construct
VLYMGNGIWV

SEQ ID NO: 273 - protein, 124 aa, synthetic construct
EVQLVESGGGLVQPGRSLRLSCAASGFTFDDYAMHWVRQAPGKGLEWVSVIRRNSGSKAYADSVKGRITISRDNAEKTLFLQLNSLRPEDTAVYYCAKSSSFGVDIDLGPFDCWGQGTLVTVSS

SEQ ID NO: 274 - protein, 8 aa, synthetic construct
GFTFDDYA

SEQ ID NO: 275 - protein, 8 aa, synthetic construct
IRRNSGSK

SEQ ID NO: 276 - protein, 17 aa, synthetic construct
AKSSSFGVDIDLGPFDC

SEQ ID NO: 277 - protein, 107 aa, synthetic construct; identical to SEQ ID NO: 261

SEQ ID NO: 278 - protein, 6 aa, synthetic construct
QGIRND

SEQ ID NO: 279 - skipped

SEQ ID NO: 280 - protein, 9 aa, synthetic construct
LQDYLYPLT

SEQ ID NO: 281 - protein, 124 aa, synthetic construct; identical to SEQ ID NO: 273

SEQ ID NO: 282 - protein, 8 aa, synthetic construct
GFTFDDYA

SEQ ID NO: 283 - protein, 8 aa, synthetic construct
IRRNSGSK

SEQ ID NO: 284 - protein, 17 aa, synthetic construct
AKSSSFGVDIDLGPFDC

SEQ ID NO: 285 - protein, 110 aa, synthetic construct; identical to SEQ ID NO: 269

SEQ ID NO: 286 - protein, 9 aa, synthetic construct
SGSVSTNYY

SEQ ID NO: 287 - skipped

SEQ ID NO: 288 - protein, 10 aa, synthetic construct
VLYMGNGIWV

SEQ ID NO: 289 - protein, 123 aa, synthetic construct
QVQLVQSGPEVKKPGTSMKVSCKASGFTFLTSSVQWVRQARGQRLEWIGWIVVGSGNTNYAQKFQERVSITRDVSKSTAYLELSSLRSEDTAVYYCAAPSCNRTTCFDGFNVWGRGTMVTVSS

SEQ ID NO: 290 - protein, 8 aa, synthetic construct
GFTFLTSS

SEQ ID NO: 291 - protein, 8 aa, synthetic construct
IVVGSGNT

SEQ ID NO: 292 - protein, 16 aa, synthetic construct
AAPSCNRTTCFDGFNV

SEQ ID NO: 293 - protein, 106 aa, synthetic construct
DIQMTQSPSSLSASVGDRVTITCRTSQSIGFHLNWYQQKPGKAPNLLIYSASSLQSGVPSRFSGSGSETDFTLTISSLQPEDFATYYCQQSYITPRFGGGTKVEIK

SEQ ID NO: 294 - protein, 6 aa, synthetic construct
QSIGFH

SEQ ID NO: 295 - skipped

SEQ ID NO: 296 - protein, 8 aa, synthetic construct
QQSYITPR

SEQ ID NO: 297 - protein, 129 aa, synthetic construct
QVQLVESGGGVVQPGRSLRLSCAASGFTFSDYGMHWVRQAPGKGLEWLAVIWYDGSNIYSADSVKGRFTISRDNSKNTLFLHLSGLRVEDTAVYYCARDTMYTSTWFWGGSKYHGMDVWGRGTTVTVSS

SEQ ID NO: 298 - protein, 8 aa, synthetic construct
GFTFSDYG

SEQ ID NO: 299 - protein, 8 aa, synthetic construct
IWYDGSNI

SEQ ID NO: 300 - protein, 22 aa, synthetic construct
ARDTMYTSTWFWGGSKYHGMDV

SEQ ID NO: 301 - protein, 107 aa, synthetic construct
DIQMTQSPSTLSASVGDRVTITCRASQSIRTWLAWYQQKPGKAPKLLIYKASNLESGVPSRFSGSGSGTEFTLTISSLQPDDFATYFCQQYDSFSGTFGLGTKVEIK

SEQ ID NO: 302 - protein, 6 aa, synthetic construct
QSIRTW

SEQ ID NO: 303 - skipped

SEQ ID NO: 304 - protein, 9 aa, synthetic construct
QQYDSFSGT

SEQ ID NO: 305 - protein, 122 aa, synthetic construct
QVQLVQSGAEVKKPGSSVKVSCEASGGPFNSYTINWVRQAPGQRLEWMGSIIPILDVADYAQKFQGRVTITADKSTSTAYMELSSLRSEDTAVYYCARPAPYCTSTSCFLNWGQGTLVTVSS

SEQ ID NO: 306 - protein, 8 aa, synthetic construct
GGPFNSYT

SEQ ID NO: 307 - protein, 8 aa, synthetic construct
IIPILDVA

SEQ ID NO: 308 - protein, 15 aa, synthetic construct
ARPAPYCTSTSCFLN

SEQ ID NO: 309 - protein, 111 aa, synthetic construct
QSILTQPPSVSGAPGQRVTISCTGSNSNIGAGYDVHWYQQLPGTAPKLLIYDNTNRPSGVPDRFSGSKSDTSASLAITGLQAEDEADYYCQSYDSSLIHVIFGGGTKLTVL

SEQ ID NO: 310 - protein, 9 aa, synthetic construct
NSNIGAGYD

SEQ ID NO: 311 - skipped

SEQ ID NO: 312 - protein, 11 aa, synthetic construct
QSYDSSLIHVI

SEQ ID NO: 313 - protein, 130 aa, synthetic construct
QVQLVQSGAEVKKPGSSVKVSCMASGGTFSSYAISWVRQAPGQGLEWMGGIIPIFASSAHYAQKFQGRVTITADESTSTAYMEVSSLRSEDTAVYYCARDSSVTTTRGGPSYYYYAMDVWGQGTTVTVSS

SEQ ID NO: 314 - protein, 8 aa, synthetic construct
GGTFSSYA

SEQ ID NO: 315 - protein, 9 aa, synthetic construct
IIPIFASSA

SEQ ID NO: 316 - protein, 22 aa, synthetic construct
ARDSSVTTTRGGPSYYYYAMDV

SEQ ID NO: 317 - protein, 107 aa, synthetic construct
DIQMTQSPSTLSASVGDRVTITCRASQSISSWLAWYQQKPGKVPKLLINKASTLESGVPSRFSGSGSGTEFTLTISSLQPDDIATYYCQHYNMLSITFGQGTRLEIK

SEQ ID NO: 318 - protein, 6 aa, synthetic construct
QSISSW

SEQ ID NO: 319 - skipped

SEQ ID NO: 320 - protein, 9 aa, synthetic construct
QHYNMLSIT

SEQ ID NO: 321 - protein, 123 aa, synthetic construct
QRQLVQSGPEVKKPGTSVKVSCKASGFTFSISAVQWVRQARGQRLEWIGWIAPGSGDTDYAQKVQQRVTITRDTSTDTAYMELSSLRAEDTAVYYCAAPYCTGGVCSDGFDIWGQGTTVTVSS

SEQ ID NO: 322 - protein, 8 aa, synthetic construct
GFTFSISA

SEQ ID NO: 323 - protein, 8 aa, synthetic construct
IAPGSGDT

SEQ ID NO: 324 - protein, 16 aa, synthetic construct
AAPYCTGGVCSDGFDI

SEQ ID NO: 325 - protein, 108 aa, synthetic construct
EIVLTQSPGTLSLSPGERATLSCRASQSVRSSYFAWYQQKPGQAPRLLIYGASSRATGIPDRFSGSGSGTDFTLTISRLEPEDFAVYHCQQFGNSPWTFGQGTKVEIK

SEQ ID NO: 326 - protein, 7 aa, synthetic construct
QSVRSSY

SEQ ID NO: 327 - skipped

SEQ ID NO: 328 - protein, 9 aa, synthetic construct
QQFGNSPWT

SEQ ID NO: 329 - protein, 126 aa, synthetic construct
EVQLVESGGGLVQPGGSLRLSCAASGFTFSSYWMAWVRQAPGKGLEWVANINEDGSEEYYVDSVKGRFTISRDNAKNSLYLQMNSLRAEDTAVYYCARDRHQYYDLWSGYSYFDYWGQGSTVTVSS

SEQ ID NO: 330 - protein, 8 aa, synthetic construct
GFTFSSYW

SEQ ID NO: 331 - protein, 8 aa, synthetic construct
INEDGSEE

SEQ ID NO: 332 - protein, 19 aa, synthetic construct
ARDRHQYYDLWSGYSYFDY

SEQ ID NO: 333 - protein, 113 aa, synthetic construct
DIVMTQSPDSLAVSLGERATINCKSSQSILYSSINKNYLAWYQQKAGQPPKLLIYWASTRESGVPGRFSGSGSGTDFTLTINGLQAEDVAVYYCHQYYSTPQTFGQGTKVEIK

SEQ ID NO: 334 - protein, 12 aa, synthetic construct
QSILYSSINKNY

SEQ ID NO: 335 - skipped

SEQ ID NO: 336 - protein, 9 aa, synthetic construct
HQYYSTPQT

SEQ ID NO: 337 - protein, 121 aa, synthetic construct
QVQLVQSGAEVKKPGSSVKVSCKASGGTFSSTAINWVRQAPGQGLEWMGGIVPIFRTTNYAQKFQGRLTITADESTSTAYMELRSLRSDDTAVYYCARDLEMSTVYGMDVWGQGTTVTVSS

SEQ ID NO: 338 - protein, 8 aa, synthetic construct
GGTFSSTA

SEQ ID NO: 339 - protein, 8 aa, synthetic construct
IVPIFRTT

SEQ ID NO: 340 - protein, 14 aa, synthetic construct
ARDLEMSTVYGMDV

SEQ ID NO: 341 - protein, 109 aa, synthetic construct
DIQLTQSPSFLSASVGDRVTITCRASQGISNYLAWYQQKPGQAPNLLIYAASTLQSGVPSRFSGSGSGTEFTLTISSLQPEDFATYYCQQLNSYPPQITFGGGTKVEIK

SEQ ID NO: 342 - protein, 6 aa, synthetic construct
QGISNY

SEQ ID NO: 343 - skipped

SEQ ID NO: 344 - protein, 11 aa, synthetic construct
QQLNSYPPQIT

SEQ ID NO: 345 - protein, 123 aa, synthetic construct
QVQLVQSGPDVKKPGTSVKVSCKASGFTFITSAVQWVRQARGQRLEWIGWIAVGSGNTEYAQRFQERVTITRDMSTSTVYMELNSLRSEDTAVYYCAAPHCSGGTCRDGFDIWGQGTMVTVSS

SEQ ID NO: 346 - protein, 8 aa, synthetic construct
GFTFITSA

SEQ ID NO: 347 - protein, 8 aa, synthetic construct
IAVGSGNT

SEQ ID NO: 348 - protein, 16 aa, synthetic construct
AAPHCSGGTCRDGFDI

SEQ ID NO: 349 - protein, 110 aa, synthetic construct
QSALTQPASVSGSPGQSITISCTGTSSDVGGYNYVSWYQQHPGKAPKLMTYDVSNRPSGVSNRFSGSKSGNTASLTISGLQAEDETDYYCSSYTSSSTLVFGTGTKVTVL

SEQ ID NO: 350 - protein, 9 aa, synthetic construct
SSDVGGYNY

SEQ ID NO: 351 - skipped

SEQ ID NO: 352 - protein, 10 aa, synthetic construct
SSYTSSSTLV

SEQ ID NO: 353 - protein, 123 aa, synthetic construct; identical to SEQ ID NO: 345

SEQ ID NO: 354 - protein, 8 aa, synthetic construct
GFTFITSA

SEQ ID NO: 355 - protein, 8 aa, synthetic construct
IAVGSGNT

SEQ ID NO: 356 - protein, 16 aa, synthetic construct
AAPHCSGGTCRDGFDI

SEQ ID NO: 357 - protein, 108 aa, synthetic construct
EIVLTQSPGTLSLSPGERATLSCRASQTVRSSFLAWYQKKPGQAPRLLIYVASSRATGIPDRFSGSGSGTDFTLTISRLEPEDFAVYYCQQYGTSPWTFGQGTKLEIK

SEQ ID NO: 358 - protein, 7 aa, synthetic construct
QTVRSSF

SEQ ID NO: 359 - skipped

SEQ ID NO: 360 - protein, 9 aa, synthetic construct
QQYGTSPWT

SEQ ID NO: 361 - protein, 117 aa, synthetic construct
EVQLVESGGDLVQPGGSLRLSCAASGLIVSSNYMNWVRQAPGKGLEWVSVIYSGGSTFYADSVKGRFTISRHDSKNTLYLQMIGLRAEDTAVYFCARDLGPYGMDVWGQGTTVTVSS

SEQ ID NO: 362 - protein, 8 aa, synthetic construct
GLIVSSNY

SEQ ID NO: 363 - protein, 7 aa, synthetic construct
IYSGGST

SEQ ID NO: 364 - protein, 11 aa, synthetic construct
ARDLGPYGMDV

SEQ ID NO: 365 - protein, 110 aa, synthetic construct; identical to SEQ ID NO: 349

SEQ ID NO: 366 - protein, 9 aa, synthetic construct
SSDVGGYNY

SEQ ID NO: 367 - skipped

SEQ ID NO: 368 - protein, 10 aa, synthetic construct
SSYTSSSTLV

SEQ ID NO: 369 - protein, 117 aa, synthetic construct; identical to SEQ ID NO: 361

SEQ ID NO: 370 - protein, 8 aa, synthetic construct
GLIVSSNY

SEQ ID NO: 371 - protein, 7 aa, synthetic construct
IYSGGST

SEQ ID NO: 372 - protein, 11 aa, synthetic construct
ARDLGPYGMDV

SEQ ID NO: 373 - protein, 108 aa, synthetic construct; identical to SEQ ID NO: 357

SEQ ID NO: 374 - protein, 7 aa, synthetic construct
QTVRSSF

SEQ ID NO: 375 - skipped

SEQ ID NO: 376 - protein, 9 aa, synthetic construct
QQYGTSPWT

SEQ ID NO: 377 - protein, 120 aa, synthetic construct
EVQLVETGGGLIQPGGSLRLSCAASGITVSSNYMNWVRQAPGKGLEWVSVIYSGGSTFYADSVRGRFTISRDNSKNTLYLQMNSLRAEDTAVYYCAREGATNAGTAFDIWGRGTTVTVSS

SEQ ID NO: 378 - protein, 8 aa, synthetic construct
GITVSSNY

SEQ ID NO: 379 - protein, 7 aa, synthetic construct
IYSGGST

SEQ ID NO: 380 - protein, 14 aa, synthetic construct
AREGATNAGTAFDI

SEQ ID NO: 381 - protein, 107 aa, synthetic construct
DIQMTQSPSTLSASVGDRVTITCRASQSIVTWLAWYQQKPGKVPKLLINKASSLESGVPSRFSGSGSGTEFTLTISSLQPDDFATYYCQHYNSFSVTFGQGTRLEIK

SEQ ID NO: 382 - protein, 6 aa, synthetic construct
QSIVTW

SEQ ID NO: 383 - skipped

SEQ ID NO: 384 - protein, 9 aa, synthetic construct
QHYNSFSVT

SEQ ID NO: 385 - protein, 127 aa, synthetic construct
EVQLVESGGGLVKPGGSLRLSCAASGFTFSSYSMNWVRQAPGKGLEWVSSISSSSSFIYYADSVKGRLTISRDNAKNSLYLQMNSLRAEDTAVYYCARVPIIAARPEYFYYHYMDVWGKGTTVTVSS

SEQ ID NO: 386 - protein, 8 aa, synthetic construct
GFTFSSYS

SEQ ID NO: 387 - protein, 8 aa, synthetic construct
ISSSSSFI

SEQ ID NO: 388 - protein, 20 aa, synthetic construct
ARVPIIAARPEYFYYHYMDV

SEQ ID NO: 389 - protein, 107 aa, synthetic construct
DIQMTQSPSSLSASVGDRVTITCRASQSMSSYLNWYQQKPGKAPKLLIYAASSLQSGVPSRFSGSGSGTDFTLTISSLQPEDFATYYCQQSYSTPLIFGGGTKLEIK

SEQ ID NO: 390 - protein, 6 aa, synthetic construct
QSMSSY

SEQ ID NO: 391 - skipped

SEQ ID NO: 392 - protein, 9 aa, synthetic construct
QQSYSTPLI

SEQ ID NO: 393 - protein, 122 aa, synthetic construct
EVQLVQSGAEVKKPGESLRISCKGSGYTFTNFWISWVRQMPGKGLEWMGMIDPGDSYTNYSPSFQGHVTFSADKSISTAYLQWSSLKASDTAMYYCARHVGPYRQADAFDFWGQGTTVTVSS

SEQ ID NO: 394 - protein, 8 aa, synthetic construct
GYTFTNFW

SEQ ID NO: 395 - protein, 8 aa, synthetic construct
IDPGDSYT

SEQ ID NO: 396 - protein, 15 aa, synthetic construct
ARHVGPYRQADAFDF

SEQ ID NO: 397 - protein, 107 aa, synthetic construct
DIQMTQSPSTLSASVGDRVTITCRASQSISSWLAWYQQKPGKVPKLLINKASSLESGVPSRFSGSGSGTEFTLTISSLQPDDFATYYCQQYNMFSITFGQGTRLEIK

SEQ ID NO: 398 - protein, 6 aa, synthetic construct
QSISSW

SEQ ID NO: 399 - skipped

SEQ ID NO: 400 - protein, 9 aa, synthetic construct
QQYNMFSIT

SEQ ID NO: 401 - protein, 124 aa, synthetic construct
EVQLVESGGGLVQPGGSLRLSCAASGFTFRNYSMNWVRQAPGKGLEWVSYISSSGSSIYYADSLKGRFTISRDNAKNSLYLQMNSLRAEDTAVYYCVREGWIQLWYRSYYFDYWGQGTLVTVSS

SEQ ID NO: 402 - protein, 8 aa, synthetic construct
GFTFRNYS

SEQ ID NO: 403 - protein, 8 aa, synthetic construct
ISSSGSSI

SEQ ID NO: 404 - protein, 17 aa, synthetic construct
VREGWIQLWYRSYYFDY

SEQ ID NO: 405 - protein, 111 aa, synthetic construct
QSALTQPASVSGSPGQSITISCTGSSSDVGSYNLVSWYQQHPGKAPKLMIYDVSKRPSGVPNRFSGSKSGNTASLTISGLQAEDEADYYCYSYAGSNTFVVFGGGTKLTVL

SEQ ID NO: 406 - protein, 9 aa, synthetic construct
SSDVGSYNL

SEQ ID NO: 407 - skipped

SEQ ID NO: 408 - protein, 11 aa, synthetic construct
YSYAGSNTFVV

SEQ ID NO: 409 - protein, 127 aa, synthetic construct
QVQLVQSGAEVKKPGASVKVSCKASGYMFIRYAMHWVRQAPGQSLEWMGWINPGNGKTIYSQDFQGRVTITRDTSANTVYMELSSLRSKDAAVYYCARFGHYYGSGNYSTWPHFDNWGQGTLVTVSS

SEQ ID NO: 410 - protein, 8 aa, synthetic construct
GYMFIRYA

SEQ ID NO: 411 - protein, 8 aa, synthetic construct
INPGNGKT

SEQ ID NO: 412 - protein, 20 aa, synthetic construct
ARFGHYYGSGNYSTWPHFDN

SEQ ID NO: 413 - protein, 108 aa, synthetic construct
SYVLTQPPSVSVAPGKTARITCGENNIGSKSVHWYQQKPGQAPVLVIYDDSDRPSGIPERFSGSNSGNTATLTISRVEAGDEADYYCQVWDSTRDHPVFGGGTKLTVL

SEQ ID NO: 414 - protein, 6 aa, synthetic construct
NIGSKS

SEQ ID NO: 415 - skipped

SEQ ID NO: 416 - protein, 11 aa, synthetic construct
QVWDSTRDHPV

SEQ ID NO: 417 - protein, 122 aa, synthetic construct
QVQLVQSGTEVKKPGASVKVSCKASGNTFTSYYMHWVRQAPGQGLEWMGIINPGAGSTSYAQKFQGRVTMTSDTSTSTVYMELSSLRSEDAAVYYCARDFGLVPAMLGLDVWGQGTTVTVSS

SEQ ID NO: 418 - protein, 8 aa, synthetic construct
GNTFTSYY

SEQ ID NO: 419 - protein, 8 aa, synthetic construct
INPGAGST

SEQ ID NO: 420 - protein, 15 aa, synthetic construct
ARDFGLVPAMLGLDV

SEQ ID NO: 421 - protein, 109 aa, synthetic construct
EIVLTQSPATLSLSPGERATLSCRASQSVSSYLAWYQQKPGQAPRLLIYDASNRATGIPARFSGSGSGTDFTLTISSLEPEDFAVYYCQQRSNWPRALTFGGGTKVEIK

SEQ ID NO: 422 - protein, 6 aa, synthetic construct
QSVSSY

SEQ ID NO: 423 - skipped

SEQ ID NO: 424 - protein, 11 aa, synthetic construct
QQRSNWPRALT

SEQ ID NO: 425 - protein, 117 aa, synthetic construct
EVQLVESGRDLVHPGGSLRLSCAASGITVSSNYMTWVRQAPGKGLEWVSVLYAGGSSFYTDSVKGRFIISRHNSENTLYLQMNSLRAEDTAVYYCARDLVDYGMDVWGQGTTVTVSS

SEQ ID NO: 426 - protein, 8 aa, synthetic construct
GITVSSNY

SEQ ID NO: 427 - protein, 8 aa, synthetic construct
LYAGGSSF

SEQ ID NO: 428 - protein, 11 aa, synthetic construct
ARDLVDYGMDV

SEQ ID NO: 429 - protein, 107 aa, synthetic construct
DIQMTQSPSSLSASVGDRVTITCRASQDVSSWLAWYQQKPGKAPNSLIYAASSLQSGVPSRFSGSGSGTEFTLTISSLQPEDFATYYCQQYNSYPLTFGGGTKLEIK

SEQ ID NO: 430 - protein, 6 aa, synthetic construct
QDVSSW

SEQ ID NO: 431 - skipped

SEQ ID NO: 432 - protein, 9 aa, synthetic construct
QQYNSYPLT

SEQ ID NO: 433 - protein, 117 aa, synthetic construct; identical to SEQ ID NO: 425

SEQ ID NO: 434 - protein, 8 aa, synthetic construct
GITVSSNY

SEQ ID NO: 435 - protein, 8 aa, synthetic construct
LYAGGSSF

SEQ ID NO: 436 - protein, 11 aa, synthetic construct
ARDLVDYGMDV

SEQ ID NO: 437 - protein, 107 aa, synthetic construct
DTQLTQSPSLLSAFVGDRVTITCRASQGISSYLAWYQQKPGKAPKLLIYGATTLQSGVPSRFSGSGSGTEFTLTISSLQPEDFATYYCQLLNDYPITFGQGTRLEIK

SEQ ID NO: 438 - protein, 6 aa, synthetic construct
QGISSY

SEQ ID NO: 439 - skipped

SEQ ID NO: 440 - protein, 9 aa, synthetic construct
QLLNDYPIT

SEQ ID NO: 441 - protein, 124 aa, synthetic construct
EVQLVESGGSLVHPGRSLRLSCAASGFTFDDYAMHWVRQAPGKGLEWVSGISWNTGSIGYADSVRGRFTISRDNAKNSLYLQMNSLRAEDTALYYCARGGQYYYDRSGNYYDFWGQGTLVTVSS

SEQ ID NO: 442 - protein, 8 aa, synthetic construct
GFTFDDYA

SEQ ID NO: 443 - protein, 8 aa, synthetic construct
ISWNTGSI

SEQ ID NO: 444 - protein, 17 aa, synthetic construct
ARGGQYYYDRSGNYYDF

SEQ ID NO: 445 - protein, 107 aa, synthetic construct; identical to SEQ ID NO: 429

SEQ ID NO: 446 - protein, 6 aa, synthetic construct
QDVSSW

SEQ ID NO: 447 - skipped

SEQ ID NO: 448 - protein, 9 aa, synthetic construct
QQYNSYPLT

SEQ ID NO: 449 - protein, 124 aa, synthetic construct; identical to SEQ ID NO: 441

SEQ ID NO: 450 - protein, 8 aa, synthetic construct
GFTFDDYA

SEQ ID NO: 451 - protein, 8 aa, synthetic construct
ISWNTGSI

SEQ ID NO: 452 - protein, 17 aa, synthetic construct
ARGGQYYYDRSGNYYDF

SEQ ID NO: 453 - protein, 107 aa, synthetic construct; identical to SEQ ID NO: 437

SEQ ID NO: 454 - protein, 6 aa, synthetic construct
QGISSY

SEQ ID NO: 455 - skipped

SEQ ID NO: 456 - protein, 9 aa, synthetic construct
QLLNDYPIT

SEQ ID NO: 457 - protein, 117 aa, synthetic construct
EVYLVESGGGLVQPGGSLRLSCAVSEFTVSSNYMSWVRQAPGKGLEWVSTLYAGGSTFYADSVRGRFTISRDDSRNTLYLQMNSLRAEDTAVYYCARDYGDFYFDYWGQGTLVTVSS

SEQ ID NO: 458 - protein, 8 aa, synthetic construct
EFTVSSNY

SEQ ID NO: 459 - protein, 7 aa, synthetic construct
LYAGGST

SEQ ID NO: 460 - protein, 11 aa, synthetic construct
ARDYGDFYFDY

SEQ ID NO: 461 - protein, 107 aa, synthetic construct
DIQMTQSPSSLSASVGDRVTITCRASQGISNSLAWYQQKPGKAPKLLVYAASKLENGVPSRFSGSGSGTDYTLTINSLQPEDFATYYCQHYYNTPRTFGQGTKVEIK

SEQ ID NO: 462 - protein, 6 aa, synthetic construct
QGISNS

SEQ ID NO: 463 - skipped

SEQ ID NO: 464 - protein, 9 aa, synthetic construct
QHYYNTPRT

SEQ ID NO: 465 - protein, 126 aa, synthetic construct
QVQLVESGGGVVQPGRSLRLSCAASGFSFYTYGMHWVRQAPGKGLEWVAVISSDGGRKNYADSVKGRFTISKDSSKNTLYLQMNSLRTEDTAVYYCAKEEYYGSGSDTPAPKNDYWGQGTLVTVSS

SEQ ID NO: 466 - protein, 8 aa, synthetic construct
GFSFYTYG

SEQ ID NO: 467 - protein, 8 aa, synthetic construct
ISSDGGRK

SEQ ID NO: 468 - protein, 19 aa, synthetic construct
AKEEYYGSGSDTPAPKNDY

SEQ ID NO: 469 - protein, 108 aa, synthetic construct
EIVLTQSPATLSLSPGERATLSCRASQSVSSYLAWYQQKPGQAPRLLIYDASNRATGIPARFSGSGSGTDFTLTISSLEPEDFAVYYCQQRSNWPGYTFGQGTKVEIK

SEQ ID NO: 470 - protein, 6 aa, synthetic construct
QSVSSY

SEQ ID NO: 471 - skipped

SEQ ID NO: 472 - protein, 10 aa, synthetic construct
QQRSNWPGYT

SEQ ID NO: 473 - protein, 126 aa, synthetic construct; identical to SEQ ID NO: 465

SEQ ID NO: 474 - protein, 8 aa, synthetic construct
GFSFYTYG

SEQ ID NO: 475 - protein, 8 aa, synthetic construct
ISSDGGRK

SEQ ID NO: 476 - protein, 19 aa, synthetic construct
AKEEYYGSGSDTPAPKNDY

SEQ ID NO: 477 - protein, 107 aa, synthetic construct
DIQMTQSPSSLSASVGDRVTITCRASQTISNYLNWYQQKPGKAPKLLIFGASSLQSGVPSRFSGSGSGTEFTLTISSLHPEDFATYSCQQSFSTPWTFGQGTKLEIK

SEQ ID NO: 478 - protein, 6 aa, synthetic construct
QTISNY

SEQ ID NO: 479 - skipped

SEQ ID NO: 480 - protein, 9 aa, synthetic construct
QQSFSTPWT

SEQ ID NO: 481 - protein, 122 aa, synthetic construct
EVQLVESGGGLVQPGRSLRLSCAGSGFTFDDYAMHWVRQAPGRGLEWVSGISWNSGIIDYADSVKGRFTISRDNAKNSLYLQMNSLRDEDTALYYCAKGPQRWLQISPFVYWGQGTLVTVSS

SEQ ID NO: 482 - protein, 8 aa, synthetic construct
GFTFDDYA

SEQ ID NO: 483 - protein, 8 aa, synthetic construct
ISWNSGII

SEQ ID NO: 484 - protein, 15 aa, synthetic construct
AKGPQRWLQISPFVY

SEQ ID NO: 485 - protein, 108 aa, synthetic construct; identical to SEQ ID NO: 469

SEQ ID NO: 486 - protein, 6 aa, synthetic construct
QSVSSY

SEQ ID NO: 487 - skipped

SEQ ID NO: 488 - protein, 10 aa, synthetic construct
QQRSNWPGYT

SEQ ID NO: 489 - protein, 122 aa, synthetic construct; identical to SEQ ID NO: 481

SEQ ID NO: 490 - protein, 8 aa, synthetic construct
GFTFDDYA

SEQ ID NO: 491 - protein, 8 aa, synthetic construct
ISWNSGII

SEQ ID NO: 492 - protein, 15 aa, synthetic construct
AKGPQRWLQISPFVY

SEQ ID NO: 493 - protein, 107 aa, synthetic construct; identical to SEQ ID NO: 477

SEQ ID NO: 494 - protein, 6 aa, synthetic construct
QTISNY

SEQ ID NO: 495 - skipped

SEQ ID NO: 496 - protein, 9 aa, synthetic construct
QQSFSTPWT

SEQ ID NO: 497 - protein, 123 aa, synthetic construct
QRPLLQSGPEVKKPGTSVKVSCKASGFTFFTSAVQWVRQARGQRLEWIGWIAVGSGNTDYAQTFQERVTITRDMSTSTAYMELSSLRSEDTAAYYCAAPTCSGGSCYDGFDLWGQGTMVTVSS

SEQ ID NO: 498 - protein, 8 aa, synthetic construct
GFTFFTSA

SEQ ID NO: 499 - protein, 8 aa, synthetic construct
IAVGSGNT

SEQ ID NO: 500 - protein, 16 aa, synthetic construct
AAPTCSGGSCYDGFDL

SEQ ID NO: 501 - protein, 108 aa, synthetic construct
SYELTQPPSVSVSPGQTARITCSGDALPKQHAYWYQQKPGQAPVLVIYKDSERPSGIPERLSGSSSGTTVTLTISGVQAEDEADYYCQSADSSGTLVVFGGGTKVTVL

SEQ ID NO: 502 - protein, 6 aa, synthetic construct
ALPKQH

SEQ ID NO: 503 - skipped

SEQ ID NO: 504 - protein, 11 aa, synthetic construct
QSADSSGTLVV

SEQ ID NO: 505 - protein, 118 aa, synthetic construct
EVLLAETGGGLIQPGGSLRLSCEASGFTVSRNYMSWVRQAPGKGLEWVSVLYSGGSTYYADSVKGRFTISRDNSKNTLYLQMNSLRVEDTAVYYCARGDYYYYYMDVWGKGTTVTVSS

SEQ ID NO: 506 - protein, 8 aa, synthetic construct
GFTVSRNY

SEQ ID NO: 507 - protein, 7 aa, synthetic construct
LYSGGST

SEQ ID NO: 508 - protein, 12 aa, synthetic construct
ARGDYYYYYMDV

SEQ ID NO: 509 - protein, 112 aa, synthetic construct
QSVLTQPPSASGTPGQRVTISCSGSSSNIGSNTVNWYQQLPGTAPKLLIYSNNQRPSGVPDRFSGSKSGTSASLAISGLQSEDEADYSCAAWDDSLNGPNWVFGGGTKLTVL

SEQ ID NO: 510 - protein, 8 aa, synthetic construct
SSNIGSNT

SEQ ID NO: 511 - skipped

SEQ ID NO: 512 - protein, 13 aa, synthetic construct
AAWDDSLNGPNWV

SEQ ID NO: 513 - protein, 125 aa, synthetic construct
EVQLAESGGGLVQPGGSLRLSCAASGFTFSYYWMSWVRQAPGKGLEWVANIKQDGGEKYYVDSVKGRFTISRDNAKNSLYLQMNSLRAEDTAVYYCARGDDIRGYPWSLDAFDIWGQGTMVTVSS

SEQ ID NO: 514 - protein, 8 aa, synthetic construct
GFTFSYYW

SEQ ID NO: 515 - protein, 8 aa, synthetic construct
IKQDGGEK

SEQ ID NO: 516 - protein, 18 aa, synthetic construct
ARGDDIRGYPWSLDAFDI

SEQ ID NO: 517 - protein, 108 aa, synthetic construct
DIQMTQSPSSLSASVGDRVTITCRASQSISRYLSWYQQKPGKAPKLLIHSVSSLQSGVPSRFSGGGSGTHFTLTITSLQREDFATYYCQQSYDTPAPTFGGGTKVEIK

SEQ ID NO: 518 - protein, 6 aa, synthetic construct
QSISRY

SEQ ID NO: 519 - skipped

SEQ ID NO: 520 - protein, 10 aa, synthetic construct
QQSYDTPAPT

SEQ ID NO: 521 - protein, 118 aa, synthetic construct
EVQLVESGGGLVQPGGSLRLSCAASEVIVSSNYMNWVRQAPGKGLEWVSVIYSGGTTYYADSVKGRFTISRDNSKNTLYLQMNSLRVEDTAVYYCARDLDIVGGMDVWGQGTTVTVSS

SEQ ID NO: 522 - protein, 8 aa, synthetic construct
EVIVSSNY

SEQ ID NO: 523 - protein, 7 aa, synthetic construct
IYSGGTT

SEQ ID NO: 524 - protein, 12 aa, synthetic construct
ARDLDIVGGMDV

SEQ ID NO: 525 - protein, 107 aa, synthetic construct
DIQMTQSPSTLSASVGDRVTITCRASQSVNSWLAWYQQKPGKAPKLLVHKASTLESGVPSRFSGSGSGTEFTLTISSLQPDDFATYYCHQYNSNLWTFGQGTKVEIK

SEQ ID NO: 526 - protein, 6 aa, synthetic construct
QSVNSW

SEQ ID NO: 527 - skipped

SEQ ID NO: 528 - protein, 9 aa, synthetic construct
HQYNSNLWT

SEQ ID NO: 529 - protein, 121 aa, synthetic construct
QVRLQESGPGLVKPSETLSLTCTVSGGSIGNHYWSWIRQTPGKGLEWIGYIYYSGSTKYNPSLKSRVTISVDTAKNQFTLKLNSMTAADTAVYYCARGRGVFGVITLFDYWGQGTLVTVSS

SEQ ID NO: 530 - protein, 8 aa, synthetic construct
GGSIGNHY

SEQ ID NO: 531 - protein, 7 aa, synthetic construct
IYYSGST

SEQ ID NO: 532 - protein, 15 aa, synthetic construct
ARGRGVFGVITLFDY

SEQ ID NO: 533 - protein, 108 aa, synthetic construct
EIVLTQSPGTLSLSPGERATLSCRASQSFRSSHLAWYQQIPGQAPRLLIYGASNRATGIPDRFSGSGSGTDFTLTISRLEPEDFAVYYCQQYDKSPWTFGQGTKVEIK

SEQ ID NO: 534 - protein, 7 aa, synthetic construct
QSFRSSH

SEQ ID NO: 535 - skipped

SEQ ID NO: 536 - protein, 9 aa, synthetic construct
QQYDKSPWT

SEQ ID NO: 537 - protein, 124 aa, synthetic construct
QVQLVQSGAEVKKPGSSVKVSCKASGGTFSSYTISWVRQAPGQGLEWMGRIIPILGIANYAQKFQGRVTITADKSTSTAYMELSSLRSEDTAVYYCARDGSYSGSGSNHYFDYWGQGTLVTVSS

SEQ ID NO: 538 - protein, 8 aa, synthetic construct
GGTFSSYT

SEQ ID NO: 539 - protein, 8 aa, synthetic construct
IIPILGIA

SEQ ID NO: 540 - protein, 17 aa, synthetic construct
ARDGSYSGSGSNHYFDY

SEQ ID NO: 541 - protein, 111 aa, synthetic construct
QSVVTQPPSVSGAPGQRVTISCTGSSSNIGAGYDVHWYQHLPGTAPKLLIYVNSNRPSGVPDRFSGSKSGTSASLAITGLQAEDEADYYCQSYDSSLSDSVFGGGTKLTVL

SEQ ID NO: 542 - protein, 9 aa, synthetic construct
SSNIGAGYD

SEQ ID NO: 543 - skipped

SEQ ID NO: 544 - protein, 11 aa, synthetic construct
QSYDSSLSDSV

SEQ ID NO: 545 - protein, 121 aa, synthetic construct
QVQLVQSGAEVKKPGSSVKVSCKASGGTFSSYAINWVRQAPGQGLEWMGGYTPVFGSVNYAQKFQDRVTITADESTSTVYMELSSLRSEDAAVYFCGREVEYSPLYGMNVWGQGTTVTVSS

SEQ ID NO: 546 - protein, 8 aa, synthetic construct
GGTFSSYA

SEQ ID NO: 547 - protein, 8 aa, synthetic construct
YTPVFGSV

SEQ ID NO: 548 - protein, 14 aa, synthetic construct
GREVEYSPLYGMNV

SEQ ID NO: 549 - protein, 108 aa, synthetic construct; identical to SEQ ID NO: 533

SEQ ID NO: 550 - protein, 7 aa, synthetic construct
QSFRSSH

SEQ ID NO: 551 - skipped

SEQ ID NO: 552 - protein, 9 aa, synthetic construct
QQYDKSPWT

SEQ ID NO: 553 - protein, 121 aa, synthetic construct; identical to SEQ ID NO: 545

SEQ ID NO: 554 - protein, 8 aa, synthetic construct
GGTFSSYA

SEQ ID NO: 555 - protein, 8 aa, synthetic construct
YTPVFGSV

SEQ ID NO: 556 - protein, 14 aa, synthetic construct
GREVEYSPLYGMNV

SEQ ID NO: 557 - protein, 108 aa, synthetic construct
SYVLTQPPSVSVAPGQTATVTCGDNNIGSKSVHWYQQKPGQAPILMVFDASDRPSGIPERFSGSNSGNTATLTISRVEAGDEADYYCQVWDSSSDHVLFGGGTKLTVL

SEQ ID NO: 558 - protein, 6 aa, synthetic construct
NIGSKS

SEQ ID NO: 559 - skipped

SEQ ID NO: 560 - protein, 11 aa, synthetic construct
QVWDSSSDHVL

SEQ ID NO: 561 - protein, 120 aa, synthetic construct
QVHLVESGGGVVQPGRSLRLSCAASGFTFSTYAMHWVRQAPGKGLEWVAVILYDGSYKDYADSVKGRFTISRDNSKNTLYLQMNSLRVEDTAVYYCARDWGTTVTTQDYWGQGTLVTVSS

SEQ ID NO: 562 - protein, 8 aa, synthetic construct
GFTFSTYA

SEQ ID NO: 563 - protein, 8 aa, synthetic construct
ILYDGSYK

SEQ ID NO: 564 - protein, 13 aa, synthetic construct
ARDWGTTVTTQDY

SEQ ID NO: 565 - protein, 108 aa, synthetic construct
DIQMTQSPSSLSASVGDRVTITCRASQNINNYLNWFQQKPGNAPKLLIYTTSSLQSGVPSRFSGSGSGTDFTLTISSMQPEDFATYYCQQNYGTPPWTFGQGTKVEIK

SEQ ID NO: 566 - protein, 6 aa, synthetic construct
QNINNY

SEQ ID NO: 567 - skipped

SEQ ID NO: 568 - protein, 10 aa, synthetic construct
QQNYGTPPWT

SEQ ID NO: 569 - protein, 121 aa, synthetic construct
QVTLKESGPVLVKPTETLTLTCAVSGFSLTNAKMGVSWIRQPPGKALEWLAHIFSNDEKSYSTSLKGRLTISKDIFKSQVVLTMTNMDPVDTATYYCARIVWFAEPGLDYWGQGTLVTVSS

SEQ ID NO: 570 - protein, 10 aa, synthetic construct
GFSLTNAKMG

SEQ ID NO: 571 - protein, 7 aa, synthetic construct
IFSNDEK

SEQ ID NO: 572 - protein, 13 aa, synthetic construct
ARIVWFAEPGLDY

SEQ ID NO: 573 - protein, 107 aa, synthetic construct
DIQMTQSPSSLSASVGDRVTITCRASQDIRYNLGWYQQKPGKAPKRLIYAASNLQSGVPSRFSGSGSETEFTLTISSLQPEDFATYYCLHHSTYPWTFGQGTKLEIK

SEQ ID NO: 574 - protein, 6 aa, synthetic construct
QDIRYN

SEQ ID NO: 575 - skipped

SEQ ID NO: 576 - protein, 9 aa, synthetic construct
LHHSTYPWT

SEQ ID NO: 577 - protein, 119 aa, synthetic construct
EVQLVETGGGLIHPGGSLRLSCVASEFIVTANYMSWVRQAPGKGLEWVSIIYPGGSAFYADSVKGRFTISRDNSKNTLYLQMNSLRVEDTAVYYCARVLPTHGDYADYWGQGTLVTVSS

SEQ ID NO: 578 - protein, 8 aa, synthetic construct
EFIVTANY

SEQ ID NO: 579 - protein, 7 aa, synthetic construct
IYPGGSA

SEQ ID NO: 580 - protein, 13 aa, synthetic construct
ARVLPTHGDYADY

SEQ ID NO: 581 - protein, 106 aa, synthetic construct
SYELTQPPSVSVSPGQTASITCSGDNLGDKYACWYQQKPGQSPVLVIYQDTKRPSGIPERFSGSNSGNTATLTISGTQAMDEADYYCQAWDMSSYVFGSGTKVTVL

SEQ ID NO: 582 - protein, 6 aa, synthetic construct
NLGDKY

SEQ ID NO: 583 - skipped

SEQ ID NO: 584 - protein, 9 aa, synthetic construct
QAWDMSSYV

SEQ ID NO: 585 - protein, 123 aa, synthetic construct
QTQLVQSGPEVKKPGTSVKVSCKASGFTFFNSAVQWVRQARGQRLEWIGWIVVGSGNTNYAPKFQESVTITRDMSTSTAYMELSSLRSEDTAVYYCAAPTCSGGTCYDGFNLWGQGTMVTVSS

SEQ ID NO: 586 - protein, 8 aa, synthetic construct
GFTFFNSA

SEQ ID NO: 587 - protein, 8 aa, synthetic construct
IVVGSGNT

SEQ ID NO: 588 - protein, 16 aa, synthetic construct
AAPTCSGGTCYDGFNL

SEQ ID NO: 589 - protein, 108 aa, synthetic construct
EIVLAQSPGTLSLSPGERATLSCRASQSVRSGYFAWYQQKPGQAPRLLIYGASSRATGIPDRFSGSGSGTDFTLTISRLDPEDFAVYFCQQYDASPWTFGQGTKLEIK

SEQ ID NO: 590 - protein, 7 aa, synthetic construct
QSVRSGY

SEQ ID NO: 591 - skipped

SEQ ID NO: 592 - protein, 9 aa, synthetic construct
QQYDASPWT

SEQ ID NO: 593 - protein, 123 aa, synthetic construct
QRPLLQSGPEVKKPGTSVKVSCKASGFTFFTSAVQWVRQARGQRLEWIGWIAVGSGNTDYAQTFQERVTITRDMSTSTAYMELSSLRSEDTAVYYCAAPTCSGGSCYDGFDLWGQGTTVTVSS

SEQ ID NO: 594 - protein, 8 aa, synthetic construct
GFTFFTSA

SEQ ID NO: 595 - protein, 8 aa, synthetic construct
IAVGSGNT

SEQ ID NO: 596 - protein, 16 aa, synthetic construct
AAPTCSGGSCYDGFDL

SEQ ID NO: 597 - protein, 108 aa, synthetic construct; identical to SEQ ID NO: 533

SEQ ID NO: 598 - protein, 7 aa, synthetic construct
QSFRSSH

SEQ ID NO: 599 - skipped

SEQ ID NO: 600 - protein, 9 aa, synthetic construct
QQYDKSPWT

SEQ ID NO: 601 - protein, 123 aa, synthetic construct
QRPLLQSGPEVKKPGTSVKVSCKASGFTFFTSAVQWVRQARGQRLEWIGWIAVGSGNTDYAQTFQERVTITRDMSTSTAYMELSSLRSEDTAVYYCAAPTCSGGSCYDGFDLWGQGTMVTVSS

SEQ ID NO: 602 - protein, 8 aa, synthetic construct
GFTFFTSA

SEQ ID NO: 603 - protein, 8 aa, synthetic construct
IAVGSGNT

SEQ ID NO: 604 - protein, 16 aa, synthetic construct
AAPTCSGGSCYDGFDL

SEQ ID NO: 605 - protein, 107 aa, synthetic construct
DIQMTQSPSSLSASVGDRVTITCRASQDIRYNLGWYQQKPGKAPKRLIYAASNLQSGVPSRFSGSGSETEFTLTISSLQPEDFATYYCLHHSTYPWTFGQGTKVEIK

SEQ ID NO: 606 - protein, 6 aa, synthetic construct
QDIRYN

SEQ ID NO: 607 - skipped

SEQ ID NO: 608 - protein, 9 aa, synthetic construct
LHHSTYPWT

SEQ ID NO: 609 - protein, 122 aa, synthetic construct
QVQLVQSGGEVRKPGASVKVSCKASGYTFTNSGISWVRQAPGQGLEWMGWISVFNGDTNYAQKFQGRVTMTTDTSTNTAYMELRSLRSDDTAVYYCARDRQHLSLFGVLDYWGQGTLVTVSS

SEQ ID NO: 610 - protein, 8 aa, synthetic construct
GYTFTNSG

SEQ ID NO: 611 - protein, 8 aa, synthetic construct
ISVFNGDT

SEQ ID NO: 612 - protein, 15 aa, synthetic construct
ARDRQHLSLFGVLDY

SEQ ID NO: 613 - protein, 107 aa, synthetic construct
DIQMTQSPSSLSASVGDRVTITCRASQSITTFLNWYQQKPGKAPKLLIHAASSLQSGIPSRFSGSGFGTDFTLTISSLQPEDFATYYCQQSFSTPFTFGGGTKVEIK

SEQ ID NO: 614 - protein, 6 aa, synthetic construct
QSITTF

SEQ ID NO: 615 - skipped

SEQ ID NO: 616 - protein, 9 aa, synthetic construct
QQSFSTPFT

SEQ ID NO: 617 - protein, 117 aa, synthetic construct
EVQLVESGGGLVQPGGSLRLSCAASGIIVNRNYMSWVRQAPGKGLEWVSLLYSGGSTFYADSVKGRFTISRDSSKNTLYLDMNTLRTEDTAVYYCVRDLVTYGMDVWGQGTTVTVSS

SEQ ID NO: 618 - protein, 8 aa, synthetic construct
GIIVNRNY

SEQ ID NO: 619 - protein, 7 aa, synthetic construct
LYSGGST

SEQ ID NO: 620 - protein, 11 aa, synthetic construct
VRDLVTYGMDV

SEQ ID NO: 621 - protein, 108 aa, synthetic construct
DIQLTQSPSFLSASVGDRVTITCRASQGISTDLAWYQQKPGKAPKLLIYAASTLQSGVPSRFSGSGSGTEFTLTISSLQPEDFATYYCQQLNSYPPITFGQGTRLEIK

SEQ ID NO: 622 - protein, 6 aa, synthetic construct
QGISTD

SEQ ID NO: 623 - skipped

SEQ ID NO: 624 - protein, 10 aa, synthetic construct
QQLNSYPPIT

SEQ ID NO: 625 - protein, 123 aa, synthetic construct
QMQLVQSGPEVKKPGTSVKVSCKASGFTFSSAAVQWVRQARGQRLEWIGWIVVGSGKTEYAQRFQEKVTISGDMSTSTAYMELSSLRSEDTAVYYCAAPDCNTTSCLDGFDIWGQGTTVTVSS

SEQ ID NO: 626 - protein, 8 aa, synthetic construct
GFTFSSAA

SEQ ID NO: 627 - protein, 8 aa, synthetic construct
IVVGSGKT

SEQ ID NO: 628 - protein, 16 aa, synthetic construct
AAPDCNTTSCLDGFDI

SEQ ID NO: 629 - protein, 108 aa, synthetic construct
EIVLTQSPGTLSLSPGERASLSCRASQSVTRSYLAWYQQKPGQAPRLLIYAASSRATGIPDRFSGSGSGTDFTLTITRLEAEDFAVYHCQQYGSSPWTFGQGTKVEIK

SEQ ID NO: 630 - protein, 7 aa, synthetic construct
QSVTRSY

SEQ ID NO: 631 - skipped

SEQ ID NO: 632 - protein, 9 aa, synthetic construct
QQYGSSPWT

SEQ ID NO: 633 - protein, 123 aa, synthetic construct
EVQLVESGGGLVQPGRSLRLSCVASGFTFDEHAMHWVRQLPGKGLEWVSGASWNSATLGYADSVKGRFIISRDNAKNSLYLQMRSLRPEDTALYYCAKDISRGDPAPEYFHHWGQGTLVTVSS

SEQ ID NO: 634 - protein, 8 aa, synthetic construct
GFTFDEHA

SEQ ID NO: 635 - protein, 8 aa, synthetic construct
ASWNSATL

SEQ ID NO: 636 - protein, 16 aa, synthetic construct
AKDISRGDPAPEYFHH

SEQ ID NO: 637 - protein, 107 aa, synthetic construct
SYELTQPPSVSVSPGQTARITCSGDALPKKYAYWYQQKPGQAPVLVMYKDTQRPSGIPERFSGSNSGTAVTLTISGVQAEDEADYYCQSAGNSSSWVFGGGTKLTVL

SEQ ID NO: 638 - protein, 6 aa, synthetic construct
ALPKKY

SEQ ID NO: 639 - skipped

SEQ ID NO: 640 - protein, 10 aa, synthetic construct
QSAGNSSSWV

SEQ ID NO: 641 - protein, 122 aa, synthetic construct
EVQLVQSGAEVKKPGEFLRISCKGSEYTFDNHWITWVRQMPGKGLEWMGKIDPGDSYTIYSPSFQGHVTISADKSINTAFLQWSSLKASDTAMYYCARHRRWQHQSDAFDVWGQGTMVTVSS

SEQ ID NO: 642 - protein, 8 aa, synthetic construct
EYTFDNHW

SEQ ID NO: 643 - protein, 8 aa, synthetic construct
IDPGDSYT

SEQ ID NO: 644 - protein, 15 aa, synthetic construct
ARHRRWQHQSDAFDV

SEQ ID NO: 645 - protein, 107 aa, synthetic construct
DIQMTQSPSTLSASVGDRVTITCRASQSISSWLAWYQQKPGKAPKLLIYEASSLENGVPSRFSGSGSGTEFTLTISSLQPDDFATYYCQHYSSFSGTFGQGTKLEIK

SEQ ID NO: 646 - protein, 6 aa, synthetic construct
QSISSW

SEQ ID NO: 647 - skipped

SEQ ID NO: 648 - protein, 9 aa, synthetic construct
QHYSSFSGT

SEQ ID NO: 649 - protein, 123 aa, synthetic construct
QRPLLQSGPEVKKPGTSVKVSCKASGFTFFTSAVQWVRQARGQRLEWIGWIAVGSGNTDYAQSFQERVTITRDMSTSTAYMELSSLRSEDTAVYYCAAPTCSGGSCYDGFDLWGQGTMVTVSS

SEQ ID NO: 650 - protein, 8 aa, synthetic construct
GFTFFTSA

SEQ ID NO: 651 - protein, 8 aa, synthetic construct
IAVGSGNT

SEQ ID NO: 652 - protein, 16 aa, synthetic construct
AAPTCSGGSCYDGFDL

SEQ ID NO: 653 - protein, 112 aa, synthetic construct
NFMLTQPHSVSESPGKTVTISCTRSSGSVASNYVQWYQQRPGSAPTTVIYEDNQRPSGVPDRFSGSIDSSSNSASLIISGLKTEDEADYYCQSYDTRNRDVVFGGGTKLTVL

SEQ ID NO: 654 - protein, 8 aa, synthetic construct
SGSVASNY

SEQ ID NO: 655 - skipped

SEQ ID NO: 656 - protein, 11 aa, synthetic construct
QSYDTRNRDVV

SEQ ID NO: 657 - protein, 119 aa, synthetic construct
EVQLVESGGGLVQPGGSLRLSCAASGIIVNRNYMSWVRQAPGKGLEWVSLIYSGGSTFYADSVKGRFTISRHTSENTLYLQMDSLRVEDTAVYFCARSLPLHGDYFDFWGQGTLVTVSS

SEQ ID NO: 658 - protein, 8 aa, synthetic construct
GIIVNRNY

SEQ ID NO: 659 - protein, 7 aa, synthetic construct
IYSGGST

SEQ ID NO: 660 - protein, 13 aa, synthetic construct
ARSLPLHGDYFDF

SEQ ID NO: 661 - protein, 106 aa, synthetic construct
SHELTQPPSVSVSPGQTARITCSGDTFPNQYAYWYQQKPGQAPVLVIYKDSERPSGIPERFSGSSSGTTVTLTISGVQAEDEADYYCQIADSSGVVFGGGTKLTVL

SEQ ID NO: 662 - protein, 6 aa, synthetic construct
TFPNQY

SEQ ID NO: 663 - skipped

SEQ ID NO: 664 - protein, 9 aa, synthetic construct
QIADSSGVV

SEQ ID NO: 665 - protein, 119 aa, synthetic construct
EVQLVESGGGLVQPGGSLRLSCAASEFIVNRNYMSWVRQAPGKGLEWVSLIYPGGSTYYADSVKGRFTISRHSSENTLYLQMNSLRVEDTAVYYCARSLPLYGDYFDFWGQGTLVTVSS

SEQ ID NO: 666 - protein, 8 aa, synthetic construct
EFIVNRNY

SEQ ID NO: 667 - protein, 7 aa, synthetic construct
IYPGGST

SEQ ID NO: 668 - protein, 13 aa, synthetic construct
ARSLPLYGDYFDF

SEQ ID NO: 669 - protein, 108 aa, synthetic construct
DIQMTQSPSSLSASVGDRVTITCRASQSINNYLNWYQHRPGKAPKLLIYAASSLQSGVPSRFSGSGSGTDFTLTISSLQPEDFATYYCQQSYSTPPITFGQGTRLEIK

SEQ ID NO: 670 - protein, 6 aa, synthetic construct
QSINNY

SEQ ID NO: 671 - skipped

SEQ ID NO: 672 - protein, 10 aa, synthetic construct
QQSYSTPPIT

SEQ ID NO: 673 - protein, 131 aa, synthetic construct
EVQLLESGGGLVQPGGSLRLSCAASGFTFSSNAMSWVRQAPGKGLEWVSAISGSGGSTYYADSVKGRCTISRDNSENMLYLQMNSLRAEDTAVYYCAKQGRDYYDRSGYLTLDYDYGMDVWGQGTTVTVSS

SEQ ID NO: 674 - protein, 8 aa, synthetic construct
GFTFSSNA

SEQ ID NO: 675 - protein, 8 aa, synthetic construct
ISGSGGST

SEQ ID NO: 676 - protein, 24 aa, synthetic construct
AKQGRDYYDRSGYLTLDYDYGMDV

SEQ ID NO: 677 - protein, 108 aa, synthetic construct; identical to SEQ ID NO: 669

SEQ ID NO: 678 - protein, 6 aa, synthetic construct
QSINNY

SEQ ID NO: 679 - skipped

SEQ ID NO: 680 - protein, 10 aa, synthetic construct
QQSYSTPPIT

SEQ ID NO: 681 - protein, 127 aa, synthetic construct
QDQLVQSGAEVKKPGSSVRVSCKATAGTFSSYSIHWVRQAPGQGLEWMGRTIPILDITNYAQKFQGRITITADKITTTAYMELTSLTSEDTALYYCARGHPDYGDLLLAGTNWFDPWGQGTLVTVSS

SEQ ID NO: 682 - protein, 8 aa, synthetic construct
AGTFSSYS

SEQ ID NO: 683 - protein, 8 aa, synthetic construct
TIPILDIT

SEQ ID NO: 684 - protein, 20 aa, synthetic construct
ARGHPDYGDLLLAGTNWFDP

SEQ ID NO: 685 - protein, 113 aa, synthetic construct
DIVMTQSPDSLAVSLGERATINCKSSQSVLYSSNNKNYLAWYQQKPGQPPKLLIYWASTRESGVPDRFSGSGSGTDFTLTISSLQAEDVAVYYCQQYSGTPTTFGQGTKVEIK

SEQ ID NO: 686 - protein, 12 aa, synthetic construct
QSVLYSSNNKNY

SEQ ID NO: 687 - skipped

SEQ ID NO: 688 - protein, 9 aa, synthetic construct
QQYSGTPTT

SEQ ID NO: 689 - protein, 125 aa, synthetic construct
EVQLLESGGGLVQPGGSLRLSCAASGFTFSAYAINWVRQAPGKGLEWVSVISGSGTNTYYADSVKGRFTISRDNSKNTLYLQMNSLRAEDTAIYYCAKASYSSSWADYFYYMDVWGKGTTVTVSS

SEQ ID NO: 690 - protein, 8 aa, synthetic construct
GFTFSAYA

SEQ ID NO: 691 - protein, 8 aa, synthetic construct
ISGSGTNT

SEQ ID NO: 692 - protein, 18 aa, synthetic construct
AKASYSSSWADYFYYMDV

SEQ ID NO: 693 - protein, 108 aa, synthetic construct
DIQMTQSPSSLSASVGDRVTITCRTSQSISNYLNWYQQKPGKAPKLLIYAASTLQSGVPSRFSGSGSGTDFTLTISSLQPEDFATYYCQQSYSTPPITFGQGTRLEIK

SEQ ID NO: 694 - protein, 6 aa, synthetic construct
QSISNY

SEQ ID NO: 695 - skipped

SEQ ID NO: 696 - protein, 10 aa, synthetic construct
QQSYSTPPIT

SEQ ID NO: 697 - protein, 119 aa, synthetic construct; identical to SEQ ID NO: 657

SEQ ID NO: 698 - protein, 8 aa, synthetic construct
GIIVNRNY

SEQ ID NO: 699 - protein, 7 aa, synthetic construct
IYSGGST

SEQ ID NO: 700 - protein, 13 aa, synthetic construct
ARSLPLHGDYFDF

SEQ ID NO: 701 - protein, 108 aa, synthetic construct; identical to SEQ ID NO: 669

SEQ ID NO: 702 - protein, 6 aa, synthetic construct
QSINNY

SEQ ID NO: 703 - skipped

SEQ ID NO: 704 - protein, 10 aa, synthetic construct
QQSYSTPPIT

SEQ ID NO: 705 - protein, 129 aa, synthetic construct
EVQLVESGGGVVQPGRSLRLSCAASGFTFSLYGMHWVRQAPGKGLEWVAVMSFDGSKKYYADSVKGRFTISRDNSKNTVYLQMNSLSAEDTAVYYCARPGRDYYDRSGETQLAEDFQHWGQGTLVTVSS

SEQ ID NO: 706 - protein, 8 aa, synthetic construct
GFTFSLYG

SEQ ID NO: 707 - protein, 8 aa, synthetic construct
MSFDGSKK

SEQ ID NO: 708 - protein, 22 aa, synthetic construct
ARPGRDYYDRSGETQLAEDFQH

SEQ ID NO: 709 - protein, 107 aa, synthetic construct
DIQMTQSPSTLSASVGDRVTITCRASQSISRWLAWYQQKPGKAPKLLIYKASSLDSGVPSRFSGSGSGTEFTLTISSLQPDDFATYYCQQYDGYFVTFGQGTKVEIK

SEQ ID NO: 710 - protein, 6 aa, synthetic construct
QSISRW

SEQ ID NO: 711 - skipped

SEQ ID NO: 712 - protein, 9 aa, synthetic construct
QQYDGYFVT

SEQ ID NO: 713 - protein, 119 aa, synthetic construct; identical to SEQ ID NO: 657

SEQ ID NO: 714 - protein, 8 aa, synthetic construct
GIIVNRNY

SEQ ID NO: 715 - protein, 7 aa, synthetic construct
IYSGGST

SEQ ID NO: 716 - protein, 13 aa, synthetic construct
ARSLPLHGDYFDF

SEQ ID NO: 717 - protein, 111 aa, synthetic construct
QSVLTQPPSASGTPGQRVTISCSGSSSNIGSNFVYWYQQLPGTAPKLLIYNNNQRPSGVPDRFSGSKSGTSASLAISGLRSEDEADYYCAAWDDSLSGYAVFGGGTQLTVL

SEQ ID NO: 718 - protein, 8 aa, synthetic construct
SSNIGSNF

SEQ ID NO: 719 - skipped

SEQ ID NO: 720 - protein, 12 aa, synthetic construct
AAWDDSLSGYAV

SEQ ID NO: 721 - protein, 120 aa, synthetic construct
EVQLVESGGGLVQPGGSLRLSCAASGFTFSEYDMHWVRQVTGKGLEWVSTIGTAGDRYYLGSVKGRFTISRENGKNSLYLQMNTLRGGDTAVYYCARGLSNWQTVAFDIWGQGTMVTVSS

SEQ ID NO: 722 - protein, 8 aa, synthetic construct
GFTFSEYD

SEQ ID NO: 723 - protein, 7 aa, synthetic construct
IGTAGDR

SEQ ID NO: 724 - protein, 14 aa, synthetic construct
ARGLSNWQTVAFDI

SEQ ID NO: 725 - protein, 108 aa, synthetic construct
DIQMTQSPSTLSASIGDTVTIACRASENINSWLAWFQQKPGKAPKVLISDASSLESGVPSRFSGSGSGTEFTLTISSLQPDDFATYYCQQYHSYSPITFGQGTRLEIK

SEQ ID NO: 726 - protein, 6 aa, synthetic construct
ENINSW

SEQ ID NO: 727 - skipped

SEQ ID NO: 728 - protein, 10 aa, synthetic construct
QQYHSYSPIT

SEQ ID NO: 729 - protein, 127 aa, synthetic construct
EVQLVESGGGLVKPGGSLRLSCAASGFTFSSYDMHWVRQRTGKGLEWVSTIGTSGDTYYEDSVKGRFTISREDATNSLYLQMNSLRAGDTAVYYCVRGDSITMVRGVTSYYYVMDVWGQGTTVTVSS

SEQ ID NO: 730 - protein, 8 aa, synthetic construct
GFTFSSYD

SEQ ID NO: 731 - protein, 7 aa, synthetic construct
IGTSGDT

SEQ ID NO: 732 - protein, 21 aa, synthetic construct
VRGDSITMVRGVTSYYYVMDV

SEQ ID NO: 733 - protein, 108 aa, synthetic construct
DIQMTQSPSSLSASVGDRVTLTCRASQSISSYLNWYQHKPGKAPKLLIYAASSLQSGVPSRFSGSGSGTEFTLTISSLQPEDFATYYCQESYSNPPWTFGLGTKVEIK

SEQ ID NO: 734 - protein, 6 aa, synthetic construct
QSISSY

SEQ ID NO: 735 - skipped

SEQ ID NO: 736 - protein, 10 aa, synthetic construct
QESYSNPPWT

SEQ ID NO: 737 - protein, 118 aa, synthetic construct
QVQLVQSGAEVKKPGSSVKVSCKASGVTFSMYTISWVRQAPGQGLEWLGRIIPMADTTNYAQKFQGRVTLTADKSTNTASMELRSLRYEDTAVYYCARDSGRDAYNYWGQGTLVTVSS

SEQ ID NO: 738 - protein, 8 aa, synthetic construct
GVTFSMYT

SEQ ID NO: 739 - protein, 8 aa, synthetic construct
IIPMADTT

SEQ ID NO: 740 - protein, 11 aa, synthetic construct
ARDSGRDAYNY

SEQ ID NO: 741 - protein, 108 aa, synthetic construct
DIQMTQSPSTLSASVGDRVTITCRASQNINMWLAWYQQTPGKAPKLLIYDASSLESGVPSRFSGSGSGTDFTLTISSLQPDDFATYYCQQYHSYSPLTFGGGTKVEIK

SEQ ID NO: 742 - protein, 6 aa, synthetic construct
QNINMW

SEQ ID NO: 743 - skipped

SEQ ID NO: 744 - protein, 10 aa, synthetic construct
QQYHSYSPLT

SEQ ID NO: 745 - protein, 129 aa, synthetic construct
EVQLVESGGGSVQPGRSLRLSCAASGFPSGSPFGDHAMHWVRQAPGKGLEWVSSISWNSGNIGYLDSVKGRFTISRDNAKNSLYLQMNILRPEDTAWYYCVKDKNYDSSGYLVNAFDVWGQGTMVTVSS

SEQ ID NO: 746 - protein, 12 aa, synthetic construct
GFPSGSPFGDHA

SEQ ID NO: 747 - protein, 8 aa, synthetic construct
ISWNSGNI

SEQ ID NO: 748 - protein, 18 aa, synthetic construct
VKDKNYDSSGYLVNAFDV

SEQ ID NO: 749 - protein, 107 aa, synthetic construct
DIQMTQSPSSLSASAGDRVTITCRASQNISTYVNWYQQRPGRAPKLLIYTASSLQSGVPSRFSGSGSGTDFTLTIGSLQPRDFATYYCQQSYSDPLTFGGGTKVEIK

SEQ ID NO: 750 - protein, 6 aa, synthetic construct
QNISTY

SEQ ID NO: 751 - skipped

SEQ ID NO: 752 - protein, 9 aa, synthetic construct
QQSYSDPLT

SEQ ID NO: 753 - protein, 123 aa, synthetic construct
EVQLVESGGGLVQPGRSLRLSCAASGFTFDDYAMYWVRQGPGKGLEWVSGISWNSGSIMYADSVKGRFTISRDNAKNSLYLQMNSLRGEDTALYYCAKGLGSKHQYYYGMDVWGQGTTVTVSS

SEQ ID NO: 754 - protein, 8 aa, synthetic construct
GFTFDDYA

SEQ ID NO: 755 - protein, 8 aa, synthetic construct
ISWNSGSI

SEQ ID NO: 756 - protein, 16 aa, synthetic construct
AKGLGSKHQYYYGMDV

SEQ ID NO: 757 - protein, 107 aa, synthetic construct
ATQLTQSPSSLSASVGDGVTITCRASQGISNALAWYQQRPGRGPNLLISNASNLKSGVPSRFSGSGSGTDFTLTINSLQPEDFATYYCQQFNSYPWTFGQGTKVEIK

SEQ ID NO: 758 - protein, 6 aa, synthetic construct
QGISNA

SEQ ID NO: 759 - skipped

SEQ ID NO: 760 - protein, 9 aa, synthetic construct
QQFNSYPWT

SEQ ID NO: 761 - protein, 123 aa, synthetic construct
QVQLVESGGGVVQPGRSLRLSCAASGFTFSSFDFHWVRQAPGKGLEWVALISYDGIGKFYADSVEGRFTISRDNSKNTVYLQMSSLRGEDTAVYHCARDSLSSLSTTVVLEYWGQGSLVTVSS

SEQ ID NO: 762 - protein, 8 aa, synthetic construct
GFTFSSFD

SEQ ID NO: 763 - protein, 8 aa, synthetic construct
ISYDGIGK

SEQ ID NO: 764 - protein, 16 aa, synthetic construct
ARDSLSSLSTTVVLEY

SEQ ID NO: 765 - protein, 108 aa, synthetic construct
DIQMTQSPSSLSASVGDRVTITCRASQSIGRYLNWYQHKPGKAPNLLIYAASNLQSGVPSRFSGSGSGTDFTLTISSLQPEDFATYFCQQSYSTPSITFGQGTRLEIK

SEQ ID NO: 766 - protein, 6 aa, synthetic construct
QSIGRY

SEQ ID NO: 767 - skipped

SEQ ID NO: 768 - protein, 10 aa, synthetic construct
QQSYSTPSIT

SEQ ID NO: 769 - protein, 124 aa, synthetic construct
EVQLVQSGSEVKKPGESLRISCKGSGYPFSTFWIGWVRQMPGKGLEWMGVIYPGDSETKYSPSFQGQVSFSADKSISTAYLQWSSLEASDTAMYYCARLPITGSFTEYFGLDVWGQGTTVTVSS

SEQ ID NO: 770 - protein, 8 aa, synthetic construct
GYPFSTFW

SEQ ID NO: 771 - protein, 8 aa, synthetic construct
IYPGDSET

SEQ ID NO: 772 - protein, 17 aa, synthetic construct
ARLPITGSFTEYFGLDV

SEQ ID NO: 773 - protein, 108 aa, synthetic construct
EIVLTQSPGTLSLSPGERASLSCRASQSVSTYYLAWYQQKAGQAPRLLIYGASSRATGIPDRFSGSGSGTDFTLTINRLEPEDFAVYYCQQYGSSPWTFGQGTKVEIK

SEQ ID NO: 774 - protein, 7 aa, synthetic construct
QSVSTYY

SEQ ID NO: 775 - skipped

SEQ ID NO: 776 - protein, 9 aa, synthetic construct
QQYGSSPWT

SEQ ID NO: 777 - protein, 118 aa, synthetic construct
EVQLVESGGGLVQPGGSLRLSCAASGITVTSNYMNWVRQAPGRGLEWVSVIYSGGTTNYADSVKGRFTISRHDSKNTLYLQMNSLRIEDTAVYYCARGDPYYYGMDVWGQGTTVTVSS

SEQ ID NO: 778 - protein, 8 aa, synthetic construct
GITVTSNY

SEQ ID NO: 779 - protein, 7 aa, synthetic construct
IYSGGTT

SEQ ID NO: 780 - protein, 12 aa, synthetic construct
ARGDPYYYGMDV

SEQ ID NO: 781 - protein, 106 aa, synthetic construct
DIQLTQSPSFLSASVGDRVTITCRPSQGIGSYLAWYQQKPGKAPKLLIYGGSTLQSGVPSRFSGSGSGTEFTLTISSLQPEDFATYFCQQLDTYPSFGGGTKVEIK

SEQ ID NO: 782 - protein, 6 aa, synthetic construct
QGIGSY

SEQ ID NO: 783 - skipped

SEQ ID NO: 784 - protein, 8 aa, synthetic construct
QQLDTYPS

SEQ ID NO: 785 - protein, 122 aa, synthetic construct
QVQLVESGGGVVQPGRSLRLSCAASGFAFSSFDMHWVRQAPGKGLEWVAVILFDGTNKYYADSVKGRFTLSRDNSKNTLYLQMNSLRAEDTAFYYCARSDYYGAGTGYFQHWGQGTLVTVSS

SEQ ID NO: 786 - protein, 8 aa, synthetic construct
GFAFSSFD

SEQ ID NO: 787 - protein, 8 aa, synthetic construct
ILFDGTNK

SEQ ID NO: 788 - protein, 15 aa, synthetic construct
ARSDYYGAGTGYFQH

SEQ ID NO: 789 - protein, 113 aa, synthetic construct
DIVMTQTPLSLPVTPGEPASISCRSSQNLLDSDEGNIYLDWYLQKPGQSPQLLIYTLSYRASGVPDRFSGSGSGTDFTLKISRVEAEDVGVYYCMQRIEFPYSFGQGTKLEIK

SEQ ID NO: 790 - protein, 12 aa, synthetic construct
QNLLDSDEGNIY

SEQ ID NO: 791 - skipped

SEQ ID NO: 792 - protein, 9 aa, synthetic construct
MQRIEFPYS

SEQ ID NO: 793 - protein, 117 aa, synthetic construct
EVQLVESGGHLVQPGGSLRLSCAASGLTVSSNYMNWVRQAPGKGLEWVSVLYAGGSTFYADSVKGRFTISRHNSNNTLYLQMNSLRAEDTAVYYCARDLVSYGMDVWGQGTTVTVSS

SEQ ID NO: 794 - protein, 8 aa, synthetic construct
GLTVSSNY

SEQ ID NO: 795 - protein, 7 aa, synthetic construct
LYAGGST

SEQ ID NO: 796 - protein, 11 aa, synthetic construct
ARDLVSYGMDV

SEQ ID NO: 797 - protein, 106 aa, synthetic construct
DIQLTQSPSFLSASIGDRVTITCRASQGISRSLAWYQQKPGKAPKLLIYAASTLQSGVPSRFSGSGSGTEFTLTISSLQPEDFATYYCQQLDSFPKFGQGTRLEIK

SEQ ID NO: 798 - protein, 6 aa, synthetic construct
QGISRS

SEQ ID NO: 799 - skipped

SEQ ID NO: 800 - protein, 8 aa, synthetic construct
QQLDSFPK

SEQ ID NO: 801 - protein, 117 aa, synthetic construct; identical to SEQ ID NO: 793

SEQ ID NO: 802 - protein, 8 aa, synthetic construct
GLTVSSNY

SEQ ID NO: 803 - protein, 7 aa, synthetic construct
LYAGGST

SEQ ID NO: 804 - protein, 11 aa, synthetic construct
ARDLVSYGMDV

SEQ ID NO: 805 - protein, 110 aa, synthetic construct
QSALTQPPSASGSPGQSVTISCTGTSSDVGGYNYVSWYQQFPGKAPKLMIYEVIKRPSGVPDRFSGSKSGNTASLTVSGLQAEDEADYYCGSYAGSNNWVFGGGTKLTVL

SEQ ID NO: 806 - protein, 9 aa, synthetic construct
SSDVGGYNY

SEQ ID NO: 807 - skipped

SEQ ID NO: 808 - protein, 10 aa, synthetic construct
GSYAGSNNWV

SEQ ID NO: 809 - protein, 117 aa, synthetic construct
EVQLVESGGGLVQPGGSLRLSCAASGVIVNRNYMNWVRQAPGKGLEWVSLLYAGGTTFYADSVKGRFTVSRDNSKNTLYLQMNSLRPEDTAVYYCARDLVVYGMDVWGQGTTVTVSS

SEQ ID NO: 810 - protein, 8 aa, synthetic construct
GVIVNRNY

SEQ ID NO: 811 - protein, 7 aa, synthetic construct
LYAGGTT

SEQ ID NO: 812 - protein, 11 aa, synthetic construct
ARDLVVYGMDV

SEQ ID NO: 813 - protein, 106 aa, synthetic construct
DIQLTQSPSFLSASVGDRVTITCRASQGISSDLAWYQQKPGKAPKLLIYAASTLQSGVPSRFTGSGSGTEFTLTISSLQPEDFATYYCQQLNNYYLFGGGTKVEIK

SEQ ID NO: 814 - protein, 6 aa, synthetic construct
QGISSD

SEQ ID NO: 815 - skipped

SEQ ID NO: 816 - protein, 8 aa, synthetic construct
QQLNNYYL

SEQ ID NO: 817 - protein, 121 aa, synthetic construct
EVQLVESGGGLVQPGGSLRLSCAASGFNLSRSDMHWVRQVIGKGLEWVSFIGSAGDTYYAGSVKGRFTISRENAKNSLYLQMNSLRAGDTALYYCARMRYDGYDFYGLDVWGQGTTVTVSS

SEQ ID NO: 818 - protein, 8 aa, synthetic construct
GFNLSRSD

SEQ ID NO: 819 - protein, 7 aa, synthetic construct
IGSAGDT

SEQ ID NO: 820 - protein, 15 aa, synthetic construct
ARMRYDGYDFYGLDV

SEQ ID NO: 821 - protein, 107 aa, synthetic construct
DIQMTQSPSSLSASVGDRVTITCQASQDIMKYLNWYQQKPGKAPNLLIYDASNLETGVPSRFSGSGSGTDFTLTISSLQPEDIATYYCLQYDNLPLTFGGGTKVEIK

SEQ ID NO: 822 - protein, 6 aa, synthetic construct
QDIMKY

SEQ ID NO: 823 - skipped

SEQ ID NO: 824 - protein, 9 aa, synthetic construct
LQYDNLPLT

SEQ ID NO: 825 - protein, 121 aa, synthetic construct
QVQLAQAGAEVKKPGASVKVSCKASGYTFTTYYIHWVRQAPGQGLEWMGIINPSGGSTSYALKFQGRVTVTSDTSTSTVYMELSSLTSEDTAVYYCAREVVVPAAGYMDVWGKGTTVTVSS

SEQ ID NO: 826 - protein, 8 aa, synthetic construct
GYTFTTYY

SEQ ID NO: 827 - protein, 8 aa, synthetic construct
INPSGGST

SEQ ID NO: 828 - protein, 14 aa, synthetic construct
AREVVVPAAGYMDV

SEQ ID NO: 829 - protein, 107 aa, synthetic construct; identical to SEQ ID NO: 821

SEQ ID NO: 830 - protein, 6 aa, synthetic construct
QDIMKY

SEQ ID NO: 831 - skipped

SEQ ID NO: 832 - protein, 9 aa, synthetic construct
LQYDNLPLT

SEQ ID NO: 833 - protein, 121 aa, synthetic construct; identical to SEQ ID NO: 825

SEQ ID NO: 834 - protein, 8 aa, synthetic construct
GYTFTTYY

SEQ ID NO: 835 - protein, 8 aa, synthetic construct
INPSGGST

SEQ ID NO: 836 - protein, 14 aa, synthetic construct
AREVVVPAAGYMDV

SEQ ID NO: 837 - protein, 108 aa, synthetic construct
SYVLTQAPSVSVAPGRTARITCGADDIGSKSVHWYQQKPGQAPVLVVYDDSVRPSGIPERFSGSNSGSTATLTISRVDSGDEADYYCQVWNSGRDHYVFGSGTKVTVL

SEQ ID NO: 838 - protein, 6 aa, synthetic construct
DIGSKS

SEQ ID NO: 839 - skipped

SEQ ID NO: 840 - protein, 11 aa, synthetic construct
QVWNSGRDHYV

SEQ ID NO: 841 - protein, 117 aa, synthetic construct; identical to SEQ ID NO: 793

SEQ ID NO: 842 - protein, 8 aa, synthetic construct
GLTVSSNY

SEQ ID NO: 843 - protein, 7 aa, synthetic construct
LYAGGST

SEQ ID NO: 844 - protein, 11 aa, synthetic construct
ARDLVSYGMDV

SEQ ID NO: 845 - protein, 107 aa, synthetic construct; identical to SEQ ID NO: 821

SEQ ID NO: 846 - protein, 6 aa, synthetic construct
QDIMKY

SEQ ID NO: 847 - skipped

SEQ ID NO: 848 - protein, 9 aa, synthetic construct
LQYDNLPLT

SEQ ID NO: 849 - protein, 118 aa, synthetic construct
QVQLQESGPGLVKPSATLSLTCTVSGGSINSYYWSWIRQPPGKGLEWIGYIYYSGSTNYNPSLKSRVTISVDTSKNQFSLKLRSVTAADTAMYYCARVEGLGQHIDYWGQGTLVTVSS

SEQ ID NO: 850 - protein, 8 aa, synthetic construct
GGSINSYY

SEQ ID NO: 851 - protein, 7 aa, synthetic construct
IYYSGST

SEQ ID NO: 852 - protein, 12 aa, synthetic construct
ARVEGLGQHIDY

SEQ ID NO: 853 - protein, 107 aa, synthetic construct
DIQLTQSPSSLSASVGDRVTITCQASQHIANYLNWYQQKSGKAPKLLIYDGANLEAGVPSRFSGSGSGPDFTLIISSLQPEDIATYYCQQYDSLPLTFGQGTRLEIK

SEQ ID NO: 854 - protein, 6 aa, synthetic construct
QHIANY

SEQ ID NO: 855 - skipped

SEQ ID NO: 856 - protein, 9 aa, synthetic construct
QQYDSLPLT

SEQ ID NO: 857 - protein, 124 aa, synthetic construct
QVQLVQSGAEVKKPGSSVKVSCKASGGTFSSYTVNWVRQAPGQGLEWMGRIIPILGRASYAQKFQGRVTITADKSTSTAYMELSSLTSEDTAVYYCARMGDGGNSDYYYGMDVWGQGTTVTVSS

SEQ ID NO: 858 - protein, 8 aa, synthetic construct
GGTFSSYT

SEQ ID NO: 859 - protein, 8 aa, synthetic construct
IIPILGRA

SEQ ID NO: 860 - protein, 17 aa, synthetic construct
ARMGDGGNSDYYYGMDV

SEQ ID NO: 861 - protein, 107 aa, synthetic construct
DIQMTQSPSSLSASVGDRVTITCRASQDITNYLVWYQQKPGKVPKVLIYAASTLQSGVPSRFSGSGSGTDFTLTINSLQPEDVATYYCQKYNNALLTFGGGTKVEIK

SEQ ID NO: 862 - protein, 6 aa, synthetic construct
QDITNY

SEQ ID NO: 863 - skipped

SEQ ID NO: 864 - protein, 9 aa, synthetic construct
QKYNNALLT

SEQ ID NO: 865 - protein, 125 aa, synthetic construct
QVQLVESGGGVVQPGRSLRLSCAADGFIFSVYGMHWVRQAPGKGLEWLAVISSDGRNKYYADSVKGRFTISRDNSKNTLYLQMNSLRADDTAVYYCSNPWQLGRSSTNTDVFDIWGQGTMVTVSS

SEQ ID NO: 866 - protein, 8 aa, synthetic construct
GFIFSVYG

SEQ ID NO: 867 - protein, 8 aa, synthetic construct
ISSDGRNK

SEQ ID NO: 868 - protein, 18 aa, synthetic construct
SNPWQLGRSSTNTDVFDI

SEQ ID NO: 869 - protein, 108 aa, synthetic construct
SYVLTQPPSVSVAPGKTARITCGGNNIGSKTVHWCRQKPGQAPVLVVYDDDDRPSGIPERFSGSNSGSTATLTISRVEAGDEADYFCQVWESSGDHVVFGGGTKLTVL

SEQ ID NO: 870 - protein, 6 aa, synthetic construct
NIGSKT

SEQ ID NO: 871 - skipped

SEQ ID NO: 872 - protein, 11 aa, synthetic construct
QVWESSGDHVV

SEQ ID NO: 873 - protein, 128 aa, synthetic construct
QVQLVESGGGVVQPGGSLRLSCAASGFTFSDYGMHWIRQAPGKGLEWVAIMWLDGIENYYADSVKGRFTVSRDNSSNTLYLQINSLRPEDTAVYYCARTRQDYDDRIVYFYPYGMDVWGQGTTVTVSS

SEQ ID NO: 874 - protein, 8 aa, synthetic construct
GFTFSDYG

SEQ ID NO: 875 - protein, 8 aa, synthetic construct
MWLDGIEN

SEQ ID NO: 876 - protein, 21 aa, synthetic construct
ARTRQDYDDRIVYFYPYGMDV

SEQ ID NO: 877 - protein, 107 aa, synthetic construct
DIQMTQSPSSLSASVGDRVTLTCRASQTIHSYLNWYQQRPGKAPELLIYAASSLQSGVPSRFSGSGSATDFTLTISSLQPEDFATYYCQQSFVTPPTFGQGTKLEIK

SEQ ID NO: 878 - protein, 6 aa, synthetic construct
QTIHSY

SEQ ID NO: 879 - skipped

SEQ ID NO: 880 - protein, 9 aa, synthetic construct
QQSFVTPPT

SEQ ID NO: 881 - protein, 126 aa, synthetic construct
QVQLQESGPGLVKPSGTLSLTCSVSGGSVSSDSHYWSWIRQPPGKGLEWLGYIYYTGNTNYNPSLKSRVTIAVDTSKNHFSLRLTSVTAADTAVYFCAREPLFTVTLVARGAFDIWGQGTMVTVSS

SEQ ID NO: 882 - protein, 10 aa, synthetic construct
GGSVSSDSHY

SEQ ID NO: 883 - protein, 7 aa, synthetic construct
IYYTGNT

SEQ ID NO: 884 - protein, 18 aa, synthetic construct
AREPLFTVTLVARGAFDI

SEQ ID NO: 885 - protein, 110 aa, synthetic construct
QSALTQPASVSGSPGQSITISCTGSSSDVGGYNYLSWYQQHPGKAPKLMIYDVTNRPSGISNRFSGSKSGNTASLTISGLQAEDEADYYCSSYTSSNSKLFGGGTKLTVL

SEQ ID NO: 886 - protein, 9 aa, synthetic construct
SSDVGGYNY

SEQ ID NO: 887 - skipped

SEQ ID NO: 888 - protein, 10 aa, synthetic construct
SSYTSSNSKL

SEQ ID NO: 889 - protein, 124 aa, synthetic construct
QVQLVQSGAEVKKSGSSVKVSCKASGGTFSSYAISWVRQAPGQGLEWMGGIFAMFGRATYAQKFQGRVTITADRSTSTAYMELNSLRSEDTAVYYCARTSDQFYSNYAYGMDVWGKGTTVTVSS

SEQ ID NO: 890 - protein, 8 aa, synthetic construct
GGTFSSYA

SEQ ID NO: 891 - protein, 8 aa, synthetic construct
IFAMFGRA

SEQ ID NO: 892 - protein, 17 aa, synthetic construct
ARTSDQFYSNYAYGMDV

SEQ ID NO: 893 - protein, 108 aa, synthetic construct
EIVMTQSPATLSVSPGERVTLSCRASQSVSTNLAWYQQKPGQAPRLLIYGASTRATGIPARFSGSGSGTEFTFTIGSLQSEDFAVYYCQQYNYWPPVTFGQGTKVEIK

SEQ ID NO: 894 - protein, 6 aa, synthetic construct
QSVSTN

SEQ ID NO: 895 - skipped

SEQ ID NO: 896 - protein, 10 aa, synthetic construct
QQYNYWPPVT

SEQ ID NO: 897 - protein, 125 aa, synthetic construct
EVQLVESGGGLVQPGRSLRLSCTASGFTFDDYTMNWVRQAPGKGLEWVSSISWNSGSIDYADSVKGRFTISRDNAKNSLYLQMNSLRAEDTALYYCTKSAYPGISAHHYYGLAVWGQGTTVTVSS

SEQ ID NO: 898 - protein, 8 aa, synthetic construct
GFTFDDYT

SEQ ID NO: 899 - protein, 8 aa, synthetic construct
ISWNSGSI

SEQ ID NO: 900 - protein, 18 aa, synthetic construct
TKSAYPGISAHHYYGLAV

SEQ ID NO: 901 - protein, 113 aa, synthetic construct
DIVMTQSPDSLAVSLGERATINCKSSQSVFYSSSNKNNIAWYQQKPGQPPKLLIYWASTRESGVPDRFSGSGSGTDFTLTISSLQAEDVAVYHCQQYLTTPLTFGGGTKVEIK

SEQ ID NO: 902 - protein, 12 aa, synthetic construct
QSVFYSSSNKNN

SEQ ID NO: 903 - skipped

SEQ ID NO: 904 - protein, 9 aa, synthetic construct
QQYLTTPLT

SEQ ID NO: 905 - protein, 125 aa, synthetic construct; identical to SEQ ID NO: 897

SEQ ID NO: 906 - protein, 8 aa, synthetic construct
GFTFDDYT

SEQ ID NO: 907 - protein, 8 aa, synthetic construct
ISWNSGSI

SEQ ID NO: 908 - protein, 18 aa, synthetic construct
TKSAYPGISAHHYYGLAV

SEQ ID NO: 909 - protein, 110 aa, synthetic construct
QSALTQPPSASGSLGQSVTISCTGTSSDVGGYNYVSWYRQHPGKAPKLMIYEVSERPSGVPDRFSGSKSGNTASLTVSGLQAEDEADYYCSSYAGSNNLVFGGGTKLTVL

SEQ ID NO: 910 - protein, 9 aa, synthetic construct
SSDVGGYNY

SEQ ID NO: 911 - skipped

SEQ ID NO: 912 - protein, 10 aa, synthetic construct
SSYAGSNNLV

SEQ ID NO: 913 - protein, 124 aa, synthetic construct; identical to SEQ ID NO: 889

SEQ ID NO: 914 - protein, 8 aa, synthetic construct
GGTFSSYA

SEQ ID NO: 915 - protein, 8 aa, synthetic construct
IFAMFGRA

SEQ ID NO: 916 - protein, 17 aa, synthetic construct
ARTSDQFYSNYAYGMDV

SEQ ID NO: 917 - protein, 113 aa, synthetic construct
DIVMTQSPDSLAVSLGERATINCKSSQSVLKSSINKNYLAWYQQKPGQPPKLLIYWASTRESGVPDRFSGSGSGTDFTLTISSLQAEDVAVYYCQQYYSTPLTFGGGTKVEIK

SEQ ID NO: 918 - protein, 12 aa, synthetic construct
QSVLKSSINKNY

SEQ ID NO: 919 - skipped

SEQ ID NO: 920 - protein, 9 aa, synthetic construct
QQYYSTPLT

SEQ ID NO: 921 - protein, 124 aa, synthetic construct; identical to SEQ ID NO: 889

SEQ ID NO: 922 - protein, 8 aa, synthetic construct
GGTFSSYA

SEQ ID NO: 923 - protein, 8 aa, synthetic construct
IFAMFGRA

SEQ ID NO: 924 - protein, 17 aa, synthetic construct
ARTSDQFYSNYAYGMDV

SEQ ID NO: 925 - protein, 110 aa, synthetic construct
NFILTQPHSVSASPGKTVTISCTGNSGSIASNYVHWYQQRPGSAPTTIIYEDNQRPSGVPDRFSGSIDSSSNSASLTISGLKTEDEADYYCQSFDGNNEVFGGGTKLTVL

SEQ ID NO: 926 - protein, 8 aa, synthetic construct
SGSIASNY

SEQ ID NO: 927 - skipped

SEQ ID NO: 928 - protein, 9 aa, synthetic construct
QSFDGNNEV

SEQ ID NO: 929 - protein, 126 aa, synthetic construct
QVQLVQSGAEVKKPGASVKVSCKASGYTFTGYYMHWVRQAPGQGLEWMGRINPNSGDTNYAQKFQGRVTMTRDTSISTAYMELSRLRSDDTAVYYCARDYYASGSYYSYDYGIDVWGKGTTVTVSS

SEQ ID NO: 930 - protein, 8 aa, synthetic construct
GYTFTGYY

SEQ ID NO: 931 - protein, 8 aa, synthetic construct
INPNSGDT

SEQ ID NO: 932 - protein, 19 aa, synthetic construct
ARDYYASGSYYSYDYGIDV

SEQ ID NO: 933 - protein, 113 aa, synthetic construct; identical to SEQ ID NO: 917

SEQ ID NO: 934 - protein, 12 aa, synthetic construct
QSVLKSSINKNY

SEQ ID NO: 935 - skipped

SEQ ID NO: 936 - protein, 9 aa, synthetic construct
QQYYSTPLT

SEQ ID NO: 937 - protein, 123 aa, synthetic construct
QVQLQQWGAGLLKPSETLSLTCTVSGGSFSGYYWSWIRQPPGKGLEWIGEITHGGGTNYKPSLKSRVTITLDTSENQFSLKLSSVTAADTAVYYCARTGWEYYGSGSLPFDYWGHGTLVTVSS

SEQ ID NO: 938 - protein, 8 aa, synthetic construct
GGSFSGYY

SEQ ID NO: 939 - protein, 7 aa, synthetic construct
ITHGGGT

SEQ ID NO: 940 - protein, 17 aa, synthetic construct
ARTGWEYYGSGSLPFDY

SEQ ID NO: 941 - protein, 117 aa, synthetic construct
DIVMTQSPDSLAVSLGERATINCKSSQSVLYSSLLTSNNKNYLAWYQQKPGQPPKLLIYWASTRESGVPDRFSGSGSGTDFTLTISSLQAEDVAVYYCQQYYTTPRTFGQGTKVEIK

SEQ ID NO: 942 - protein, 16 aa, synthetic construct
QSVLYSSLLTSNNKNY

SEQ ID NO: 943 - skipped

SEQ ID NO: 944 - protein, 9 aa, synthetic construct
QQYYTTPRT

SEQ ID NO: 945 - protein, 124 aa, synthetic construct; identical to SEQ ID NO: 889

SEQ ID NO: 946 - protein, 8 aa, synthetic construct
GGTFSSYA

SEQ ID NO: 947 - protein, 8 aa, synthetic construct
IFAMFGRA

SEQ ID NO: 948 - protein, 17 aa, synthetic construct
ARTSDQFYSNYAYGMDV

SEQ ID NO: 949 - protein, 107 aa, synthetic construct
DIQMTQSPSSLSASVGDRVTITCRASQGVSNYLAWFQQKPGKAPKSLIYAASSLQIGVPSRFSGSGSGTHFTLTISSLHPEDFATYYCQEYYSYPGTFGQGTKVEIK

SEQ ID NO: 950 - protein, 6 aa, synthetic construct
QGVSNY

SEQ ID NO: 951 - skipped

SEQ ID NO: 952 - protein, 9 aa, synthetic construct
QEYYSYPGT

SEQ ID NO: 953 - protein, 122 aa, synthetic construct
EVQLVQSGAEVKKPGESLRISCKGSGYSFTTYWISWVRQMPGKGLEWMGKIDPSNSYSNYSPSFQGHVTISVDRSISTAYLQWSSLKASDTAMYYCASLCRGGLGDPYNCDWGQGTLVTVSS

SEQ ID NO: 954 - protein, 8 aa, synthetic construct
GYSFTTYW

SEQ ID NO: 955 - protein, 8 aa, synthetic construct
IDPSNSYS

SEQ ID NO: 956 - protein, 15 aa, synthetic construct
ASLCRGGLGDPYNCD

SEQ ID NO: 957 - protein, 113 aa, synthetic construct; identical to SEQ ID NO: 917

SEQ ID NO: 958 - protein, 12 aa, synthetic construct
QSVLKSSINKNY

SEQ ID NO: 959 - skipped

SEQ ID NO: 960 - protein, 9 aa, synthetic construct
QQYYSTPLT

SEQ ID NO: 961 - protein, 126 aa, synthetic construct
QVQLVESGGGVVQPGRSLRLSCAASGFTFSSYGMHWVRQAPGKGLEWVALIWYDGSNKYYADSVKGRFTISRDNSKNTLYLQVNSLRAEDTAVYYCARCGFDYVWGTYRSDALDIWGQGTMVTVSS

SEQ ID NO: 962 - protein, 8 aa, synthetic construct
GFTFSSYG

SEQ ID NO: 963 - protein, 8 aa, synthetic construct
IWYDGSNK

SEQ ID NO: 964 - protein, 19 aa, synthetic construct
ARCGFDYVWGTYRSDALDI

SEQ ID NO: 965 - protein, 107 aa, synthetic construct
EIVLTQSPGTLSLSPGERATLSCRASQTVRSSYLAWYQQKPGQAPRLLISAASSRAAGIPDRFSGSGSGTDFTLTINRLEPEDFAVYYCQQYDSSLTFGGGTKVEIK

SEQ ID NO: 966 - protein, 7 aa, synthetic construct
QTVRSSY

SEQ ID NO: 967 - skipped

SEQ ID NO: 968 - protein, 8 aa, synthetic construct
QQYDSSLT

SEQ ID NO: 969 - protein, 125 aa, synthetic construct
EVQLVESGGGLVQPGGSLRLSCVASGFTFSNYNMNWVRQAPGKGLEWVSYIDYSSSTIYYADSVKGRFTISRDNAKNSLYMQMNSLRDEDTAVYYCARRGDGNTAIYYYYYMDVWGKGTTVTVSS

SEQ ID NO: 970 - protein, 8 aa, synthetic construct
GFTFSNYN

SEQ ID NO: 971 - protein, 8 aa, synthetic construct
IDYSSSTI

SEQ ID NO: 972 - protein, 18 aa, synthetic construct
ARRGDGNTAIYYYYYMDV

SEQ ID NO: 973 - protein, 108 aa, synthetic construct
EIVMTQSPATLSVSPGERATLSCRASQNVNSNLAWYQQKPGQAPRLLIYGASTRATGIPARFSGSGSGTEFTLTISSLQSEDFAVYYCQQYNYWPPLTFGGGTKVEIK

SEQ ID NO: 974 - protein, 6 aa, synthetic construct
QNVNSN

SEQ ID NO: 975 - skipped

SEQ ID NO: 976 - protein, 10 aa, synthetic construct
QQYNYWPPLT

SEQ ID NO: 977 - protein, 125 aa, synthetic construct
EVQLVESGGGLVQPGGSLRLSCAASGFTVSSNYMSWVRQAPGKGLEWVSVIYSGGSTYYADSVKGRFTISRDNSKNTLYLQMNSLRAEDTAMYYCARDLGTFYYDTSGYPLIPIWGQGTLVTVSS

SEQ ID NO: 978 - protein, 8 aa, synthetic construct
GFTVSSNY

SEQ ID NO: 979 - protein, 7 aa, synthetic construct
IYSGGST

SEQ ID NO: 980 - protein, 19 aa, synthetic construct
ARDLGTFYYDTSGYPLIPI

SEQ ID NO: 981 - protein, 108 aa, synthetic construct
DIQLTQSPSFLSASVGDRVTITCRASQGISNYLAWYQQKPGKAPKLLIYAASTLQSGVPSRFSGSGSGTEFTLTISSLQPEDFASYYCQQLNSDPPYTFGQGTKLEIK

SEQ ID NO: 982 - protein, 6 aa, synthetic construct
QGISNY

SEQ ID NO: 983 - skipped

SEQ ID NO: 984 - protein, 10 aa, synthetic construct
QQLNSDPPYT

SEQ ID NO: 985 - protein, 125 aa, synthetic construct; identical to SEQ ID NO: 969

SEQ ID NO: 986 - protein, 8 aa, synthetic construct
GFTFSNYN

SEQ ID NO: 987 - protein, 8 aa, synthetic construct
IDYSSSTI

SEQ ID NO: 988 - protein, 18 aa, synthetic construct
ARRGDGNTAIYYYYYMDV

SEQ ID NO: 989 - protein, 109 aa, synthetic construct
EIVLTQSPGTLSLSPGERATLSCRASQSVNRNYLAWYQQKAGQAPRLLIYGASSRATGIPDRFSGSGSGTDFSLIISRLEPEDFAVYYCQQYDRSPTWTFGQGTKVEIK

SEQ ID NO: 990 - protein, 7 aa, synthetic construct
QSVNRNY

SEQ ID NO: 991 - skipped

SEQ ID NO: 992 - protein, 10 aa, synthetic construct
QQYDRSPTWT

SEQ ID NO: 993 - protein, 122 aa, synthetic construct
QVQLVESGGGVVQPGGSLRLSCAASGFTFSSYGMHWVRQAPGKGLEWVAFIRYDGSNKYYADSVKGRFTISRDNSKNTLYLQMNSLRAEDTAVYYCAKDPGRSYDYYYMDVWGKGTTVTVSS

SEQ ID NO: 994 - protein, 8 aa, synthetic construct
GFTFSSYG

SEQ ID NO: 995 - protein, 8 aa, synthetic construct
IRYDGSNK

SEQ ID NO: 996 - protein, 15 aa, synthetic construct
AKDPGRSYDYYYMDV

SEQ ID NO: 997 - protein, 109 aa, synthetic construct
EIVLTQSPGTLSLSPGERATLSCRASQSVNRNYLAWYQQKPGQAPRLLIYGASSRATGIPDRFSGSGSGTDFSLIISRLEPEDFAVYYCQQYDSSPTWTFGQGTKVEIK

SEQ ID NO: 998 - protein, 7 aa, synthetic construct
QSVNRNY

SEQ ID NO: 999 - skipped

SEQ ID NO: 1000 - protein, 10 aa, synthetic construct
QQYDSSPTWT

SEQ ID NO: 1001 - protein, 121 aa, synthetic construct
EVQLVESGGGLTQPGGSLRLSCAASGFTFSSYTMNWVRQAPGKGLEWVSAISGSGGRTYYADSVKGRFTISRDNSKNTLFLQMNSLRAEDTAVYYCAKASAVGYYYYMDVWGKGTTVTVSS

SEQ ID NO: 1002 - protein, 8 aa, synthetic construct
GFTFSSYT

SEQ ID NO: 1003 - protein, 8 aa, synthetic construct
ISGSGGRT

SEQ ID NO: 1004 - protein, 14 aa, synthetic construct
AKASAVGYYYYMDV

SEQ ID NO: 1005 - protein, 108 aa, synthetic construct; identical to SEQ ID NO: 973

SEQ ID NO: 1006 - protein, 6 aa, synthetic construct
QNVNSN

SEQ ID NO: 1007 - skipped

SEQ ID NO: 1008 - protein, 10 aa, synthetic construct
QQYNYWPPLT

SEQ ID NO: 1009 - protein, 119 aa, synthetic construct
EVQLVESGGGLVKPGGSLRLSCAASGFTFSSSTMNWVRQAPGKGLEWVSSISSSSNYIYYADSVKGRFTISRDNAKNSLYLQMSSLRAEDTAVYYCATETNSAWVFDYWGQGTLVTVSS

SEQ ID NO: 1010 - protein, 8 aa, synthetic construct
GFTFSSST

SEQ ID NO: 1011 - protein, 8 aa, synthetic construct
ISSSSNYI

SEQ ID NO: 1012 - protein, 12 aa, synthetic construct
ATETNSAWVFDY

SEQ ID NO: 1013 - protein, 107 aa, synthetic construct
EIVLTQSPGTLSLSPGERATLSCRASQSISSNYLAWYQQKPGQAPRLLIYGASSRATGIPDRFSGSGSGTDFTLTISRLEPEDFAVYYCQQYVTSPTFGQGTKVEIK

SEQ ID NO: 1014 - protein, 7 aa, synthetic construct
QSISSNY

SEQ ID NO: 1015 - skipped

SEQ ID NO: 1016 - protein, 8 aa, synthetic construct
QQYVTSPT

SEQ ID NO: 1017 - protein, 121 aa, synthetic construct; identical to SEQ ID NO: 1001

SEQ ID NO: 1018 - protein, 8 aa, synthetic construct
GFTFSSYT

SEQ ID NO: 1019 - protein, 8 aa, synthetic construct
ISGSGGRT

SEQ ID NO: 1020 - protein, 14 aa, synthetic construct
AKASAVGYYYYMDV

SEQ ID NO: 1021 - protein, 109 aa, synthetic construct
QSVLTQPPSASGTPGQRVTISCSGSSSNIGSNTVNWYQQLPGTAPKLLIYSNNQRPSGVPDRFSGSKSGTSASLAISGLQSEDEADYYCAAWDDSLNGLFGTGTKVTVL

SEQ ID NO: 1022 - protein, 8 aa, synthetic construct
SSNIGSNT

SEQ ID NO: 1023 - skipped

SEQ ID NO: 1024 - protein, 10 aa, synthetic construct
AAWDDSLNGL

SEQ ID NO: 1025 - protein, 121 aa, synthetic construct; identical to SEQ ID NO: 1001

SEQ ID NO: 1026 - protein, 8 aa, synthetic construct
GFTFSSYT

SEQ ID NO: 1027 - protein, 8 aa, synthetic construct
ISGSGGRT

SEQ ID NO: 1028 - protein, 14 aa, synthetic construct
AKASAVGYYYYMDV

SEQ ID NO: 1029 - protein, 107 aa, synthetic construct
DIQMTQSPSSLSASVGDRVTITCQASQDISNYLNWYQQKPGKAPKLLIYDASNLETGVPSRFSGSGSGTDFTFTISSLQPEDIATYYCQQYDNLPLTFGGGTKVEIK

SEQ ID NO: 1030 - protein, 6 aa, synthetic construct
QDISNY

SEQ ID NO: 1031 - skipped

SEQ ID NO: 1032 - protein, 9 aa, synthetic construct
QQYDNLPLT

SEQ ID NO: 1033 - protein, 130 aa, synthetic construct
QVQLVESGGGVVQPGRSLRLSCATSGFTFRSYGMHWVRQAPGKGLEWVAVISFDGSSKYYADSVKGRFTISRDNSENTLYLQMNSLRAQDTAVYFCAKGAFGGFCRGGSCYDVPLSIDYWGRGTTVTVSS

SEQ ID NO: 1034 - protein, 8 aa, synthetic construct
GFTFRSYG

SEQ ID NO: 1035 - protein, 8 aa, synthetic construct
ISFDGSSK

SEQ ID NO: 1036 - protein, 23 aa, synthetic construct
AKGAFGGFCRGGSCYDVPLSIDY

SEQ ID NO: 1037 - protein, 110 aa, synthetic construct
QSVLTQPPSASGTPGQRVTISCSGSSSNIGSNTVNWYQQLPGTAPKLLIYSNNQRPSGVPDRFSGSKSGTSASLAISGLQSEDEADYYCAPWDDSLNGPVFGGGTKLTVL

SEQ ID NO: 1038 - protein, 8 aa, synthetic construct
SSNIGSNT

SEQ ID NO: 1039 - skipped

SEQ ID NO: 1040 - protein, 11 aa, synthetic construct
APWDDSLNGPV

SEQ ID NO: 1041 - protein, 25 aa, synthetic construct [sequence omitted]

SEQ ID NO: 1042 - protein, 17 aa, synthetic construct
MHWVRQAPGRGLEWMGI

SEQ ID NO: 1043 - protein, 38 aa, synthetic construct
TYAPKFQGRVTMTRDTSTSRVYLEMSSLRSEDTAVYYC

SEQ ID NO: 1044 - protein, 11 aa, synthetic construct
WGQGTTVTVSS

SEQ ID NO: 1045 - protein, 25 aa, synthetic construct
QTVVTQEPSLTVSPGGTVTLTCASS

SEQ ID NO: 1046 - protein, 17 aa, synthetic construct
PNWFQQKPGQAPRALIY

SEQ ID NO: 1047 - protein, 36 aa, synthetic construct
NKHSWTPARFSGSLLGGKAALTLSGVQPEDEAEYYC

SEQ ID NO: 1048 - protein, 10 aa, synthetic construct
FGGGTKLTVL

SEQ ID NO: 1049 - protein, 25 aa, synthetic construct
EVQLVESGGGLVQPGRSLRLSCVGS

SEQ ID NO: 1050 - protein, 17 aa, synthetic construct
MHWVRQVPGKGLEWVSG

SEQ ID NO: 1051 - protein, 38 aa, synthetic construct
GYVDSVKGRFSISRDNAKKSLYLQMNSLRAEDTGLYYC

SEQ ID NO: 1052 - protein, 11 aa, synthetic construct
WGQGTLVTVSS

SEQ ID NO: 1053 - protein, 26 aa, synthetic construct
DIQMTQSPSSLSASVGDRVTITCQAS

SEQ ID NO: 1054 - protein, 17 aa, synthetic construct
LNWYQQKPGKAPKLLIY

SEQ ID NO: 1055 - protein, 36 aa, synthetic construct
NLEPGVPSRFSGTGSGTDFTFTISSLQPEDVATYYC

SEQ ID NO: 1056 - protein, 10 aa, synthetic construct
FGQGTKVEIK

SEQ ID NO: 1057 - protein, 25 aa, synthetic construct
EVHLVESGGGLVQPGRSLRLSCAAS

SEQ ID NO: 1058 - protein, 17 aa, synthetic construct
MHWVRQPPGKGLEWVSG

SEQ ID NO: 1059 - protein, 38 aa, synthetic construct
AYADSVKGRFTISRDNAKNSLSLQMNSLRAEDSAFYYC

SEQ ID NO: 1060 - protein, 11 aa, synthetic construct
WGQGTLVTVSS

SEQ ID NO: 1061 - protein, 25 aa, synthetic construct
QSVLTQPPSVFGAPGQRVTISCTGS

SEQ ID NO: 1062 - protein, 17 aa, synthetic construct
VHWYQQLPGTAPKVLIY

SEQ ID NO: 1063 - protein, 36 aa, synthetic construct
KRPSGVPDRFSGSKSGTSASLAITGLQAEDEADYYC

SEQ ID NO: 1064 - protein, 10 aa, synthetic construct
FGGGTKLTVL

SEQ ID NO: 1065 - protein, 25 aa, synthetic construct
EVHLVESGGGLVQPGRSLRLSCAAS

SEQ ID NO: 1066 - protein, 17 aa, synthetic construct
MHWVRQPPGKGLEWVSG

SEQ ID NO: 1067 - protein, 38 aa, synthetic construct; identical to SEQ ID NO: 1059

SEQ ID NO: 1068 - protein, 11 aa, synthetic construct
WGQGTLVTVSS

SEQ ID NO: 1069 - protein, 25 aa, synthetic construct
QSALTQPASVSGSPGQPITISCTGT

SEQ ID NO: 1070 - protein, 17 aa, synthetic construct
VSWYQQHPGKAPKLMIY

SEQ ID NO: 1071 - protein, 36 aa, synthetic construct
ERPSGVSSRFSGSKSGNTASLTISGLQAEDEADYYC

SEQ ID NO: 1072 - protein, 10 aa, synthetic construct
FGGGTKLTVL

SEQ ID NO: 1073 - protein, 25 aa, synthetic construct [sequence omitted]

SEQ ID NO: 1074 - protein, 17 aa, synthetic construct
MNWVRQAPGKGLEWVSY

SEQ ID NO: 1075 - protein, 38 aa, synthetic construct
YYADSVKGRFTISRDNAKNSLYLQMNSLRDEDTAFYYC

SEQ ID NO: 1076 - protein, 11 aa, synthetic construct
WGQGTLVTVSS

SEQ ID NO: 1077 - protein, 25 aa, synthetic construct
QSVLTQPPSVFGAPGQRVTISCTGS

SEQ ID NO: 1078 - protein, 17 aa, synthetic construct
VHWYQQLPGTAPKVLIY

SEQ ID NO: 1079 - protein, 36 aa, synthetic construct; identical to SEQ ID NO: 1063

SEQ ID NO: 1080 - protein, 10 aa, synthetic construct
FGGGTKLTVL

SEQ ID NO: 1081 - protein, 25 aa, synthetic construct [sequence omitted]

SEQ ID NO: 1082 - protein, 17 aa, synthetic construct
MNWVRQAPGKGLEWVSY

SEQ ID NO: 1083 - protein, 38 aa, synthetic construct; identical to SEQ ID NO: 1075

SEQ ID NO: 1084 - protein, 11 aa, synthetic construct
WGQGTLVTVSS

SEQ ID NO: 1085 - protein, 25 aa, synthetic construct
QSALTQPASVSGSPGQPITISCTGT

SEQ ID NO: 1086 - protein, 17 aa, synthetic construct
VSWYQQHPGKAPKLMIY

SEQ ID NO: 1087 - protein, 36 aa, synthetic construct; identical to SEQ ID NO: 1071

SEQ ID NO: 1088 - protein, 10 aa, synthetic construct
FGGGTKLTVL

SEQ ID NO: 1089 - protein, 25 aa, synthetic construct
QVQLLQSGAEVKKPGSSVKVSCKAS

SEQ ID NO: 1090 - protein, 17 aa, synthetic construct
MTWVRQAPGQGFEWMGE

SEQ ID NO: 1091 - protein, 38 aa, synthetic construct
KYAQKFQGRVTITADESTTTAYMDLRSLRSDDTAVYYC

SEQ ID NO: 1092 - protein, 11 aa, synthetic construct
WGQGTLVTVSS

SEQ ID NO: 1093 - protein, 26 aa, synthetic construct
DIQMTQSPSSLSASVRDRVTITCRAS

SEQ ID NO: 1094 - protein, 17 aa, synthetic construct
LNWYQQKPGKAPNLLIY

SEQ ID NO: 1095 - protein, 36 aa, synthetic construct
SLHSGVPSRFSGSGSGSDFTLTISSLQPEDFGYYYC

SEQ ID NO: 1096 - protein, 10 aa, synthetic construct
FGQGTKVEIK

SEQ ID NO: 1097 - protein, 25 aa, synthetic construct
QVQLLQSGAEVKKPGSSVKVSCKAS

SEQ ID NO: 1098 - protein, 17 aa, synthetic construct
MTWVRQAPGQGFEWMGE

SEQ ID NO: 1099 - protein, 38 aa, synthetic construct; identical to SEQ ID NO: 1091

SEQ ID NO: 1100 - protein, 11 aa, synthetic construct
WGQGTLVTVSS

SEQ ID NO: 1101 - protein, 26 aa, synthetic construct [sequence omitted]

SEQ ID NO: 1102 - protein, 17 aa, synthetic construct
LAWYQQKSGQAPRLLIY

SEQ ID NO: 1103 - protein, 36 aa, synthetic construct
SRATGIPDRFSGSGSGTDFTLTISRLEPEDFAVYFC

SEQ ID NO: 1104 - protein, 10 aa, synthetic construct
FGGGTKVEIK

SEQ ID NO: 1105 - protein, 25 aa, synthetic construct
QVQLVESGGGVVQPGRSLRLSCAAS

SEQ ID NO: 1106 - protein, 17 aa, synthetic construct
MHWVRQAPGKGLEWVAI

SEQ ID NO: 1107 - protein, 38 aa, synthetic construct
NHADSVKDRFTISRDNSKNTLFLQMNSLRAEDTAVYYC

SEQ ID NO: 1108 - protein, 11 aa, synthetic construct
WGQGTTVTVSS

SEQ ID NO: 1109 - protein, 26 aa, synthetic construct
DIQMTQSPSSLSASVRDRVTITCRAS

SEQ ID NO: 1110 - protein, 17 aa, synthetic construct
LNWYQQKPGKAPNLLIY

SEQ ID NO: 1111 - protein, 36 aa, synthetic construct; identical to SEQ ID NO: 1095

SEQ ID NO: 1112 - protein, 10 aa, synthetic construct
FGQGTKVEIK

SEQ ID NO: 1113 - protein, 25 aa, synthetic construct
QVQLVESGGGVVQPGRSLRLSCAAS

SEQ ID NO: 1114 - protein, 17 aa, synthetic construct
MHWVRQAPGKGLEWVAI

SEQ ID NO: 1115 - protein, 38 aa, synthetic construct; identical to SEQ ID NO: 1107

SEQ ID NO: 1116 - protein, 11 aa, synthetic construct
WGQGTTVTVSS

SEQ ID NO: 1117 - protein, 26 aa, synthetic construct [sequence omitted]

SEQ ID NO: 1118 - protein, 17 aa, synthetic construct
LAWYQQKSGQAPRLLIY

SEQ ID NO: 1119 - protein, 36 aa, synthetic construct; identical to SEQ ID NO: 1103

SEQ ID NO: 1120 - protein, 10 aa, synthetic construct
FGGGTKVEIK

SEQ ID NO: 1121 - protein, 25 aa, synthetic construct [sequence omitted]

SEQ ID NO: 1122 - protein, 17 aa, synthetic construct
VIWVRQASGQGLEWMGR

SEQ ID NO: 1123 - protein, 38 aa, synthetic construct
DYAQKFQGRVTMTTDTSTSTVYMELRSLRADDTAVYYC

SEQ ID NO: 1124 - protein, 11 aa, synthetic construct
WGQGTTVTVSS

SEQ ID NO: 1125 - protein, 26 aa, synthetic construct
DIQMTQSPSSLSASVGDRVTITCQAS

SEQ ID NO: 1126 - protein, 17 aa, synthetic construct
LNWYQQKPGKAPRLLIS

SEQ ID NO: 1127 - protein, 36 aa, synthetic construct
SLETGVPSRFSGSGSGTDFTFTISSLQPEDIATYYC

SEQ ID NO: 1128 - protein, 10 aa, synthetic construct
FGGGTKLEIK

SEQ ID NO: 1129 - protein, 25 aa, synthetic construct
QVQLVESGGGVVQPGRSLRLSCAAS

SEQ ID NO: 1130 - protein, 17 aa, synthetic construct
MHWVRQAPGKGLEWVAA

SEQ ID NO: 1131 - protein, 38 aa, synthetic construct
FYADSVKGRFTISRDNSKNTLYLQMNSLRVEDTAMYFC

SEQ ID NO: 1132 - protein, 11 aa, synthetic construct
WGLGTLVTVSS

SEQ ID NO: 1133 - protein, 26 aa, synthetic construct [sequence omitted]

SEQ ID NO: 1134 - protein, 17 aa, synthetic construct
LNWFQQKPGKAPKLLIY

SEQ ID NO: 1135 - protein, 36 aa, synthetic construct
SLQSGVPSRFSGSGSGTDFTLTISSLQYEDFATYYC

SEQ ID NO: 1136 - protein, 10 aa, synthetic construct
FGQGTKVEIK

SEQ ID NO: 1137 - protein, 25 aa, synthetic construct
QVQLGESGGGVVQPGRSLRLSCAAS

SEQ ID NO: 1138 - protein, 17 aa, synthetic construct
MHWVRQAPGKGLEWVAV

SEQ ID NO: 1139 - protein, 38 aa, synthetic construct
YYADSVKGRFTISSDNSNNTLYLQMNTLRAEDTAVYYC

SEQ ID NO: 1140 - protein, 11 aa, synthetic construct
WGQGTTVTVSS

SEQ ID NO: 1141 - protein, 26 aa, synthetic construct [sequence omitted]

SEQ ID NO: 1142 - protein, 17 aa, synthetic construct
LAWYQQKPGQAPRLLID

SEQ ID NO: 1143 - protein, 36 aa, synthetic construct [sequence omitted]

SEQ ID NO: 1144 - protein, 10 aa, synthetic construct
FGQGTKLEIK

SEQ ID NO: 1145 - protein, 25 aa, synthetic construct [sequence omitted]

SEQ ID NO: 1146 - protein, 17 aa, synthetic construct
MNWVRQTPGKGLEWVSV

SEQ ID NO: 1147 - protein, 38 aa, synthetic construct
YYADSVKGRFTISRDNSKNTLNLQMISLRPEDTAIYYC

SEQ ID NO: 1148 - protein, 11 aa, synthetic construct
WGPGTLVTVSS

SEQ ID NO: 1149 - protein, 25 aa, synthetic construct
QSALTQPASVSGSPGQSITISCTGT

SEQ ID NO: 1150 - protein, 17 aa, synthetic construct
VSWYQQHPGKAPKLIIY

SEQ ID NO: 1151 - protein, 36 aa, synthetic construct
KRPAGVSHRFSGSESGNTASLTISGLQAEDEADYYC

SEQ ID NO: 1152 - protein, 10 aa, synthetic construct
FGGGTKLTVL

SEQ ID NO: 1153 - protein, 25 aa, synthetic construct
QVQVVQSGAEVKKPGASVKVSCKAS

SEQ ID NO: 1154 - protein, 17 aa, synthetic construct
MHWVRQAPGQGLEWMGW

SEQ ID NO: 1155 - protein, 38 aa, synthetic construct
NYAQKFQGRVTMTRDTSISTAYMELSRLRSDDTAVYYC

SEQ ID NO: 1156 - protein, 11 aa, synthetic construct
WGQGTLVTVSS

SEQ ID NO: 1157 - protein, 25 aa, synthetic construct
QSALTQPPSASGSPGQSVTISCTGT

SEQ ID NO: 1158 - protein, 17 aa, synthetic construct
VSWYQQHPGKAPKLMIY

SEQ ID NO: 1159 - protein, 36 aa, synthetic construct
KRPSGVPDRFSGSKSGNTASLTVSGLQAEDEADYYC

SEQ ID NO: 1160 - protein, 10 aa, synthetic construct
FGGGTKVTVL

SEQ ID NO: 1161 - protein, 25 aa, synthetic construct [sequence omitted]

SEQ ID NO: 1162 - protein, 17 aa, synthetic construct
MHWVRQAPGKGPEWVSG

SEQ ID NO: 1163 - protein, 38 aa, synthetic construct
GYADSVKGQFIISRDNAKNSLYLQMNSLRPEDTALYYC

SEQ ID NO: 1164 - protein, 11 aa, synthetic construct
WGQGTTVTVSS

SEQ ID NO: 1165 - protein, 25 aa, synthetic construct
NFMLTQPHSVSESPGKTVSISCTRS

SEQ ID NO: 1166 - protein, 17 aa, synthetic construct
VQWYQQRPGSAPTTVIY

SEQ ID NO: 1167 - protein, 38 aa, synthetic construct
QRPSGVPDRFSGSIDSSSNSASLTISGLKTEDEADYYC

SEQ ID NO: 1168 - protein, 10 aa, synthetic construct
FGGGTKVTVL

SEQ ID NO: 1169 - protein, 25 aa, synthetic construct [sequence omitted]

SEQ ID NO: 1170 - protein, 17 aa, synthetic construct
MHWVRQAPGKGLEWVSG

SEQ ID NO: 1171 - protein, 38 aa, synthetic construct
GYADSVKGRFTISRDNAKNSLYLQMNRLRAEDTALYYC

SEQ ID NO: 1172 - protein, 11 aa, synthetic construct
WGQGTTVTVSS

SEQ ID NO: 1173 - protein, 26 aa, synthetic construct
DIQLTQSPSFLSASVGDRVTLTCRAS

SEQ ID NO: 1174 - protein, 17 aa, synthetic construct
LAWYQQKPGKAPNLLIY

SEQ ID NO: 1175 - protein, 36 aa, synthetic construct
TLQSGVPSRFSGSGSGTEFTLTISSLQPEDFATYYC

SEQ ID NO: 1176 - protein, 10 aa, synthetic construct
FGGGTKVEIK

SEQ ID NO: 1177 - protein, 25 aa, synthetic construct [sequence omitted]

SEQ ID NO: 1178 - protein, 17 aa, synthetic construct
MHWVRQAPGKGLEWVSG

SEQ ID NO: 1179 - protein, 38 aa, synthetic construct; identical to SEQ ID NO: 1171

SEQ ID NO: 1180 - protein, 11 aa, synthetic construct
WGQGTTVTVSS

SEQ ID NO: 1181 - protein, 25 aa, synthetic construct
QSALTQPASVSGSPGQSITISCTGT

SEQ ID NO: 1182 - protein, 17 aa, synthetic construct
VSWYQQHPGKAPKLMIY

SEQ ID NO: 1183 - protein, 36 aa, synthetic construct
HRPSGVSNRFSGSKSGNTASLTISGLQAEDEADYYC

SEQ ID NO: 1184 - protein, 10 aa, synthetic construct
FGGGTKVTVL

SEQ ID NO: 1185 - protein, 25 aa, synthetic construct
QVQLVESGGGVVQPGRSLRLSCAAS

SEQ ID NO: 1186 - protein, 17 aa, synthetic construct
MHWVRQAPGKGLEWVAF

SEQ ID NO: 1187 - protein, 38 aa, synthetic construct
YYADSVKGRFTISRDNSKNTLYLQMNSLRVEDTAVYYC

SEQ ID NO: 1188 - protein, 11 aa, synthetic construct
WGQGILVTVSS

SEQ ID NO: 1189 - protein, 26 aa, synthetic construct
DIQLTQSPSFLSASVGDRVTLTCRAS

SEQ ID NO: 1190 - protein, 17 aa, synthetic construct
LAWYQQKPGKAPNLLIY

SEQ ID NO: 1191 - protein, 36 aa, synthetic construct; identical to SEQ ID NO: 1175

SEQ ID NO: 1192 - protein, 10 aa, synthetic construct
FGGGTKVEIK

SEQ ID NO: 1193 - protein, 25 aa, synthetic construct
QVQLVESGGGVVQPGRSLRLSCAAS

SEQ ID NO: 1194 - protein, 17 aa, synthetic construct
MHWVRQAPGKGLEWVAF

SEQ ID NO: 1195 - protein, 38 aa, synthetic construct; identical to SEQ ID NO: 1187

SEQ ID NO: 1196 - protein, 11 aa, synthetic construct
WGQGILVTVSS

SEQ ID NO: 1197 - protein, 25 aa, synthetic construct
QSALTQPASVSGSPGQSITISCTGT

SEQ ID NO: 1198 - protein, 17 aa, synthetic construct
VSWYQQHPGKAPKLMIY

SEQ ID NO: 1199 - protein, 36 aa, synthetic construct; identical to SEQ ID NO: 1183

SEQ ID NO: 1200 - protein, 10 aa, synthetic construct
FGGGTKVTVL

SEQ ID NO: 1201 - protein, 25 aa, synthetic construct
EVLLVESGGGLVQPGGSLRLSCAAS

SEQ ID NO: 1202 - protein, 17 aa, synthetic construct
MNWVRQAPGKGLEWVSV

SEQ ID NO: 1203 - protein, 38 aa, synthetic construct
DYGDSVKGRFTISRDKSKNTLSLQMNSLRAEDTAVYYC

SEQ ID NO: 1204 - protein, 11 aa, synthetic construct
WGQGTTVTVSS

SEQ ID NO: 1205 - protein, 26 aa, synthetic construct
EMVMTQSPATLSVSPGERATLSCRAS

SEQ ID NO: 1206 - protein, 17 aa, synthetic construct
LAWYQQKNGQAPRLLIY

SEQ ID NO: 1207 - protein, 36 aa, synthetic construct
TRATGIPARFSGSGSGTEFTLTISSLQSEDFAIYYC

SEQ ID NO: 1208 - protein, 10 aa, synthetic construct
FGQGTKVEIK

SEQ ID NO: 1209 - protein, 25 aa, synthetic construct
QMQLVQSGPEVKKPGTSVKVSCKAS

SEQ ID NO: 1210 - protein, 17 aa, synthetic construct
VQWVRQARGQRLEWIGW

SEQ ID NO: 1211 - protein, 38 aa, synthetic construct
NYAQMFQERVTITRDMSTSTAYMELSSLRSEDTAVYYC

SEQ ID NO: 1212 - protein, 11 aa, synthetic construct
WGKGTTVTVSS

SEQ ID NO: 1213 - protein, 26 aa, synthetic construct
EIVLTQSPGTLSLSPGERATLFCRAS

SEQ ID NO: 1214 - protein, 17 aa, synthetic construct
LAWYQQKPGQAPRLLIY

SEQ ID NO: 1215 - protein, 36 aa, synthetic construct
SRATGTPDRFSGSGSGTDFTLTISRLEPEDFAVYYC

SEQ ID NO: 1216 - protein, 10 aa, synthetic construct
FGQGTKVEIK

SEQ ID NO: 1217 - protein, 25 aa, synthetic construct
EVQLVESGGGLVKPGGSLRLSCVAS

SEQ ID NO: 1218 - protein, 17 aa, synthetic construct
MSWVRQAPGKGLEWVGR

SEQ ID NO: 1219 - protein, 38 aa, synthetic construct
DYAAPVKGRFTISRDDSRNTLYLQMNSLKTEDTAVYYC

SEQ ID NO: 1220 - protein, 11 aa, synthetic construct
WGQGTLVTVSS

SEQ ID NO: 1221 - protein, 26 aa, synthetic construct
DVVMTQSPLSLPVTLGQPASISCRSS

SEQ ID NO: 1222 - protein, 17 aa, synthetic construct
LSWLQQRPGQSPRRLIY

SEQ ID NO: 1223 - protein, 36 aa, synthetic construct
NRDSGVPDRFSGSGSGTYFTLKISRVEAEDVGVYYC

SEQ ID NO: 1224 - protein, 10 aa, synthetic construct
FGQGTRLEIK

SEQ ID NO: 1225 - protein, 25 aa, synthetic construct
EVQLLESGGGLVKPGGSLRLSCAAS

SEQ ID NO: 1226 - protein, 17 aa, synthetic construct
MGWVRQAPGKGLEWVST

SEQ ID NO: 1227 - protein, 38 aa, synthetic construct
YYTESVRGRFTISRDNSKNTLFLQMGSLRAEDTAVYYC

SEQ ID NO: 1228 - protein, 11 aa, synthetic construct
WGQGTLVTVSS

SEQ ID NO: 1229 - protein, 26 aa, synthetic construct
DIQMTQSPSSLSASVGDRVTITCQAS

SEQ ID NO: 1230 - protein, 17 aa, synthetic construct
LNWYQQKAGKAPKLLIY

SEQ ID NO: 1231 - protein, 36 aa, synthetic construct
NLQIGVPSRFSGSGSGTDFTFSISSLQPEDIATYYC

SEQ ID NO: 1232 - protein, 10 aa, synthetic construct
FGGGTKVEIK

SEQ ID NO: 1233 - protein, 25 aa, synthetic construct
QVQLVESGGGVVQPGRSLRLSCAAS

SEQ ID NO: 1234 - protein, 17 aa, synthetic construct
MHWVRQAPGKGLEWVAV

SEQ ID NO: 1235 - protein, 38 aa, synthetic construct
YYADSVKGRFTISRDNSKNTLNLQMNSLKVEDTAVYYC

SEQ ID NO: 1236 - protein, 11 aa, synthetic construct
WGKGTTVTVSS

SEQ ID NO: 1237 - protein, 25 aa, synthetic construct
QSALTQTASVSGSPGQSITISCTGT

SEQ ID NO: 1238 - protein, 17 aa, synthetic construct
VSWYQQHPGKAPKIMVF

SEQ ID NO: 1239 - protein, 36 aa, synthetic construct
KRPSGVSNRFSGSKSGNTASLTISGLQAEDDADYYC

SEQ ID NO: 1240 - protein, 10 aa, synthetic construct
FGGGTKVTVL

SEQ ID NO: 1241 - protein, 25 aa, synthetic construct
QVQLVESGGGVVQPGRSLRLSCEAS

SEQ ID NO: 1242 - protein, 17 aa, synthetic construct
MHWVRQAPGKGLEWVAV

SEQ ID NO: 1243 - protein, 38 aa, synthetic construct
YYADSVKGRFTISRDNSKNTLYLQMNSLRAEDTAVYYC

SEQ ID NO: 1244 - protein, 12 aa, synthetic construct
WWGQGTLVTVSS

SEQ ID NO: 1245 - protein, 26 aa, synthetic construct
DIVMTQSPDSLAVSLGERATINCKSS

SEQ ID NO: 1246 - protein, 17 aa, synthetic construct
LAWYQQKPGQPPKLLIY

SEQ ID NO: 1247 - protein, 36 aa, synthetic construct
TRESGVSDRFSGSGSGTDFTLTISSLQAEDVAVYYC

SEQ ID NO: 1248 - protein, 10 aa, synthetic construct
FGGGTKVEIK

SEQ ID NO: 1249 - protein, 25 aa, synthetic construct [sequence omitted]

SEQ ID NO: 1250 - protein, 17 aa, synthetic construct
FNWVRQAPGMGLEWLSY

SEQ ID NO: 1251 - protein, 38 aa, synthetic construct
HYAASVKGRFTISRDNAKNSLYLQMNSLKGEDTGVYYC

SEQ ID NO: 1252 - protein, 11 aa, synthetic construct
WGQGTLVTVSS

SEQ ID NO: 1253 - protein, 25 aa, synthetic construct
QSVLTQPPSASGTPGQRVSISCSGS

SEQ ID NO: 1254 - protein, 17 aa, synthetic construct
VEWYQQVPGTAPKLLIC

SEQ ID NO: 1255 - protein, 36 aa, synthetic construct
QRPSGVPDRFSGSKSGTSASLAISGLRSEDEAYYYC

SEQ ID NO: 1256 - protein, 10 aa, synthetic construct
FGGGTKLTVL

SEQ ID NO: 1257 - protein, 25 aa, synthetic construct
QVQLVESGGGLVKPGGSLRLSCAAS

SEQ ID NO: 1258 - protein, 17 aa, synthetic construct
MNWIRQAPGRGLEWISY

SEQ ID NO: 1259 - protein, 38 aa, synthetic construct
KYTDSVKGRFTISRDNAKKSLSLQMNSLRDEDTAVYYC

SEQ ID NO: 1260 - protein, 11 aa, synthetic construct
WGQGTLVTVSS

SEQ ID NO: 1261 - protein, 25 aa, synthetic construct
QSVLTQPPSVSAAPGQKVTIACSGS

SEQ ID NO: 1262 - protein, 17 aa, synthetic construct
VTWYQQLPGTAPKLLIY

SEQ ID NO: 1263 - protein, 36 aa, synthetic construct
KRPSGIPVRFSGSKSATSASLGITGLQTGDEADYYC

SEQ ID NO: 1264 - protein, 10 aa, synthetic construct
FGGGTKLTVL

SEQ ID NO: 1265 - protein, 25 aa, synthetic construct
QEQLVESGGGLVKPGGSLRLSCAAS

SEQ ID NO: 1266 - protein, 17 aa, synthetic construct
MSWIRQAPGKGLEWISY

SEQ ID NO: 1267 - protein, 38 aa, synthetic construct
DYADSVKGRFTISRDNAKNSVYLQMNSLRAEDTAVYYC

SEQ ID NO: 1268 - protein, 11 aa, synthetic construct
WGQGTTVTVSS

SEQ ID NO: 1269 - protein, 26 aa, synthetic construct
DIVMTQSPDSLAVSLGERATINCKSS

SEQ ID NO: 1270 - protein, 17 aa, synthetic construct
LAWYQQKPGQPPKLLIY

SEQ ID NO: 1271 - protein, 36 aa, synthetic construct
TRESGVPDRFSGSGSGTDFTLTISSLQAEDVAVYYC

SEQ ID NO: 1272 - protein, 10 aa, synthetic construct
FGQGTKVEIK

SEQ ID NO: 1273 - protein, 25 aa, synthetic construct
EVELLESGGGLVQPGGSLRLFCAAS

SEQ ID NO: 1274 - protein, 17 aa, synthetic construct
MSWVRQAPGKGLEWVSV

SEQ ID NO: 1275 - protein, 38 aa, synthetic construct
YYADSVKGRFTIARDNSKNTLYLQMDSLRAEDTAVYYC

SEQ ID NO: 1276 - protein, 11 aa, synthetic construct
WGQGTTVTVSS

SEQ ID NO: 1277 - protein, 26 aa, synthetic construct
GIQMTQSPSSLSASLGDRVTITCQAS

SEQ ID NO: 1278 - protein, 17 aa, synthetic construct
LNWYQQKPGKAPKLLIH

SEQ ID NO: 1279 - protein, 36 aa, synthetic construct
NLETGVPSTFSGGGSGTHFTFTINSLQPEDVATYYC

SEQ ID NO: 1280 - protein, 10 aa, synthetic construct
FGGGTKVEIK

SEQ ID NO: 1281 - protein, 25 aa, synthetic construct
EVQLVESGGSVVRPGGSLRLSCAAS

SEQ ID NO: 1282 - protein, 17 aa, synthetic construct
MSWVRQAPGKGLEWVSG

SEQ ID NO: 1283 - protein, 38 aa, synthetic construct
GYADSVKGRFTISRDNAKNSLYLQMNSLRAEDTALYHC

SEQ ID NO: 1284 - protein, 11 aa, synthetic construct
WGQGTMVTVSS

SEQ ID NO: 1285 - protein, 25 aa, synthetic construct
QSVLTQPPSVSGAPGQRVTISCTGS

SEQ ID NO: 1286 - protein, 17 aa, synthetic construct
VHWYQHLPGTAPKLLIY

SEQ ID NO: 1287 - protein, 36 aa, synthetic construct
NRPSGVPDRFSGSQSGTSASLAITGLQAEDEADYYC

SEQ ID NO: 1288 - protein, 10 aa, synthetic construct
FGGGTKLTVL

SEQ ID NO: 1289 - protein, 25 aa, synthetic construct
QVQLVQSGAEVKKPGASVKVSCKVS

SEQ ID NO: 1290 - protein, 17 aa, synthetic construct
MHWVRQAPGEGLEWMGS

SEQ ID NO: 1291 - protein, 38 aa, synthetic construct
MYSQKFQGRLTMTEDTSIDTVYMEMSSLRPEDTAIYYC

SEQ ID NO: 1292 - protein, 11 aa, synthetic construct
WGQGTTVTVSS

SEQ ID NO: 1293 - protein, 25 aa, synthetic construct
QSVLTQPPSVSAAPGQKVTISCSGS

SEQ ID NO: 1294 - protein, 17 aa, synthetic construct
VSWYQQLPGTAPRLLIF

SEQ ID NO: 1295 - protein, 36 aa, synthetic construct
KRPSGIPDRISGSKSGTSATLGITGLQPGDEADYYC

SEQ ID NO: 1296 - protein, 10 aa, synthetic construct
FGGGTKLTVL

SEQ ID NO: 1297 - protein, 25 aa, synthetic construct [sequence omitted]

SEQ ID NO: 1298 - protein, 17 aa, synthetic construct
FSWVRQAPGQGLEWMGG

SEQ ID NO: 1299 - protein, 38 aa, synthetic construct
TYAQKVQDRVTITADKSTSTAYMELSSLRSEDTSVYYC

SEQ ID NO: 1300 - protein, 11 aa, synthetic construct
WGQGTLVTVSS

SEQ ID NO: 1301 - protein, 26 aa, synthetic construct
AIQMTQSPSSLSASVGDRVTITCRAS

SEQ ID NO: 1302 - protein, 17 aa, synthetic construct
LAWYQQKPGKASKLLIY

SEQ ID NO: 1303 - protein, 36 aa, synthetic construct
SLQSGVPSRFSGSGSGTDFTLTISSLQPEDFATYYC

SEQ ID NO: 1304 - protein, 10 aa, synthetic construct
FGGGTKVEIK

SEQ ID NO: 1305 - protein, 25 aa, synthetic construct [sequence omitted]

SEQ ID NO: 1306 - protein, 17 aa, synthetic construct
FSWVRQAPGQGLEWMGG

SEQ ID NO: 1307 - protein, 38 aa, synthetic construct; identical to SEQ ID NO: 1299

SEQ ID NO: 1308 - protein, 11 aa, synthetic construct
WGQGTLVTVSS

SEQ ID NO: 1309 - protein, 25 aa, synthetic construct
QTVVTQEPSFSVSPGGTITLTCGLS

SEQ ID NO: 1310 - protein, 17 aa, synthetic construct
PSWYQQTPGQPPRTLIY

SEQ ID NO: 1311 - protein, 36 aa, synthetic construct
TRSSGVPDRFSGSIVGNKAALTITGAQADDESDYYC

SEQ ID NO: 1312 - protein, 10 aa, synthetic construct
FGGGTKVTVL

SEQ ID NO: 1313 - protein, 25 aa, synthetic construct [sequence omitted]

SEQ ID NO: 1314 - protein, 17 aa, synthetic construct
MHWVRQAPGKGLEWVSV

SEQ ID NO: 1315 - protein, 38 aa, synthetic construct
AYADSVKGRITISRDNAEKTLFLQLNSLRPEDTAVYYC

SEQ ID NO: 1316 - protein, 11 aa, synthetic construct
WGQGTLVTVSS

SEQ ID NO: 1317 - protein, 26 aa, synthetic construct
AIQMTQSPSSLSASVGDRVTITCRAS

SEQ ID NO: 1318 - protein, 17 aa, synthetic construct
LAWYQQKPGKASKLLIY

SEQ ID NO: 1319 - protein, 36 aa, synthetic construct; identical to SEQ ID NO: 1303

SEQ ID NO: 1320 - protein, 10 aa, synthetic construct
FGGGTKVEIK

SEQ ID NO: 1321 - protein, 25 aa, synthetic construct [sequence omitted]

SEQ ID NO: 1322 - protein, 17 aa, synthetic construct
MHWVRQAPGKGLEWVSV

SEQ ID NO: 1323 - protein, 38 aa, synthetic construct; identical to SEQ ID NO: 1315

SEQ ID NO: 1324 - protein, 11 aa, synthetic construct
WGQGTLVTVSS

SEQ ID NO: 1325 - protein, 25 aa, synthetic construct
QTVVTQEPSFSVSPGGTITLTCGLS

SEQ ID NO: 1326 - protein, 17 aa, synthetic construct
PSWYQQTPGQPPRTLIY

SEQ ID NO: 1327 - protein, 36 aa, synthetic construct; identical to SEQ ID NO: 1311

SEQ ID NO: 1328 - protein, 10 aa, synthetic construct
FGGGTKVTVL

SEQ ID NO: 1329 - protein, 25 aa, synthetic construct
QVQLVQSGPEVKKPGTSMKVSCKAS

SEQ ID NO: 1330 - protein, 17 aa, synthetic construct
VQWVRQARGQRLEWIGW

SEQ ID NO: 1331 - protein, 38 aa, synthetic construct
NYAQKFQERVSITRDVSKSTAYLELSSLRSEDTAVYYC

SEQ ID NO: 1332 - protein, 11 aa, synthetic construct
WGRGTMVTVSS

SEQ ID NO: 1333 - protein, 26 aa, synthetic construct
DIQMTQSPSSLSASVGDRVTITCRTS

SEQ ID NO: 1334 - protein, 17 aa, synthetic construct
LNWYQQKPGKAPNLLIY

SEQ ID NO: 1335 - protein, 36 aa, synthetic construct
SLQSGVPSRFSGSGSETDFTLTISSLQPEDFATYYC

SEQ ID NO: 1336 - protein, 10 aa, synthetic construct
FGGGTKVEIK

SEQ ID NO: 1337 - protein, 25 aa, synthetic construct
QVQLVESGGGVVQPGRSLRLSCAAS

SEQ ID NO: 1338 - protein, 17 aa, synthetic construct
MHWVRQAPGKGLEWLAV

SEQ ID NO: 1339 - protein, 38 aa, synthetic construct
YSADSVKGRFTISRDNSKNTLFLHLSGLRVEDTAVYYC

SEQ ID NO: 1340 - protein, 11 aa, synthetic construct
WGRGTTVTVSS

SEQ ID NO: 1341 - protein, 26 aa, synthetic construct
DIQMTQSPSTLSASVGDRVTITCRAS

SEQ ID NO: 1342 - protein, 17 aa, synthetic construct
LAWYQQKPGKAPKLLIY

SEQ ID NO: 1343 - protein, 36 aa, synthetic construct
NLESGVPSRFSGSGSGTEFTLTISSLQPDDFATYFC

SEQ ID NO: 1344 - protein, 10 aa, synthetic construct
FGLGTKVEIK

SEQ ID NO: 1345 - protein, 25 aa, synthetic construct
QVQLVQSGAEVKKPGSSVKVSCEAS

SEQ ID NO: 1346 - protein, 17 aa, synthetic construct
INWVRQAPGQRLEWMGS

SEQ ID NO: 1347 - protein, 38 aa, synthetic construct
DYAQKFQGRVTITADKSTSTAYMELSSLRSEDTAVYYC

SEQ ID NO: 1348 - protein, 11 aa, synthetic construct
WGQGTLVTVSS

SEQ ID NO: 1349 - protein, 25 aa, synthetic construct
QSILTQPPSVSGAPGQRVTISCTGS

SEQ ID NO: 1350 - protein, 17 aa, synthetic construct
VHWYQQLPGTAPKLLIY

SEQ ID NO: 1351 - protein, 36 aa, synthetic construct
NRPSGVPDRFSGSKSDTSASLAITGLQAEDEADYYC

SEQ ID NO: 1352 - protein, 10 aa, synthetic construct
FGGGTKLTVL

SEQ ID NO: 1353 - protein, 25 aa, synthetic construct
QVQLVQSGAEVKKPGSSVKVSCMAS

SEQ ID NO: 1354 - protein, 17 aa, synthetic construct
ISWVRQAPGQGLEWMGG

SEQ ID NO: 1355 - protein, 38 aa, synthetic construct
HYAQKFQGRVTITADESTSTAYMEVSSLRSEDTAVYYC

SEQ ID NO: 1356 - protein, 11 aa, synthetic construct
WGQGTTVTVSS

SEQ ID NO: 1357 - protein, 26 aa, synthetic construct
DIQMTQSPSTLSASVGDRVTITCRAS

SEQ ID NO: 1358 - protein, 17 aa, synthetic construct
LAWYQQKPGKVPKLLIN

SEQ ID NO: 1359 - protein, 36 aa, synthetic construct
TLESGVPSRFSGSGSGTEFTLTISSLQPDDIATYYC

SEQ ID NO: 1360 - protein, 10 aa, synthetic construct
FGQGTRLEIK

SEQ ID NO: 1361 - protein, 25 aa, synthetic construct
QRQLVQSGPEVKKPGTSVKVSCKAS

SEQ ID NO: 1362 - protein, 17 aa, synthetic construct
VQWVRQARGQRLEWIGW

SEQ ID NO: 1363 - protein, 38 aa, synthetic construct
DYAQKVQQRVTITRDTSTDTAYMELSSLRAEDTAVYYC

SEQ ID NO: 1364 - protein, 11 aa, synthetic construct
WGQGTTVTVSS

SEQ ID NO: 1365 - protein, 26 aa, synthetic construct [sequence omitted]

SEQ ID NO: 1366 - protein, 17 aa, synthetic construct
FAWYQQKPGQAPRLLIY

SEQ ID NO: 1367 - protein, 36 aa, synthetic construct
SRATGIPDRFSGSGSGTDFTLTISRLEPEDFAVYHC

SEQ ID NO: 1368 - protein, 10 aa, synthetic construct
FGQGTKVEIK

SEQ ID NO: 1369 - protein, 25 aa, synthetic construct [sequence omitted]

SEQ ID NO: 1370 - protein, 17 aa, synthetic construct
MAWVRQAPGKGLEWVAN

SEQ ID NO: 1371 - protein, 38 aa, synthetic construct
YYVDSVKGRFTISRDNAKNSLYLQMNSLRAEDTAVYYC

SEQ ID NO: 1372 - protein, 11 aa, synthetic construct
WGQGSTVTVSS

SEQ ID NO: 1373 - protein, 26 aa, synthetic construct
DIVMTQSPDSLAVSLGERATINCKSS

SEQ ID NO: 1374 - protein, 17 aa, synthetic construct
LAWYQQKAGQPPKLLIY

SEQ ID NO: 1375 - protein, 36 aa, synthetic construct
TRESGVPGRFSGSGSGTDFTLTINGLQAEDVAVYYC

SEQ ID NO: 1376 - protein, 10 aa, synthetic construct
FGQGTKVEIK

SEQ ID NO: 1377 - protein, 25 aa, synthetic construct [sequence omitted]

SEQ ID NO: 1378 - protein, 17 aa, synthetic construct
INWVRQAPGQGLEWMGG

SEQ ID NO: 1379 - protein, 38 aa, synthetic construct
NYAQKFQGRLTITADESTSTAYMELRSLRSDDTAVYYC

SEQ ID NO: 1380 - protein, 11 aa, synthetic construct
WGQGTTVTVSS

SEQ ID NO: 1381 - protein, 26 aa, synthetic construct
DIQLTQSPSFLSASVGDRVTITCRAS

SEQ ID NO: 1382 - protein, 17 aa, synthetic construct
LAWYQQKPGQAPNLLIY

SEQ ID NO: 1383 - protein, 36 aa, synthetic construct; identical to SEQ ID NO: 1175

SEQ ID NO: 1384 - protein, 10 aa, synthetic construct
FGGGTKVEIK

SEQ ID NO: 1385 - protein, 25 aa, synthetic construct
QVQLVQSGPDVKKPGTSVKVSCKAS

SEQ ID NO: 1386 - protein, 17 aa, synthetic construct
VQWVRQARGQRLEWIGW

SEQ ID NO: 1387 - protein, 38 aa, synthetic construct
EYAQRFQERVTITRDMSTSTVYMELNSLRSEDTAVYYC

SEQ ID NO: 1388 - protein, 11 aa, synthetic construct
WGQGTMVTVSS

SEQ ID NO: 1389 - protein, 25 aa, synthetic construct
QSALTQPASVSGSPGQSITISCTGT

SEQ ID NO: 1390 - protein, 17 aa, synthetic construct
VSWYQQHPGKAPKLMTY

SEQ ID NO: 1391 - protein, 36 aa, synthetic construct
NRPSGVSNRFSGSKSGNTASLTISGLQAEDETDYYC

SEQ ID NO: 1392 - protein, 10 aa, synthetic construct
FGTGTKVTVL

SEQ ID NO: 1393 - protein, 25 aa, synthetic construct
QVQLVQSGPDVKKPGTSVKVSCKAS

SEQ ID NO: 1394 - protein, 17 aa, synthetic construct
VQWVRQARGQRLEWIGW

SEQ ID NO: 1395 - protein, 38 aa, synthetic construct; identical to SEQ ID NO: 1387

SEQ ID NO: 1396 - protein, 11 aa, synthetic construct
WGQGTMVTVSS

SEQ ID NO: 1397 - protein, 26 aa, synthetic construct [sequence omitted]

SEQ ID NO: 1398 - protein, 17 aa, synthetic construct
LAWYQKKPGQAPRLLIY

SEQ ID NO: 1399 - protein, 36 aa, synthetic construct [sequence omitted]

SEQ ID NO: 1400 - protein, 10 aa, synthetic construct
FGQGTKLEIK

SEQ ID NO: 1401 - protein, 25 aa, synthetic construct
EVQLVESGGDLVQPGGSLRLSCAAS

SEQ ID NO: 1402 - protein, 17 aa, synthetic construct
MNWVRQAPGKGLEWVSV

SEQ ID NO: 1403 - protein, 38 aa, synthetic construct
FYADSVKGRFTISRHDSKNTLYLQMIGLRAEDTAVYFC

SEQ ID NO: 1404 - protein, 11 aa, synthetic construct
WGQGTTVTVSS

SEQ ID NO: 1405 - protein, 25 aa, synthetic construct
QSALTQPASVSGSPGQSITISCTGT

SEQ ID NO: 1406 - protein, 17 aa, synthetic construct
VSWYQQHPGKAPKLMTY

SEQ ID NO: 1407 - protein, 36 aa, synthetic construct; identical to SEQ ID NO: 1391

SEQ ID NO: 1408 - protein, 10 aa, synthetic construct
FGTGTKVTVL

SEQ ID NO: 1409 - protein, 25 aa, synthetic construct
EVQLVESGGDLVQPGGSLRLSCAAS

SEQ ID NO: 1410 - protein, 17 aa, synthetic construct
MNWVRQAPGKGLEWVSV

SEQ ID NO: 1411 - protein, 38 aa, synthetic construct; identical to SEQ ID NO: 1403

SEQ ID NO: 1412 - protein, 11 aa, synthetic construct
WGQGTTVTVSS

SEQ ID NO: 1413 - protein, 26 aa, synthetic construct [sequence omitted]

SEQ ID NO: 1414 - protein, 17 aa, synthetic construct
LAWYQKKPGQAPRLLIY

SEQ ID NO: 1415 - protein, 36 aa, synthetic construct [sequence omitted]

SEQ ID NO: 1416 - protein, 10 aa, synthetic construct
FGQGTKLEIK

SEQ ID NO: 1417 - protein, 25 aa, synthetic construct
EVQLVETGGGLIQPGGSLRLSCAAS

SEQ ID NO: 1418 - protein, 17 aa, synthetic construct
MNWVRQAPGKGLEWVSV

SEQ ID NO: 1419 - protein, 38 aa, synthetic construct
FYADSVRGRFTISRDNSKNTLYLQMNSLRAEDTAVYYC

SEQ ID NO: 1420 - protein, 11 aa, synthetic construct
WGRGTTVTVSS

SEQ ID NO: 1421 - protein, 26 aa, synthetic construct
DIQMTQSPSTLSASVGDRVTITCRAS

SEQ ID NO: 1422 - protein, 17 aa, synthetic construct
LAWYQQKPGKVPKLLIN

SEQ ID NO: 1423 - protein, 36 aa, synthetic construct
SLESGVPSRFSGSGSGTEFTLTISSLQPDDFATYYC

SEQ ID NO: 1424 - protein, 10 aa, synthetic construct
FGQGTRLEIK

SEQ ID NO: 1425 - protein, 25 aa, synthetic construct
EVQLVESGGGLVKPGGSLRLSCAAS

SEQ ID NO: 1426 - protein, 17 aa, synthetic construct
MNWVRQAPGKGLEWVSS

SEQ ID NO: 1427 - protein, 38 aa, synthetic construct
YYADSVKGRLTISRDNAKNSLYLQMNSLRAEDTAVYYC

SEQ ID NO: 1428 - protein, 11 aa, synthetic construct
WGKGTTVTVSS

SEQ ID NO: 1429 - protein, 26 aa, synthetic construct [sequence omitted]

SEQ ID NO: 1430 - protein, 17 aa, synthetic construct
LNWYQQKPGKAPKLLIY

SEQ ID NO: 1431 - protein, 36 aa, synthetic construct; identical to SEQ ID NO: 1303

SEQ ID NO: 1432 - protein, 10 aa, synthetic construct
FGGGTKLEIK

SEQ ID NO: 1433 - protein, 25 aa, synthetic construct
EVQLVQSGAEVKKPGESLRISCKGS

SEQ ID NO: 1434 - protein, 17 aa, synthetic construct
ISWVRQMPGKGLEWMGM

SEQ ID NO: 1435 - protein, 38 aa, synthetic construct
NYSPSFQGHVTFSADKSISTAYLQWSSLKASDTAMYYC

SEQ ID NO: 1436 - protein, 11 aa, synthetic construct
WGQGTTVTVSS

SEQ ID NO: 1437 - protein, 26 aa, synthetic construct
DIQMTQSPSTLSASVGDRVTITCRAS

SEQ ID NO: 1438 - protein, 17 aa, synthetic construct
LAWYQQKPGKVPKLLIN

SEQ ID NO: 1439 - protein, 36 aa, synthetic construct; identical to SEQ ID NO: 1423

SEQ ID NO: 1440 - protein, 10 aa, synthetic construct
FGQGTRLEIK

SEQ ID NO: 1441 - protein, 25 aa, synthetic construct [sequence omitted]

SEQ ID NO: 1442 - protein, 17 aa, synthetic construct
MNWVRQAPGKGLEWVSY

SEQ ID NO: 1443 - protein, 38 aa, synthetic construct
YYADSLKGRFTISRDNAKNSLYLQMNSLRAEDTAVYYC

SEQ ID NO: 1444 - protein, 11 aa, synthetic construct
WGQGTLVTVSS

SEQ ID NO: 1445 - protein, 25 aa, synthetic construct
QSALTQPASVSGSPGQSITISCTGS

SEQ ID NO: 1446 - protein, 17 aa, synthetic construct
VSWYQQHPGKAPKLMIY

SEQ ID NO: 1447 - protein, 36 aa, synthetic construct
KRPSGVPNRFSGSKSGNTASLTISGLQAEDEADYYC

SEQ ID NO: 1448 - protein, 10 aa, synthetic construct
FGGGTKLTVL

SEQ ID NO: 1449 - protein, 25 aa, synthetic construct [sequence omitted]

SEQ ID NO: 1450 - protein, 17 aa, synthetic construct
MHWVRQAPGQSLEWMGW

SEQ ID NO: 1451 - protein, 38 aa, synthetic construct
IYSQDFQGRVTITRDTSANTVYMELSSLRSKDAAVYYC

SEQ ID NO: 1452 - protein, 11 aa, synthetic construct
WGQGTLVTVSS

SEQ ID NO: 1453 - protein, 25 aa, synthetic construct
SYVLTQPPSVSVAPGKTARITCGEN

SEQ ID NO: 1454 - protein, 17 aa, synthetic construct
VHWYQQKPGQAPVLVIY

SEQ ID NO: 1455 - protein, 36 aa, synthetic construct
DRPSGIPERFSGSNSGNTATLTISRVEAGDEADYYC

SEQ ID NO: 1456 - protein, 10 aa, synthetic construct
FGGGTKLTVL

SEQ ID NO: 1457 - protein, 25 aa, synthetic construct
QVQLVQSGTEVKKPGASVKVSCKAS

SEQ ID NO: 1458 - protein, 17 aa, synthetic construct
MHWVRQAPGQGLEWMGI

SEQ ID NO: 1459 - protein, 38 aa, synthetic construct
SYAQKFQGRVTMTSDTSTSTVYMELSSLRSEDAAVYYC

SEQ ID NO: 1460 - protein, 11 aa, synthetic construct
WGQGTTVTVSS

SEQ ID NO: 1461 - protein, 26 aa, synthetic construct [sequence omitted]

SEQ ID NO: 1462 - protein, 17 aa, synthetic construct
LAWYQQKPGQAPRLLIY

SEQ ID NO: 1463 - protein, 36 aa, synthetic construct [sequence omitted]

SEQ ID NO: 1464 - protein, 10 aa, synthetic construct
FGGGTKVEIK

SEQ ID NO: 1465 - protein, 25 aa, synthetic construct
EVQLVESGRDLVHPGGSLRLSCAAS

SEQ ID NO: 1466 - protein, 17 aa, synthetic construct
MTWVRQAPGKGLEWVSV

SEQ ID NO: 1467 - protein, 37 aa, synthetic construct
YTDSVKGRFIISRHNSENTLYLQMNSLRAEDTAVYYC

SEQ ID NO: 1468 - protein, 11 aa, synthetic construct
WGQGTTVTVSS

SEQ ID NO: 1469 - protein, 26 aa, synthetic construct [sequence omitted]

SEQ ID NO: 1470 - protein, 17 aa, synthetic construct
LAWYQQKPGKAPNSLIY

SEQ ID NO: 1471 - protein, 36 aa, synthetic construct
SLQSGVPSRFSGSGSGTEFTLTISSLQPEDFATYYC

SEQ ID NO: 1472 - protein, 10 aa, synthetic construct
FGGGTKLEIK

SEQ ID NO: 1473 - protein, 25 aa, synthetic construct
EVQLVESGRDLVHPGGSLRLSCAAS

SEQ ID NO: 1474 - protein, 17 aa, synthetic construct
MTWVRQAPGKGLEWVSV

SEQ ID NO: 1475 - protein, 37 aa, synthetic construct; identical to SEQ ID NO: 1467

SEQ ID NO: 1476 - protein, 11 aa, synthetic construct
WGQGTTVTVSS

SEQ ID NO: 1477 - protein, 26 aa, synthetic construct
DTQLTQSPSLLSAFVGDRVTITCRAS

SEQ ID NO: 1478 - protein, 17 aa, synthetic construct
LAWYQQKPGKAPKLLIY

SEQ ID NO: 1479 - protein, 36 aa, synthetic construct; identical to SEQ ID NO: 1175

SEQ ID NO: 1480 - protein, 10 aa, synthetic construct
FGQGTRLEIK

SEQ ID NO: 1481 - protein, 25 aa, synthetic construct
EVQLVESGGSLVHPGRSLRLSCAAS

SEQ ID NO: 1482 - protein, 17 aa, synthetic construct
MHWVRQAPGKGLEWVSG

SEQ ID NO: 1483 - protein, 38 aa, synthetic construct
GYADSVRGRFTISRDNAKNSLYLQMNSLRAEDTALYYC

SEQ ID NO: 1484 - protein, 11 aa, synthetic construct
WGQGTLVTVSS

SEQ ID NO: 1485 - protein, 26 aa, synthetic construct [sequence omitted]

SEQ ID NO: 1486 - protein, 17 aa, synthetic construct
LAWYQQKPGKAPNSLIY

SEQ ID NO: 1487 - protein, 36 aa, synthetic construct; identical to SEQ ID NO: 1471

SEQ ID NO: 1488 - protein, 10 aa, synthetic construct
FGGGTKLEIK

SEQ ID NO: 1489 - protein, 25 aa, synthetic construct
EVQLVESGGSLVHPGRSLRLSCAAS

SEQ ID NO: 1490 - protein, 17 aa, synthetic construct
MHWVRQAPGKGLEWVSG

SEQ ID NO: 1491 - protein, 38 aa, synthetic construct; identical to SEQ ID NO: 1483

SEQ ID NO: 1492 - protein, 11 aa, synthetic construct
WGQGTLVTVSS

SEQ ID NO: 1493 - protein, 26 aa, synthetic construct
DTQLTQSPSLLSAFVGDRVTITCRAS

SEQ ID NO: 1494 - protein, 17 aa, synthetic construct
LAWYQQKPGKAPKLLIY

SEQ ID NO: 1495 - protein, 36 aa, synthetic construct; identical to SEQ ID NO: 1175

SEQ ID NO: 1496 - protein, 10 aa, synthetic construct
FGQGTRLEIK

SEQ ID NO: 1497 - protein, 25 aa, synthetic construct
EVYLVESGGGLVQPGGSLRLSCAVS

SEQ ID NO: 1498 - protein, 17 aa, synthetic construct
MSWVRQAPGKGLEWVST

SEQ ID NO: 1499 - protein, 38 aa, synthetic construct
FYADSVRGRFTISRDDSRNTLYLQMNSLRAEDTAVYYC

SEQ ID NO: 1500 - protein, 11 aa, synthetic construct
WGQGTLVTVSS

SEQ ID NO: 1501 - protein, 26 aa, synthetic construct [sequence omitted]

SEQ ID NO: 1502 - protein, 17 aa, synthetic construct
LAWYQQKPGKAPKLLVY

SEQ ID NO: 1503 - protein, 36 aa, synthetic construct
KLENGVPSRFSGSGSGTDYTLTINSLQPEDFATYYC

SEQ ID NO: 1504 - protein, 10 aa, synthetic construct
FGQGTKVEIK

SEQ ID NO: 1505 - protein, 25 aa, synthetic construct
QVQLVESGGGVVQPGRSLRLSCAAS

SEQ ID NO: 1506 - protein, 17 aa, synthetic construct
MHWVRQAPGKGLEWVAV

SEQ ID NO: 1507 - protein, 38 aa, synthetic construct
NYADSVKGRFTISKDSSKNTLYLQMNSLRTEDTAVYYC

SEQ ID NO: 1508 - protein, 11 aa, synthetic construct
WGQGTLVTVSS

SEQ ID NO: 1509 - protein, 26 aa, synthetic construct [sequence omitted]

SEQ ID NO: 1510 - protein, 17 aa, synthetic construct
LAWYQQKPGQAPRLLIY

SEQ ID NO: 1511 - protein, 36 aa, synthetic construct [sequence omitted]

SEQ ID NO: 1512 - protein, 10 aa, synthetic construct
FGQGTKVEIK

SEQ ID NO: 1513 - protein, 25 aa, synthetic construct
QVQLVESGGGVVQPGRSLRLSCAAS

SEQ ID NO: 1514 - protein, 17 aa, synthetic construct
MHWVRQAPGKGLEWVAV

SEQ ID NO: 1515 - protein, 38 aa, synthetic construct; identical to SEQ ID NO: 1507

SEQ ID NO: 1516 - protein, 11 aa, synthetic construct
WGQGTLVTVSS

SEQ ID NO: 1517 - protein, 26 aa, synthetic construct [sequence omitted]

SEQ ID NO: 1518 - protein, 17 aa, synthetic construct
LNWYQQKPGKAPKLLIF

SEQ ID NO: 1519 - protein, 36 aa, synthetic construct
SLQSGVPSRFSGSGSGTEFTLTISSLHPEDFATYSC

SEQ ID NO: 1520 - protein, 10 aa, synthetic construct
FGQGTKLEIK

SEQ ID NO: 1521 - protein, 25 aa, synthetic construct
EVQLVESGGGLVQPGRSLRLSCAGS

SEQ ID NO: 1522 - protein, 17 aa, synthetic construct
MHWVRQAPGRGLEWVSG

SEQ ID NO: 1523 - protein, 38 aa, synthetic construct
DYADSVKGRFTISRDNAKNSLYLQMNSLRDEDTALYYC

SEQ ID NO: 1524 - protein, 11 aa, synthetic construct
WGQGTLVTVSS

SEQ ID NO: 1525 - protein, 26 aa, synthetic construct [sequence omitted]

SEQ ID NO: 1526 - protein, 17 aa, synthetic construct
LAWYQQKPGQAPRLLIY

SEQ ID NO: 1527 - protein, 36 aa, synthetic construct [sequence omitted]

SEQ ID NO: 1528 - protein, 10 aa, synthetic construct
FGQGTKVEIK

SEQ ID NO: 1529 - protein, 25 aa, synthetic construct
EVQLVESGGGLVQPGRSLRLSCAGS

SEQ ID NO: 1530 - protein, 17 aa, synthetic construct
MHWVRQAPGRGLEWVSG

SEQ ID NO: 1531 - protein, 38 aa, synthetic construct; identical to SEQ ID NO: 1523

SEQ ID NO: 1532 - protein, 11 aa, synthetic construct
WGQGTLVTVSS

SEQ ID NO: 1533 - protein, 26 aa, synthetic construct [sequence omitted]

SEQ ID NO: 1534 - protein, 17 aa, synthetic construct
LNWYQQKPGKAPKLLIF

SEQ ID NO: 1535 - protein, 36 aa, synthetic construct; identical to SEQ ID NO: 1519

SEQ ID NO: 1536 - protein, 10 aa, synthetic construct
FGQGTKLEIK

SEQ ID NO: 1537 - protein, 25 aa, synthetic construct
QRPLLQSGPEVKKPGTSVKVSCKAS

SEQ ID NO: 1538 - protein, 17 aa, synthetic construct
VQWVRQARGQRLEWIGW

SEQ ID NO: 1539 - protein, 38 aa, synthetic construct
DYAQTFQERVTITRDMSTSTAYMELSSLRSEDTAAYYC

SEQ ID NO: 1540 - protein, 11 aa, synthetic construct
WGQGTMVTVSS

SEQ ID NO: 1541 - protein, 25 aa, synthetic construct
SYELTQPPSVSVSPGQTARITCSGD

SEQ ID NO: 1542 - protein, 17 aa, synthetic construct
AYWYQQKPGQAPVLVIY

SEQ ID NO: 1543 - protein, 36 aa, synthetic construct
ERPSGIPERLSGSSSGTTVTLTISGVQAEDEADYYC

SEQ ID NO: 1544 - protein, 10 aa, synthetic construct
FGGGTKVTVL

SEQ ID NO: 1545 - protein, 25 aa, synthetic construct
EVLLAETGGGLIQPGGSLRLSCEAS

SEQ ID NO: 1546 - protein, 17 aa, synthetic construct
MSWVRQAPGKGLEWVSV

SEQ ID NO: 1547 - protein, 38 aa, synthetic construct; identical to SEQ ID NO: 1187

SEQ ID NO: 1548 - protein, 11 aa, synthetic construct
WGKGTTVTVSS

SEQ ID NO: 1549 - protein, 25 aa, synthetic construct
QSVLTQPPSASGTPGQRVTISCSGS

SEQ ID NO: 1550 - protein, 17 aa, synthetic construct
VNWYQQLPGTAPKLLIY

SEQ ID NO: 1551 - protein, 36 aa, synthetic construct
QRPSGVPDRFSGSKSGTSASLAISGLQSEDEADYSC

SEQ ID NO: 1552 - protein, 10 aa, synthetic construct
FGGGTKLTVL

SEQ ID NO: 1553 - protein, 25 aa, synthetic construct
EVQLAESGGGLVQPGGSLRLSCAAS

SEQ ID NO: 1554 - protein, 17 aa, synthetic construct
MSWVRQAPGKGLEWVAN

SEQ ID NO: 1555 - protein, 38 aa, synthetic construct; identical to SEQ ID NO: 1371

SEQ ID NO: 1556 - protein, 11 aa, synthetic construct
WGQGTMVTVSS

SEQ ID NO: 1557 - protein, 26 aa, synthetic construct [sequence omitted]

SEQ ID NO: 1558 - protein, 17 aa, synthetic construct
LSWYQQKPGKAPKLLIH

SEQ ID NO: 1559 - protein, 36 aa, synthetic construct
SLQSGVPSRFSGGGSGTHFTLTITSLQREDFATYYC

SEQ ID NO: 1560 - protein, 10 aa, synthetic construct
FGGGTKVEIK

SEQ ID NO: 1561 - protein, 25 aa, synthetic construct [sequence omitted]

SEQ ID NO: 1562 - protein, 17 aa, synthetic construct
MNWVRQAPGKGLEWVSV

SEQ ID NO: 1563 - protein, 38 aa, synthetic construct; identical to SEQ ID NO: 1187

SEQ ID NO: 1564 - protein, 11 aa, synthetic construct
WGQGTTVTVSS

SEQ ID NO: 1565 - protein, 26 aa, synthetic construct
DIQMTQSPSTLSASVGDRVTITCRAS

SEQ ID NO: 1566 - protein, 17 aa, synthetic construct
LAWYQQKPGKAPKLLVH

SEQ ID NO: 1567 - protein, 36 aa, synthetic construct
TLESGVPSRFSGSGSGTEFTLTISSLQPDDFATYYC

SEQ ID NO: 1568 - protein, 10 aa, synthetic construct
FGQGTKVEIK

SEQ ID NO: 1569 - protein, 25 aa, synthetic construct
QVRLQESGPGLVKPSETLSLTCTVS

SEQ ID NO: 1570 - protein, 17 aa, synthetic construct
WSWIRQTPGKGLEWIGY

SEQ ID NO: 1571 - protein, 38 aa, synthetic construct
KYNPSLKSRVTISVDTAKNQFTLKLNSMTAADTAVYYC

SEQ ID NO: 1572 - protein, 11 aa, synthetic construct
WGQGTLVTVSS

SEQ ID NO: 1573 - protein, 26 aa, synthetic construct [sequence omitted]

SEQ ID NO: 1574 - protein, 17 aa, synthetic construct
LAWYQQIPGQAPRLLIY

SEQ ID NO: 1575 - protein, 36 aa, synthetic construct
NRATGIPDRFSGSGSGTDFTLTISRLEPEDFAVYYC

SEQ ID NO: 1576 - protein, 10 aa, synthetic construct
FGQGTKVEIK

SEQ ID NO: 1577 - protein, 25 aa, synthetic construct [sequence omitted]

SEQ ID NO: 1578 - protein, 17 aa, synthetic construct
ISWVRQAPGQGLEWMGR

SEQ ID NO: 1579 - protein, 38 aa, synthetic construct
NYAQKFQGRVTITADKSTSTAYMELSSLRSEDTAVYYC

SEQ ID NO: 1580 - protein, 11 aa, synthetic construct
WGQGTLVTVSS

SEQ ID NO: 1581 - protein, 25 aa, synthetic construct
QSVVTQPPSVSGAPGQRVTISCTGS

SEQ ID NO: 1582 - protein, 17 aa, synthetic construct
VHWYQHLPGTAPKLLIY

SEQ ID NO: 1583 - protein, 36 aa, synthetic construct
NRPSGVPDRFSGSKSGTSASLAITGLQAEDEADYYC

SEQ ID NO: 1584 - protein, 10 aa, synthetic construct
FGGGTKLTVL

SEQ ID NO: 1585 - protein, 25 aa, synthetic construct [sequence omitted]

SEQ ID NO: 1586 - protein, 17 aa, synthetic construct
INWVRQAPGQGLEWMGG

SEQ ID NO: 1587 - protein, 38 aa, synthetic construct
NYAQKFQDRVTITADESTSTVYMELSSLRSEDAAVYFC

SEQ ID NO: 1588 - protein, 11 aa, synthetic construct
WGQGTTVTVSS

SEQ ID NO: 1589 - protein, 26 aa, synthetic construct [sequence omitted]

SEQ ID NO: 1590 - protein, 17 aa, synthetic construct
LAWYQQIPGQAPRLLIY

SEQ ID NO: 1591 - protein, 36 aa, synthetic construct; identical to SEQ ID NO: 1575

SEQ ID NO: 1592 - protein, 10 aa, synthetic construct
FGQGTKVEIK

SEQ ID NO: 1593 - protein, 25 aa, synthetic construct [sequence omitted]

SEQ ID NO: 1594 - protein, 17 aa, synthetic construct
INWVRQAPGQGLEWMGG

SEQ ID NO: 1595 - protein, 38 aa, synthetic construct; identical to SEQ ID NO: 1587

SEQ ID NO: 1596 - protein, 11 aa, synthetic construct
WGQGTTVTVSS

SEQ ID NO: 1597 - protein, 25 aa, synthetic construct
SYVLTQPPSVSVAPGQTATVTCGDN

SEQ ID NO: 1598 - protein, 17 aa, synthetic construct
VHWYQQKPGQAPILMVF

SEQ ID NO: 1599 - protein, 36 aa, synthetic construct; identical to SEQ ID NO: 1455

SEQ ID NO: 1600 - protein, 10 aa, synthetic construct
FGGGTKLTVL

SEQ ID NO: 1601 - protein, 25 aa, synthetic construct
QVHLVESGGGVVQPGRSLRLSCAAS

SEQ ID NO: 1602 - protein, 17 aa, synthetic construct
MHWVRQAPGKGLEWVAV

SEQ ID NO: 1603 - protein, 38 aa, synthetic construct
DYADSVKGRFTISRDNSKNTLYLQMNSLRVEDTAVYYC

SEQ ID NO: 1604 - protein, 11 aa, synthetic construct
WGQGTLVTVSS

SEQ ID NO: 1605 - protein, 26 aa, synthetic construct [sequence omitted]

SEQ ID NO: 1606 - protein, 17 aa, synthetic construct
LNWFQQKPGNAPKLLIY

SEQ ID NO: 1607 - protein, 36 aa, synthetic construct
SLQSGVPSRFSGSGSGTDFTLTISSMQPEDFATYYC

SEQ ID NO: 1608 - protein, 10 aa, synthetic construct
FGQGTKVEIK

SEQ ID NO: 1609 - protein, 25 aa, synthetic construct
QVTLKESGPVLVKPTETLTLTCAVS

SEQ ID NO: 1610 - protein, 17 aa, synthetic construct
VSWIRQPPGKALEWLAH

SEQ ID NO: 1611 - protein, 38 aa, synthetic construct
SYSTSLKGRLTISKDIFKSQVVLTMTNMDPVDTATYYC

SEQ ID NO: 1612 - protein, 11 aa, synthetic construct
WGQGTLVTVSS

SEQ ID NO: 1613 - protein, 26 aa, synthetic construct [sequence omitted]

SEQ ID NO: 1614 - protein, 17 aa, synthetic construct
LGWYQQKPGKAPKRLIY

SEQ ID NO: 1615 - protein, 36 aa, synthetic construct
NLQSGVPSRFSGSGSETEFTLTISSLQPEDFATYYC

SEQ ID NO: 1616 - protein, 10 aa, synthetic construct
FGQGTKLEIK

SEQ ID NO: 1617 - protein, 25 aa, synthetic construct
EVQLVETGGGLIHPGGSLRLSCVAS

SEQ ID NO: 1618 - protein, 17 aa, synthetic construct
MSWVRQAPGKGLEWVSI

SEQ ID NO: 1619 - protein, 38 aa, synthetic construct
FYADSVKGRFTISRDNSKNTLYLQMNSLRVEDTAVYYC

SEQ ID NO: 1620 - protein, 11 aa, synthetic construct
WGQGTLVTVSS

SEQ ID NO: 1621 - protein, 25 aa, synthetic construct
SYELTQPPSVSVSPGQTASITCSGD

SEQ ID NO: 1622 - protein, 17 aa, synthetic construct
ACWYQQKPGQSPVLVIY

SEQ ID NO: 1623 - protein, 36 aa, synthetic construct
KRPSGIPERFSGSNSGNTATLTISGTQAMDEADYYC

SEQ ID NO: 1624 - protein, 10 aa, synthetic construct
FGSGTKVTVL

SEQ ID NO: 1625 - protein, 25 aa, synthetic construct
QTQLVQSGPEVKKPGTSVKVSCKAS

SEQ ID NO: 1626 - protein, 17 aa, synthetic construct
VQWVRQARGQRLEWIGW

SEQ ID NO: 1627 - protein, 38 aa, synthetic construct
NYAPKFQESVTITRDMSTSTAYMELSSLRSEDTAVYYC

SEQ ID NO: 1628 - protein, 11 aa, synthetic construct
WGQGTMVTVSS

SEQ ID NO: 1629 - protein, 26 aa, synthetic construct
EIVLAQSPGTLSLSPGERATLSCRAS

SEQ ID NO: 1630 - protein, 17 aa, synthetic construct
FAWYQQKPGQAPRLLIY

SEQ ID NO: 1631 - protein, 36 aa, synthetic construct
SRATGIPDRFSGSGSGTDFTLTISRLDPEDFAVYFC

SEQ ID NO: 1632 - protein, 10 aa, synthetic construct
FGQGTKLEIK

SEQ ID NO: 1633 - protein, 25 aa, synthetic construct
QRPLLQSGPEVKKPGTSVKVSCKAS

SEQ ID NO: 1634 - protein, 17 aa, synthetic construct
VQWVRQARGQRLEWIGW

SEQ ID NO: 1635 - protein, 38 aa, synthetic construct
DYAQTFQERVTITRDMSTSTAYMELSSLRSEDTAVYYC

SEQ ID NO: 1636 - protein, 11 aa, synthetic construct
WGQGTTVTVSS

SEQ ID NO: 1637 - protein, 26 aa, synthetic construct [sequence omitted]

SEQ ID NO: 1638 - protein, 17 aa, synthetic construct
LAWYQQIPGQAPRLLIY

SEQ ID NO: 1639 - protein, 36 aa, synthetic construct; identical to SEQ ID NO: 1575

SEQ ID NO: 1640 - protein, 10 aa, synthetic construct
FGQGTKVEIK

SEQ ID NO: 1641 - protein, 25 aa, synthetic construct
QRPLLQSGPEVKKPGTSVKVSCKAS

SEQ ID NO: 1642 - protein, 17 aa, synthetic construct
VQWVRQARGQRLEWIGW

SEQ ID NO: 1643 - protein, 38 aa, synthetic construct; identical to SEQ ID NO: 1635

SEQ ID NO: 1644 - protein, 11 aa, synthetic construct
WGQGTMVTVSS

SEQ ID NO: 1645 - protein, 26 aa, synthetic construct [sequence omitted]

SEQ ID NO: 1646 - protein, 17 aa, synthetic construct
LGWYQQKPGKAPKRLIY

SEQ ID NO: 1647 - protein, 36 aa, synthetic construct; identical to SEQ ID NO: 1615

SEQ ID NO: 1648 - protein, 10 aa, synthetic construct
FGQGTKVEIK

SEQ ID NO: 1649 - protein, 25 aa, synthetic construct
QVQLVQSGGEVRKPGASVKVSCKAS

SEQ ID NO: 1650 - protein, 17 aa, synthetic construct
ISWVRQAPGQGLEWMGW

SEQ ID NO: 1651 - protein, 38 aa, synthetic construct
NYAQKFQGRVTMTTDTSTNTAYMELRSLRSDDTAVYYC

SEQ ID NO: 1652 - protein, 11 aa, synthetic construct
WGQGTLVTVSS

SEQ ID NO: 1653 - protein, 26 aa, synthetic construct [sequence omitted]

SEQ ID NO: 1654 - protein, 17 aa, synthetic construct
LNWYQQKPGKAPKLLIH

SEQ ID NO: 1655 - protein, 36 aa, synthetic construct
SLQSGIPSRFSGSGFGTDFTLTISSLQPEDFATYYC

SEQ ID NO: 1656 - protein, 10 aa, synthetic construct
FGGGTKVEIK

SEQ ID NO: 1657 - protein, 25 aa, synthetic construct [sequence omitted]

SEQ ID NO: 1658 - protein, 17 aa, synthetic construct
MSWVRQAPGKGLEWVSL

SEQ ID NO: 1659 - protein, 38 aa, synthetic construct
FYADSVKGRFTISRDSSKNTLYLDMNTLRTEDTAVYYC

SEQ ID NO: 1660 - protein, 11 aa, synthetic construct
WGQGTTVTVSS

SEQ ID NO: 1661 - protein, 26 aa, synthetic construct
DIQLTQSPSFLSASVGDRVTITCRAS

SEQ ID NO: 1662 - protein, 17 aa, synthetic construct
LAWYQQKPGKAPKLLIY

SEQ ID NO: 1663 - protein, 36 aa, synthetic construct; identical to SEQ ID NO: 1175

SEQ ID NO: 1664 - protein, 10 aa, synthetic construct
FGQGTRLEIK

SEQ ID NO: 1665 - protein, 25 aa, synthetic construct
QMQLVQSGPEVKKPGTSVKVSCKAS

SEQ ID NO: 1666 - protein, 17 aa, synthetic construct
VQWVRQARGQRLEWIGW

SEQ ID NO: 1667 - protein, 38 aa, synthetic construct
EYAQRFQEKVTISGDMSTSTAYMELSSLRSEDTAVYYC

SEQ ID NO: 1668 - protein, 11 aa, synthetic construct
WGQGTTVTVSS

SEQ ID NO: 1669 - protein, 26 aa, synthetic construct
EIVLTQSPGTLSLSPGERASLSCRAS

SEQ ID NO: 1670 - protein, 17 aa, synthetic construct
LAWYQQKPGQAPRLLIY

SEQ ID NO: 1671 - protein, 36 aa, synthetic construct
SRATGIPDRFSGSGSGTDFTLTITRLEAEDFAVYHC

SEQ ID NO: 1672 - protein, 10 aa, synthetic construct
FGQGTKVEIK

SEQ ID NO: 1673 - protein, 25 aa, synthetic construct
EVQLVESGGGLVQPGRSLRLSCVAS

SEQ ID NO: 1674 - protein, 17 aa, synthetic construct
MHWVRQLPGKGLEWVSG

SEQ ID NO: 1675 - protein, 38 aa, synthetic construct
GYADSVKGRFIISRDNAKNSLYLQMRSLRPEDTALYYC

SEQ ID NO: 1676 - protein, 11 aa, synthetic construct
WGQGTLVTVSS

SEQ ID NO: 1677 - protein, 25 aa, synthetic construct
SYELTQPPSVSVSPGQTARITCSGD

SEQ ID NO: 1678 - protein, 17 aa, synthetic construct
AYWYQQKPGQAPVLVMY

SEQ ID NO: 1679 - protein, 36 aa, synthetic construct
QRPSGIPERFSGSNSGTAVTLTISGVQAEDEADYYC

SEQ ID NO: 1680 - protein, 10 aa, synthetic construct
FGGGTKLTVL

SEQ ID NO: 1681 - protein, 25 aa, synthetic construct
EVQLVQSGAEVKKPGEFLRISCKGS

SEQ ID NO: 1682 - protein, 17 aa, synthetic construct
ITWVRQMPGKGLEWMGK

SEQ ID NO: 1683 - protein, 38 aa, synthetic construct
IYSPSFQGHVTISADKSINTAFLQWSSLKASDTAMYYC

SEQ ID NO: 1684 - protein, 11 aa, synthetic construct
WGQGTMVTVSS

SEQ ID NO: 1685 - protein, 26 aa, synthetic construct
DIQMTQSPSTLSASVGDRVTITCRAS

SEQ ID NO: 1686 - protein, 17 aa, synthetic construct
LAWYQQKPGKAPKLLIY

SEQ ID NO: 1687 - protein, 36 aa, synthetic construct
SLENGVPSRFSGSGSGTEFTLTISSLQPDDFATYYC

SEQ ID NO: 1688 - protein, 10 aa, synthetic construct
FGQGTKLEIK

SEQ ID NO: 1689 - protein, 25 aa, synthetic construct
QRPLLQSGPEVKKPGTSVKVSCKAS

SEQ ID NO: 1690 - protein, 17 aa, synthetic construct
VQWVRQARGQRLEWIGW

SEQ ID NO: 1691 - protein, 38 aa, synthetic construct
DYAQSFQERVTITRDMSTSTAYMELSSLRSEDTAVYYC

SEQ ID NO: 1692 - protein, 11 aa, synthetic construct
WGQGTMVTVSS

SEQ ID NO: 1693 - protein, 25 aa, synthetic construct
NFMLTQPHSVSESPGKTVTISCTRS

SEQ ID NO: 1694 - protein, 17 aa, synthetic construct
VQWYQQRPGSAPTTVIY

SEQ ID NO: 1695 - protein, 38 aa, synthetic construct
QRPSGVPDRFSGSIDSSSNSASLIISGLKTEDEADYYC

SEQ ID NO: 1696 - protein, 10 aa, synthetic construct
FGGGTKLTVL

SEQ ID NO: 1697 - protein, 25 aa, synthetic construct [sequence omitted]

SEQ ID NO: 1698 - protein, 17 aa, synthetic construct
MSWVRQAPGKGLEWVSL

SEQ ID NO: 1699 - protein, 38 aa, synthetic construct
FYADSVKGRFTISRHTSENTLYLQMDSLRVEDTAVYFC

SEQ ID NO: 1700 - protein, 11 aa, synthetic construct
WGQGTLVTVSS

SEQ ID NO: 1701 - protein, 25 aa, synthetic construct
SHELTQPPSVSVSPGQTARITCSGD

SEQ ID NO: 1702 - protein, 17 aa, synthetic construct
AYWYQQKPGQAPVLVIY

SEQ ID NO: 1703 - protein, 36 aa, synthetic construct
ERPSGIPERFSGSSSGTTVTLTISGVQAEDEADYYC

SEQ ID NO: 1704 - protein, 10 aa, synthetic construct
FGGGTKLTVL

SEQ ID NO: 1705 - protein, 25 aa, synthetic construct [sequence omitted]

SEQ ID NO: 1706 - protein, 17 aa, synthetic construct
MSWVRQAPGKGLEWVSL

SEQ ID NO: 1707 - protein, 38 aa, synthetic construct
YYADSVKGRFTISRHSSENTLYLQMNSLRVEDTAVYYC

SEQ ID NO: 1708 - protein, 11 aa, synthetic construct
WGQGTLVTVSS

SEQ ID NO: 1709 - protein, 26 aa, synthetic construct [sequence omitted]

SEQ ID NO: 1710 - protein, 17 aa, synthetic construct
LNWYQHRPGKAPKLLIY

SEQ ID NO: 1711 - protein, 36 aa, synthetic construct; identical to SEQ ID NO: 1303

SEQ ID NO: 1712 - protein, 10 aa, synthetic construct
FGQGTRLEIK

SEQ ID NO: 1713 - protein, 25 aa, synthetic construct
EVQLLESGGGLVQPGGSLRLSCAAS

SEQ ID NO: 1714 - protein, 17 aa, synthetic construct
MSWVRQAPGKGLEWVSA

SEQ ID NO: 1715 - protein, 38 aa, synthetic construct
YYADSVKGRCTISRDNSENMLYLQMNSLRAEDTAVYYC

SEQ ID NO: 1716 - protein, 11 aa, synthetic construct
WGQGTTVTVSS

SEQ ID NO: 1717 - protein, 26 aa, synthetic construct [sequence omitted]

SEQ ID NO: 1718 - protein, 17 aa, synthetic construct
LNWYQHRPGKAPKLLIY

SEQ ID NO: 1719 - protein, 36 aa, synthetic construct; identical to SEQ ID NO: 1303

SEQ ID NO: 1720 - protein, 10 aa, synthetic construct
FGQGTRLEIK

SEQ ID NO: 1721 - protein, 25 aa, synthetic construct
QDQLVQSGAEVKKPGSSVRVSCKAT

SEQ ID NO: 1722 - protein, 17 aa, synthetic construct
IHWVRQAPGQGLEWMGR

SEQ ID NO: 1723 - protein, 38 aa, synthetic construct
NYAQKFQGRITITADKITTTAYMELTSLTSEDTALYYC

SEQ ID NO: 1724 - protein, 11 aa, synthetic construct
WGQGTLVTVSS

SEQ ID NO: 1725 - protein, 26 aa, synthetic construct
DIVMTQSPDSLAVSLGERATINCKSS

SEQ ID NO: 1726 - protein, 17 aa, synthetic construct
LAWYQQKPGQPPKLLIY

SEQ ID NO: 1727 - protein, 36 aa, synthetic construct; identical to SEQ ID NO: 1271

SEQ ID NO: 1728 - protein, 10 aa, synthetic construct
FGQGTKVEIK

SEQ ID NO: 1729 - protein, 25 aa, synthetic construct
EVQLLESGGGLVQPGGSLRLSCAAS

SEQ ID NO: 1730 - protein, 17 aa, synthetic construct
INWVRQAPGKGLEWVSV

SEQ ID NO: 1731 - protein, 38 aa, synthetic construct
YYADSVKGRFTISRDNSKNTLYLQMNSLRAEDTAIYYC

SEQ ID NO: 1732 - protein, 11 aa, synthetic construct
WGKGTTVTVSS

SEQ ID NO: 1733 - protein, 26 aa, synthetic construct
DIQMTQSPSSLSASVGDRVTITCRTS

SEQ ID NO: 1734 - protein, 17 aa, synthetic construct
LNWYQQKPGKAPKLLIY

SEQ ID NO: 1735 - protein, 36 aa, synthetic construct
TLQSGVPSRFSGSGSGTDFTLTISSLQPEDFATYYC

SEQ ID NO: 1736 - protein, 10 aa, synthetic construct
FGQGTRLEIK

SEQ ID NO: 1737 - protein, 25 aa, synthetic construct [sequence omitted]

SEQ ID NO: 1738 - protein, 17 aa, synthetic construct
MSWVRQAPGKGLEWVSL

SEQ ID NO: 1739 - protein, 38 aa, synthetic construct; identical to SEQ ID NO: 1699

SEQ ID NO: 1740 - protein, 11 aa, synthetic construct
WGQGTLVTVSS

SEQ ID NO: 1741 - protein, 26 aa, synthetic construct [sequence omitted]

SEQ ID NO: 1742 - protein, 17 aa, synthetic construct
LNWYQHRPGKAPKLLIY

SEQ ID NO: 1743 - protein, 36 aa, synthetic construct; identical to SEQ ID NO: 1303

SEQ ID NO: 1744 - protein, 10 aa, synthetic construct
FGQGTRLEIK

SEQ ID NO: 1745 - protein, 25 aa, synthetic construct
EVQLVESGGGVVQPGRSLRLSCAAS

SEQ ID NO: 1746 - protein, 17 aa, synthetic construct
MHWVRQAPGKGLEWVAV

SEQ ID NO: 1747 - protein, 38 aa, synthetic construct
YYADSVKGRFTISRDNSKNTVYLQMNSLSAEDTAVYYC

SEQ ID NO: 1748 - protein, 11 aa, synthetic construct
WGQGTLVTVSS

SEQ ID NO: 1749 - protein, 26 aa, synthetic construct
DIQMTQSPSTLSASVGDRVTITCRAS

SEQ ID NO: 1750 - protein, 17 aa, synthetic construct
LAWYQQKPGKAPKLLIY

SEQ ID NO: 1751 - protein, 36 aa, synthetic construct
SLDSGVPSRFSGSGSGTEFTLTISSLQPDDFATYYC

SEQ ID NO: 1752 - protein, 10 aa, synthetic construct
FGQGTKVEIK

SEQ ID NO: 1753 - protein, 25 aa, synthetic construct [sequence omitted]

SEQ ID NO: 1754 - protein, 17 aa, synthetic construct
MSWVRQAPGKGLEWVSL

SEQ ID NO: 1755 - protein, 38 aa, synthetic construct; identical to SEQ ID NO: 1699

SEQ ID NO: 1756 - protein, 11 aa, synthetic construct
WGQGTLVTVSS

SEQ ID NO: 1757 - protein, 25 aa, synthetic construct
QSVLTQPPSASGTPGQRVTISCSGS

SEQ ID NO: 1758 - protein, 17 aa, synthetic construct
VYWYQQLPGTAPKLLIY

SEQ ID NO: 1759 - protein, 36 aa, synthetic construct
QRPSGVPDRFSGSKSGTSASLAISGLRSEDEADYYC

SEQ ID NO: 1760 - protein, 10 aa, synthetic construct
FGGGTQLTVL

SEQ ID NO: 1761 - protein, 25 aa, synthetic construct [sequence omitted]

SEQ ID NO: 1762 - protein, 17 aa, synthetic construct
MHWVRQVTGKGLEWVST

SEQ ID NO: 1763 - protein, 38 aa, synthetic construct
YYLGSVKGRFTISRENGKNSLYLQMNTLRGGDTAVYYC

SEQ ID NO: 1764 - protein, 11 aa, synthetic construct
WGQGTMVTVSS

SEQ ID NO: 1765 - protein, 26 aa, synthetic construct
DIQMTQSPSTLSASIGDTVTIACRAS

SEQ ID NO: 1766 - protein, 17 aa, synthetic construct
LAWFQQKPGKAPKVLIS

SEQ ID NO: 1767 - protein, 36 aa, synthetic construct; identical to SEQ ID NO: 1423

SEQ ID NO: 1768 - protein, 10 aa, synthetic construct
FGQGTRLEIK

SEQ ID NO: 1769 - protein, 25 aa, synthetic construct
EVQLVESGGGLVKPGGSLRLSCAAS

SEQ ID NO: 1770 - protein, 17 aa, synthetic construct
MHWVRQRTGKGLEWVST

SEQ ID NO: 1771 - protein, 38 aa, synthetic construct
YYEDSVKGRFTISREDATNSLYLQMNSLRAGDTAVYYC

SEQ ID NO: 1772 - protein, 11 aa, synthetic construct
WGQGTTVTVSS

SEQ ID NO: 1773 - protein, 26 aa, synthetic construct
DIQMTQSPSSLSASVGDRVTLTCRAS

SEQ ID NO: 1774 - protein, 17 aa, synthetic construct
LNWYQHKPGKAPKLLIY

SEQ ID NO: 1775 - protein, 36 aa, synthetic construct; identical to SEQ ID NO: 1471

SEQ ID NO: 1776 - protein, 10 aa, synthetic construct
FGLGTKVEIK

SEQ ID NO: 1777 - protein, 25 aa, synthetic construct [sequence omitted]

SEQ ID NO: 1778 - protein, 17 aa, synthetic construct
ISWVRQAPGQGLEWLGR

SEQ ID NO: 1779 - protein, 38 aa, synthetic construct
NYAQKFQGRVTLTADKSTNTASMELRSLRYEDTAVYYC

SEQ ID NO: 1780 - protein, 11 aa, synthetic construct
WGQGTLVTVSS

SEQ ID NO: 1781 - protein, 26 aa, synthetic construct
DIQMTQSPSTLSASVGDRVTITCRAS

SEQ ID NO: 1782 - protein, 17 aa, synthetic construct
LAWYQQTPGKAPKLLIY

SEQ ID NO: 1783 - protein, 36 aa, synthetic construct
SLESGVPSRFSGSGSGTDFTLTISSLQPDDFATYYC

SEQ ID NO: 1784 - protein, 10 aa, synthetic construct
FGGGTKVEIK

SEQ ID NO: 1785 - protein, 25 aa, synthetic construct
EVQLVESGGGSVQPGRSLRLSCAAS

SEQ ID NO: 1786 - protein, 17 aa, synthetic construct
MHWVRQAPGKGLEWVSS

SEQ ID NO: 1787 - protein, 38 aa, synthetic construct
GYLDSVKGRFTISRDNAKNSLYLQMNILRPEDTAWYYC

SEQ ID NO: 1788 - protein, 11 aa, synthetic construct
WGQGTMVTVSS

SEQ ID NO: 1789 - protein, 26 aa, synthetic construct
DIQMTQSPSSLSASAGDRVTITCRAS

SEQ ID NO: 1790 - protein, 17 aa, synthetic construct
VNWYQQRPGRAPKLLIY

SEQ ID NO: 1791 - protein, 36 aa, synthetic construct
SLQSGVPSRFSGSGSGTDFTLTIGSLQPRDFATYYC

SEQ ID NO: 1792 - protein, 10 aa, synthetic construct
FGGGTKVEIK

SEQ ID NO: 1793 - protein, 25 aa, synthetic construct [sequence omitted]

SEQ ID NO: 1794 - protein, 17 aa, synthetic construct
MYWVRQGPGKGLEWVSG

SEQ ID NO: 1795 - protein, 38 aa, synthetic construct
MYADSVKGRFTISRDNAKNSLYLQMNSLRGEDTALYYC

SEQ ID NO: 1796 - protein, 11 aa, synthetic construct
WGQGTTVTVSS

SEQ ID NO: 1797 - protein, 26 aa, synthetic construct
ATQLTQSPSSLSASVGDGVTITCRAS

SEQ ID NO: 1798 - protein, 17 aa, synthetic construct
LAWYQQRPGRGPNLLIS

SEQ ID NO: 1799 - protein, 36 aa, synthetic construct
NLKSGVPSRFSGSGSGTDFTLTINSLQPEDFATYYC

SEQ ID NO: 1800 - protein, 10 aa, synthetic construct
FGQGTKVEIK

SEQ ID NO: 1801 - protein, 25 aa, synthetic construct
QVQLVESGGGVVQPGRSLRLSCAAS

SEQ ID NO: 1802 - protein, 17 aa, synthetic construct
FHWVRQAPGKGLEWVAL

SEQ ID NO: 1803 - protein, 38 aa, synthetic construct
FYADSVEGRFTISRDNSKNTVYLQMSSLRGEDTAVYHC

SEQ ID NO: 1804 - protein, 11 aa, synthetic construct
WGQGSLVTVSS

SEQ ID NO: 1805 - protein, 26 aa, synthetic construct [sequence omitted]

SEQ ID NO: 1806 - protein, 17 aa, synthetic construct
LNWYQHKPGKAPNLLIY

SEQ ID NO: 1807 - protein, 36 aa, synthetic construct
NLQSGVPSRFSGSGSGTDFTLTISSLQPEDFATYFC

SEQ ID NO: 1808 - protein, 10 aa, synthetic construct
FGQGTRLEIK

SEQ ID NO: 1809 - protein, 25 aa, synthetic construct
EVQLVQSGSEVKKPGESLRISCKGS

SEQ ID NO: 1810 - protein, 17 aa, synthetic construct
IGWVRQMPGKGLEWMGV

SEQ ID NO: 1811 - protein, 38 aa, synthetic construct
KYSPSFQGQVSFSADKSISTAYLQWSSLEASDTAMYYC

SEQ ID NO: 1812 - protein, 11 aa, synthetic construct
WGQGTTVTVSS

SEQ ID NO: 1813 - protein, 26 aa, synthetic construct
EIVLTQSPGTLSLSPGERASLSCRAS

SEQ ID NO: 1814 - protein, 17 aa, synthetic construct
LAWYQQKAGQAPRLLIY

SEQ ID NO: 1815 - protein, 36 aa, synthetic construct
SRATGIPDRFSGSGSGTDFTLTINRLEPEDFAVYYC

SEQ ID NO: 1816 - protein, 10 aa, synthetic construct
FGQGTKVEIK

SEQ ID NO: 1817 - protein, 25 aa, synthetic construct [sequence omitted]

SEQ ID NO: 1818 - protein, 17 aa, synthetic construct
MNWVRQAPGRGLEWVSV

SEQ ID NO: 1819 - protein, 38 aa, synthetic construct
NYADSVKGRFTISRHDSKNTLYLQMNSLRIEDTAVYYC

SEQ ID NO: 1820 - protein, 11 aa, synthetic construct
WGQGTTVTVSS

SEQ ID NO: 1821 - protein, 26 aa, synthetic construct
DIQLTQSPSFLSASVGDRVTITCRPS

SEQ ID NO: 1822 - protein, 17 aa, synthetic construct
LAWYQQKPGKAPKLLIY

SEQ ID NO: 1823 - protein, 36 aa, synthetic construct
TLQSGVPSRFSGSGSGTEFTLTISSLQPEDFATYFC

SEQ ID NO: 1824 - protein, 10 aa, synthetic construct
FGGGTKVEIK

SEQ ID NO: 1825 - protein, 25 aa, synthetic construct
QVQLVESGGGVVQPGRSLRLSCAAS

SEQ ID NO: 1826 - protein, 17 aa, synthetic construct
MHWVRQAPGKGLEWVAV

SEQ ID NO: 1827 - protein, 38 aa, synthetic construct
YYADSVKGRFTLSRDNSKNTLYLQMNSLRAEDTAFYYC

SEQ ID NO: 1828 - protein, 11 aa, synthetic construct
WGQGTLVTVSS

SEQ ID NO: 1829 - protein, 26 aa, synthetic construct
DIVMTQTPLSLPVTPGEPASISCRSS

SEQ ID NO: 1830 - protein, 17 aa, synthetic construct
LDWYLQKPGQSPQLLIY

SEQ ID NO: 1831 - protein, 36 aa, synthetic construct
YRASGVPDRFSGSGSGTDFTLKISRVEAEDVGVYYC

SEQ ID NO: 1832 - protein, 10 aa, synthetic construct
FGQGTKLEIK

SEQ ID NO: 1833 - protein, 25 aa, synthetic construct
EVQLVESGGHLVQPGGSLRLSCAAS

SEQ ID NO: 1834 - protein, 17 aa, synthetic construct
MNWVRQAPGKGLEWVSV

SEQ ID NO: 1835 - protein, 38 aa, synthetic construct
FYADSVKGRFTISRHNSNNTLYLQMNSLRAEDTAVYYC

SEQ ID NO: 1836 - protein, 11 aa, synthetic construct
WGQGTTVTVSS

SEQ ID NO: 1837 - protein, 26 aa, synthetic construct
DIQLTQSPSFLSASIGDRVTITCRAS

SEQ ID NO: 1838 - protein, 17 aa, synthetic construct
LAWYQQKPGKAPKLLIY

SEQ ID NO: 1839 - protein, 36 aa, synthetic construct; identical to SEQ ID NO: 1175

SEQ ID NO: 1840 - protein, 10 aa, synthetic construct
FGQGTRLEIK

SEQ ID NO: 1841 - protein, 25 aa, synthetic construct
EVQLVESGGHLVQPGGSLRLSCAAS

SEQ ID NO: 1842 - protein, 17 aa, synthetic construct
MNWVRQAPGKGLEWVSV

SEQ ID NO: 1843 - protein, 38 aa, synthetic construct; identical to SEQ ID NO: 1835

SEQ ID NO: 1844 - protein, 11 aa, synthetic construct
WGQGTTVTVSS

SEQ ID NO: 1845 - protein, 25 aa, synthetic construct
QSALTQPPSASGSPGQSVTISCTGT

SEQ ID NO: 1846 - protein, 17 aa, synthetic construct
VSWYQQFPGKAPKLMIY

SEQ ID NO: 1847 - protein, 36 aa, synthetic construct; identical to SEQ ID NO: 1159

SEQ ID NO: 1848 - protein, 10 aa, synthetic construct
FGGGTKLTVL

SEQ ID NO: 1849 - protein, 25 aa, synthetic construct [sequence omitted]

SEQ ID NO: 1850 - protein, 17 aa, synthetic construct
MNWVRQAPGKGLEWVSL

SEQ ID NO: 1851 - protein, 38 aa, synthetic construct
FYADSVKGRFTVSRDNSKNTLYLQMNSLRPEDTAVYYC

SEQ ID NO: 1852 - protein, 11 aa, synthetic construct
WGQGTTVTVSS

SEQ ID NO: 1853 - protein, 26 aa, synthetic construct
DIQLTQSPSFLSASVGDRVTITCRAS

SEQ ID NO: 1854 - protein, 17 aa, synthetic construct
LAWYQQKPGKAPKLLIY

SEQ ID NO: 1855 - protein, 36 aa, synthetic construct
TLQSGVPSRFTGSGSGTEFTLTISSLQPEDFATYYC

SEQ ID NO: 1856 - protein, 10 aa, synthetic construct
FGGGTKVEIK

SEQ ID NO: 1857 - protein, 25 aa, synthetic construct [sequence omitted]

SEQ ID NO: 1858 - protein, 17 aa, synthetic construct
MHWVRQVIGKGLEWVSF

SEQ ID NO: 1859 - protein, 38 aa, synthetic construct
YYAGSVKGRFTISRENAKNSLYLQMNSLRAGDTALYYC

SEQ ID NO: 1860 - protein, 11 aa, synthetic construct
WGQGTTVTVSS

SEQ ID NO: 1861 - protein, 26 aa, synthetic construct
DIQMTQSPSSLSASVGDRVTITCQAS

SEQ ID NO: 1862 - protein, 17 aa, synthetic construct
LNWYQQKPGKAPNLLIY

SEQ ID NO: 1863 - protein, 36 aa, synthetic construct
NLETGVPSRFSGSGSGTDFTLTISSLQPEDIATYYC

SEQ ID NO: 1864 - protein, 10 aa, synthetic construct
FGGGTKVEIK

SEQ ID NO: 1865 - protein, 25 aa, synthetic construct
QVQLAQAGAEVKKPGASVKVSCKAS

SEQ ID NO: 1866 - protein, 17 aa, synthetic construct
IHWVRQAPGQGLEWMGI

SEQ ID NO: 1867 - protein, 38 aa, synthetic construct
SYALKFQGRVTVTSDTSTSTVYMELSSLTSEDTAVYYC

SEQ ID NO: 1868 - protein, 11 aa, synthetic construct
WGKGTTVTVSS

SEQ ID NO: 1869 - protein, 26 aa, synthetic construct
DIQMTQSPSSLSASVGDRVTITCQAS

SEQ ID NO: 1870 - protein, 17 aa, synthetic construct
LNWYQQKPGKAPNLLIY

SEQ ID NO: 1871 - protein, 36 aa, synthetic construct; identical to SEQ ID NO: 1863

SEQ ID NO: 1872 - protein, 10 aa, synthetic construct
FGGGTKVEIK

SEQ ID NO: 1873 - protein, 25 aa, synthetic construct
QVQLAQAGAEVKKPGASVKVSCKAS

SEQ ID NO: 1874 - protein, 17 aa, synthetic construct
IHWVRQAPGQGLEWMGI

SEQ ID NO: 1875 - protein, 38 aa, synthetic construct; identical to SEQ ID NO: 1867

SEQ ID NO: 1876 - protein, 11 aa, synthetic construct
WGKGTTVTVSS

SEQ ID NO: 1877 - protein, 25 aa, synthetic construct
SYVLTQAPSVSVAPGRTARITCGAD

SEQ ID NO: 1878 - protein, 17 aa, synthetic construct
VHWYQQKPGQAPVLVVY

SEQ ID NO: 1879 - protein, 36 aa, synthetic construct
VRPSGIPERFSGSNSGSTATLTISRVDSGDEADYYC

SEQ ID NO: 1880 - protein, 10 aa, synthetic construct
FGSGTKVTVL

SEQ ID NO: 1881 - protein, 25 aa, synthetic construct
EVQLVESGGHLVQPGGSLRLSCAAS

SEQ ID NO: 1882 - protein, 17 aa, synthetic construct
MNWVRQAPGKGLEWVSV

SEQ ID NO: 1883 - protein, 38 aa, synthetic construct; identical to SEQ ID NO: 1835

SEQ ID NO: 1884 - protein, 11 aa, synthetic construct
WGQGTTVTVSS

SEQ ID NO: 1885 - protein, 26 aa, synthetic construct
DIQMTQSPSSLSASVGDRVTITCQAS

SEQ ID NO: 1886 - protein, 17 aa, synthetic construct
LNWYQQKPGKAPNLLIY

SEQ ID NO: 1887 - protein, 36 aa, synthetic construct; identical to SEQ ID NO: 1863

SEQ ID NO: 1888 - protein, 10 aa, synthetic construct
FGGGTKVEIK

SEQ ID NO: 1889 - protein, 25 aa, synthetic construct
QVQLQESGPGLVKPSATLSLTCTVS

SEQ ID NO: 1890 - protein, 17 aa, synthetic construct
WSWIRQPPGKGLEWIGY

SEQ ID NO: 1891 - protein, 38 aa, synthetic construct
NYNPSLKSRVTISVDTSKNQFSLKLRSVTAADTAMYYC

SEQ ID NO: 1892 - protein, 11 aa, synthetic construct
WGQGTLVTVSS

SEQ ID NO: 1893 - protein, 26 aa, synthetic construct
DIQLTQSPSSLSASVGDRVTITCQAS

SEQ ID NO: 1894 - protein, 17 aa, synthetic construct
LNWYQQKSGKAPKLLIY

SEQ ID NO: 1895 - protein, 36 aa, synthetic construct
NLEAGVPSRFSGSGSGPDFTLIISSLQPEDIATYYC

SEQ ID NO: 1896 - protein, 10 aa, synthetic construct
FGQGTRLEIK

SEQ ID NO: 1897 - protein, 25 aa, synthetic construct [sequence omitted]

SEQ ID NO: 1898 - protein, 17 aa, synthetic construct
VNWVRQAPGQGLEWMGR

SEQ ID NO: 1899 - protein, 38 aa, synthetic construct
SYAQKFQGRVTITADKSTSTAYMELSSLTSEDTAVYYC

SEQ ID NO: 1900 - protein, 11 aa, synthetic construct
WGQGTTVTVSS

SEQ ID NO: 1901 - protein, 26 aa, synthetic construct [sequence omitted]

SEQ ID NO: 1902 - protein, 17 aa, synthetic construct
LVWYQQKPGKVPKVLIY

SEQ ID NO: 1903 - protein, 36 aa, synthetic construct
TLQSGVPSRFSGSGSGTDFTLTINSLQPEDVATYYC

SEQ ID NO: 1904 - protein, 10 aa, synthetic construct
FGGGTKVEIK

SEQ ID NO: 1905 - protein, 25 aa, synthetic construct
QVQLVESGGGVVQPGRSLRLSCAAD

SEQ ID NO: 1906 - protein, 17 aa, synthetic construct
MHWVRQAPGKGLEWLAV

SEQ ID NO: 1907 - protein, 38 aa, synthetic construct
YYADSVKGRFTISRDNSKNTLYLQMNSLRADDTAVYYC

SEQ ID NO: 1908 - protein, 11 aa, synthetic construct
WGQGTMVTVSS

SEQ ID NO: 1909 - protein, 25 aa, synthetic construct
SYVLTQPPSVSVAPGKTARITCGGN

SEQ ID NO: 1910 - protein, 17 aa, synthetic construct
VHWCRQKPGQAPVLVVY

SEQ ID NO: 1911 - protein, 36 aa, synthetic construct
DRPSGIPERFSGSNSGSTATLTISRVEAGDEADYFC

SEQ ID NO: 1912 - protein, 10 aa, synthetic construct
FGGGTKLTVL

SEQ ID NO: 1913 - protein, 25 aa, synthetic construct
QVQLVESGGGVVQPGGSLRLSCAAS

SEQ ID NO: 1914 - protein, 17 aa, synthetic construct
MHWIRQAPGKGLEWVAI

SEQ ID NO: 1915 - protein, 38 aa, synthetic construct
YYADSVKGRFTVSRDNSSNTLYLQINSLRPEDTAVYYC

SEQ ID NO: 1916 - protein, 11 aa, synthetic construct
WGQGTTVTVSS

SEQ ID NO: 1917 - protein, 26 aa, synthetic construct
DIQMTQSPSSLSASVGDRVTLTCRAS

SEQ ID NO: 1918 - protein, 17 aa, synthetic construct
LNWYQQRPGKAPELLIY

SEQ ID NO: 1919 - protein, 36 aa, synthetic construct
SLQSGVPSRFSGSGSATDFTLTISSLQPEDFATYYC

SEQ ID NO: 1920 - protein, 10 aa, synthetic construct
FGQGTKLEIK

SEQ ID NO: 1921 - protein, 25 aa, synthetic construct
QVQLQESGPGLVKPSGTLSLTCSVS

SEQ ID NO: 1922 - protein, 17 aa, synthetic construct
WSWIRQPPGKGLEWLGY

SEQ ID NO: 1923 - protein, 38 aa, synthetic construct
NYNPSLKSRVTIAVDTSKNHFSLRLTSVTAADTAVYFC

SEQ ID NO: 1924 - protein, 11 aa, synthetic construct
WGQGTMVTVSS

SEQ ID NO: 1925 - protein, 25 aa, synthetic construct
QSALTQPASVSGSPGQSITISCTGS

SEQ ID NO: 1926 - protein, 17 aa, synthetic construct
LSWYQQHPGKAPKLMIY

SEQ ID NO: 1927 - protein, 36 aa, synthetic construct
NRPSGISNRFSGSKSGNTASLTISGLQAEDEADYYC

SEQ ID NO: 1928 - protein, 10 aa, synthetic construct
FGGGTKLTVL

SEQ ID NO: 1929 - protein, 25 aa, synthetic construct
QVQLVQSGAEVKKSGSSVKVSCKAS

SEQ ID NO: 1930 - protein, 17 aa, synthetic construct
ISWVRQAPGQGLEWMGG

SEQ ID NO: 1931 - protein, 38 aa, synthetic construct
TYAQKFQGRVTITADRSTSTAYMELNSLRSEDTAVYYC

SEQ ID NO: 1932 - protein, 11 aa, synthetic construct
WGKGTTVTVSS

SEQ ID NO: 1933 - protein, 26 aa, synthetic construct
EIVMTQSPATLSVSPGERVTLSCRAS

SEQ ID NO: 1934 - protein, 17 aa, synthetic construct
LAWYQQKPGQAPRLLIY

SEQ ID NO: 1935 - protein, 36 aa, synthetic construct
TRATGIPARFSGSGSGTEFTFTIGSLQSEDFAVYYC

SEQ ID NO: 1936 - protein, 10 aa, synthetic construct
FGQGTKVEIK

SEQ ID NO: 1937 - protein, 25 aa, synthetic construct
EVQLVESGGGLVQPGRSLRLSCTAS

SEQ ID NO: 1938 - protein, 17 aa, synthetic construct
MNWVRQAPGKGLEWVSS

SEQ ID NO: 1939 - protein, 38 aa, synthetic construct
DYADSVKGRFTISRDNAKNSLYLQMNSLRAEDTALYYC

SEQ ID NO: 1940 - protein, 11 aa, synthetic construct
WGQGTTVTVSS

SEQ ID NO: 1941 - protein, 26 aa, synthetic construct
DIVMTQSPDSLAVSLGERATINCKSS

SEQ ID NO: 1942 - protein, 17 aa, synthetic construct
IAWYQQKPGQPPKLLIY

SEQ ID NO: 1943 - protein, 36 aa, synthetic construct
TRESGVPDRFSGSGSGTDFTLTISSLQAEDVAVYHC

SEQ ID NO: 1944 - protein, 10 aa, synthetic construct
FGGGTKVEIK

SEQ ID NO: 1945 - protein, 25 aa, synthetic construct
EVQLVESGGGLVQPGRSLRLSCTAS

SEQ ID NO: 1946 - protein, 17 aa, synthetic construct
MNWVRQAPGKGLEWVSS

SEQ ID NO: 1947 - protein, 38 aa, synthetic construct; identical to SEQ ID NO: 1939

SEQ ID NO: 1948 - protein, 11 aa, synthetic construct
WGQGTTVTVSS

SEQ ID NO: 1949 - protein, 25 aa, synthetic construct
QSALTQPPSASGSLGQSVTISCTGT

SEQ ID NO: 1950 - protein, 17 aa, synthetic construct
VSWYRQHPGKAPKLMIY

SEQ ID NO: 1951 - protein, 36 aa, synthetic construct
ERPSGVPDRFSGSKSGNTASLTVSGLQAEDEADYYC

SEQ ID NO: 1952 - protein, 10 aa, synthetic construct
FGGGTKLTVL

SEQ ID NO: 1953 - protein, 25 aa, synthetic construct
QVQLVQSGAEVKKSGSSVKVSCKAS

SEQ ID NO: 1954 - protein, 17 aa, synthetic construct
ISWVRQAPGQGLEWMGG

SEQ ID NO: 1955 - protein, 38 aa, synthetic construct; identical to SEQ ID NO: 1931

SEQ ID NO: 1956 - protein, 11 aa, synthetic construct
WGKGTTVTVSS

SEQ ID NO: 1957 - protein, 26 aa, synthetic construct
DIVMTQSPDSLAVSLGERATINCKSS

SEQ ID NO: 1958 - protein, 17 aa, synthetic construct
LAWYQQKPGQPPKLLIY

SEQ ID NO: 1959 - protein, 36 aa, synthetic construct; identical to SEQ ID NO: 1271

SEQ ID NO: 1960 - protein, 10 aa, synthetic construct
FGGGTKVEIK

SEQ ID NO: 1961 - protein, 25 aa, synthetic construct
QVQLVQSGAEVKKSGSSVKVSCKAS

SEQ ID NO: 1962 - protein, 17 aa, synthetic construct
ISWVRQAPGQGLEWMGG

SEQ ID NO: 1963 - protein, 38 aa, synthetic construct; identical to SEQ ID NO: 1931

SEQ ID NO: 1964 - protein, 11 aa, synthetic construct
WGKGTTVTVSS

SEQ ID NO: 1965 - protein, 25 aa, synthetic construct
NFILTQPHSVSASPGKTVTISCTGN

SEQ ID NO: 1966 - protein, 17 aa, synthetic construct
VHWYQQRPGSAPTTIIY

SEQ ID NO: 1967 - protein, 38 aa, synthetic construct; identical to SEQ ID NO: 1167

SEQ ID NO: 1968 - protein, 10 aa, synthetic construct
FGGGTKLTVL

SEQ ID NO: 1969 - protein, 25 aa, synthetic construct [sequence omitted]

SEQ ID NO: 1970 - protein, 17 aa, synthetic construct
MHWVRQAPGQGLEWMGR

SEQ ID NO: 1971 - protein, 38 aa, synthetic construct; identical to SEQ ID NO: 1155

SEQ ID NO: 1972 - protein, 11 aa, synthetic construct
WGKGTTVTVSS

SEQ ID NO: 1973 - protein, 26 aa, synthetic construct
DIVMTQSPDSLAVSLGERATINCKSS

SEQ ID NO: 1974 - protein, 17 aa, synthetic construct
LAWYQQKPGQPPKLLIY

SEQ ID NO: 1975 - protein, 36 aa, synthetic construct; identical to SEQ ID NO: 1271

SEQ ID NO: 1976 - protein, 10 aa, synthetic construct
FGGGTKVEIK

SEQ ID NO: 1977 - protein, 25 aa, synthetic construct
QVQLQQWGAGLLKPSETLSLTCTVS

SEQ ID NO: 1978 - protein, 17 aa, synthetic construct
WSWIRQPPGKGLEWIGE

SEQ ID NO: 1979 - protein, 38 aa, synthetic construct
NYKPSLKSRVTITLDTSENQFSLKLSSVTAADTAVYYC

SEQ ID NO: 1980 - protein, 11 aa, synthetic construct
WGHGTLVTVSS

SEQ ID NO: 1981 - protein, 26 aa, synthetic construct
DIVMTQSPDSLAVSLGERATINCKSS

SEQ ID NO: 1982 - protein, 17 aa, synthetic construct
LAWYQQKPGQPPKLLIY

SEQ ID NO: 1983 - protein, 36 aa, synthetic construct; identical to SEQ ID NO: 1271

SEQ ID NO: 1984 - protein, 10 aa, synthetic construct
FGQGTKVEIK

SEQ ID NO: 1985 - protein, 25 aa, synthetic construct
QVQLVQSGAEVKKSGSSVKVSCKAS

SEQ ID NO: 1986 - protein, 17 aa, synthetic construct
ISWVRQAPGQGLEWMGG

SEQ ID NO: 1987 - protein, 38 aa, synthetic construct; identical to SEQ ID NO: 1931

SEQ ID NO: 1988 - protein, 11 aa, synthetic construct
WGKGTTVTVSS

SEQ ID NO: 1989 - protein, 26 aa, synthetic construct [sequence omitted]

SEQ ID NO: 1990 - protein, 17 aa, synthetic construct
LAWFQQKPGKAPKSLIY

SEQ ID NO: 1991 - protein, 36 aa, synthetic construct
SLQIGVPSRFSGSGSGTHFTLTISSLHPEDFATYYC

SEQ ID NO: 1992 - protein, 10 aa, synthetic construct
FGQGTKVEIK

SEQ ID NO: 1993 - protein, 25 aa, synthetic construct
EVQLVQSGAEVKKPGESLRISCKGS

SEQ ID NO: 1994 - protein, 17 aa, synthetic construct
ISWVRQMPGKGLEWMGK

SEQ ID NO: 1995 - protein, 38 aa, synthetic construct
NYSPSFQGHVTISVDRSISTAYLQWSSLKASDTAMYYC

SEQ ID NO: 1996 - protein, 11 aa, synthetic construct
WGQGTLVTVSS

SEQ ID NO: 1997 - protein, 26 aa, synthetic construct
DIVMTQSPDSLAVSLGERATINCKSS

SEQ ID NO: 1998 - protein, 17 aa, synthetic construct
LAWYQQKPGQPPKLLIY

SEQ ID NO: 1999 - protein, 36 aa, synthetic construct; identical to SEQ ID NO: 1271

SEQ ID NO: 2000 - protein, 10 aa, synthetic construct
FGGGTKVEIK

SEQ ID NO: 2001 - protein, 25 aa, synthetic construct
QVQLVESGGGVVQPGRSLRLSCAAS

SEQ ID NO: 2002 - protein, 17 aa, synthetic construct
MHWVRQAPGKGLEWVAL

SEQ ID NO: 2003 - protein, 38 aa, synthetic construct
YYADSVKGRFTISRDNSKNTLYLQVNSLRAEDTAVYYC

SEQ ID NO: 2004 - protein, 11 aa, synthetic construct
WGQGTMVTVSS

SEQ ID NO: 2005 - protein, 26 aa, synthetic construct [sequence omitted]

SEQ ID NO: 2006 - protein, 17 aa, synthetic construct
LAWYQQKPGQAPRLLIS

SEQ ID NO: 2007 - protein, 36 aa, synthetic construct
SRAAGIPDRFSGSGSGTDFTLTINRLEPEDFAVYYC

SEQ ID NO: 2008 - protein, 10 aa, synthetic construct
FGGGTKVEIK

SEQ ID NO: 2009 - protein, 25 aa, synthetic construct
EVQLVESGGGLVQPGGSLRLSCVAS

SEQ ID NO: 2010 - protein, 17 aa, synthetic construct
MNWVRQAPGKGLEWVSY

SEQ ID NO: 2011 - protein, 38 aa, synthetic construct
YYADSVKGRFTISRDNAKNSLYMQMNSLRDEDTAVYYC

SEQ ID NO: 2012 - protein, 11 aa, synthetic construct
WGKGTTVTVSS

SEQ ID NO: 2013 - protein, 26 aa, synthetic construct
EIVMTQSPATLSVSPGERATLSCRAS

SEQ ID NO: 2014 - protein, 17 aa, synthetic construct
LAWYQQKPGQAPRLLIY

SEQ ID NO: 2015 - protein, 36 aa, synthetic construct
TRATGIPARFSGSGSGTEFTLTISSLQSEDFAVYYC

SEQ ID NO: 2016 - protein, 10 aa, synthetic construct
FGGGTKVEIK

SEQ ID NO: 2017 - protein, 25 aa, synthetic construct [sequence omitted]

SEQ ID NO: 2018 - protein, 17 aa, synthetic construct
MSWVRQAPGKGLEWVSV

SEQ ID NO: 2019 - protein, 38 aa, synthetic construct
YYADSVKGRFTISRDNSKNTLYLQMNSLRAEDTAMYYC

SEQ ID NO: 2020 - protein, 11 aa, synthetic construct
WGQGTLVTVSS

SEQ ID NO: 2021 - protein, 26 aa, synthetic construct
DIQLTQSPSFLSASVGDRVTITCRAS

SEQ ID NO: 2022 - protein, 17 aa, synthetic construct
LAWYQQKPGKAPKLLIY

SEQ ID NO: 2023 - protein, 36 aa, synthetic construct
TLQSGVPSRFSGSGSGTEFTLTISSLQPEDFASYYC

SEQ ID NO: 2024 - protein, 10 aa, synthetic construct
FGQGTKLEIK

SEQ ID NO: 2025 - protein, 25 aa, synthetic construct
EVQLVESGGGLVQPGGSLRLSCVAS

SEQ ID NO: 2026 - protein, 17 aa, synthetic construct
MNWVRQAPGKGLEWVSY

SEQ ID NO: 2027 - protein, 38 aa, synthetic construct; identical to SEQ ID NO: 2011

SEQ ID NO: 2028 - protein, 11 aa, synthetic construct
WGKGTTVTVSS

SEQ ID NO: 2029 - protein, 26 aa, synthetic construct [sequence omitted]

SEQ ID NO: 2030 - protein, 17 aa, synthetic construct
LAWYQQKAGQAPRLLIY

SEQ ID NO: 2031 - protein, 36 aa, synthetic construct
SRATGIPDRFSGSGSGTDFSLIISRLEPEDFAVYYC

SEQ ID NO: 2032 - protein, 10 aa, synthetic construct
FGQGTKVEIK

SEQ ID NO: 2033 - protein, 25 aa, synthetic construct
QVQLVESGGGVVQPGGSLRLSCAAS

SEQ ID NO: 2034 - protein, 17 aa, synthetic construct
MHWVRQAPGKGLEWVAF

SEQ ID NO: 2035 - protein, 38 aa, synthetic construct; identical to SEQ ID NO: 1243

SEQ ID NO: 2036 - protein, 11 aa, synthetic construct
WGKGTTVTVSS

SEQ ID NO: 2037 - protein, 26 aa, synthetic construct [sequence omitted]

SEQ ID NO: 2038 - protein, 17 aa, synthetic construct
LAWYQQKPGQAPRLLIY

SEQ ID NO: 2039 - protein, 36 aa, synthetic construct; identical to SEQ ID NO: 2031

SEQ ID NO: 2040 - protein, 10 aa, synthetic construct
FGQGTKVEIK

SEQ ID NO: 2041 - protein, 25 aa, synthetic construct
EVQLVESGGGLTQPGGSLRLSCAAS

SEQ ID NO: 2042 - protein, 17 aa, synthetic construct
MNWVRQAPGKGLEWVSA

SEQ ID NO: 2043 - protein, 38 aa, synthetic construct
YYADSVKGRFTISRDNSKNTLFLQMNSLRAEDTAVYYC

SEQ ID NO: 2044 - protein, 11 aa, synthetic construct
WGKGTTVTVSS

SEQ ID NO: 2045 - protein, 26 aa, synthetic construct
EIVMTQSPATLSVSPGERATLSCRAS

SEQ ID NO: 2046 - protein, 17 aa, synthetic construct
LAWYQQKPGQAPRLLIY

SEQ ID NO: 2047 - protein, 36 aa, synthetic construct; identical to SEQ ID NO: 2015

SEQ ID NO: 2048 - protein, 10 aa, synthetic construct
FGGGTKVEIK

SEQ ID NO: 2049 - protein, 25 aa, synthetic construct
EVQLVESGGGLVKPGGSLRLSCAAS

SEQ ID NO: 2050 - protein, 17 aa, synthetic construct
MNWVRQAPGKGLEWVSS

SEQ ID NO: 2051 - protein, 38 aa, synthetic construct
YYADSVKGRFTISRDNAKNSLYLQMSSLRAEDTAVYYC

SEQ ID NO: 2052 - protein, 11 aa, synthetic construct
WGQGTLVTVSS

SEQ ID NO: 2053 - protein, 26 aa, synthetic construct [sequence omitted]

SEQ ID NO: 2054 - protein, 17 aa, synthetic construct
LAWYQQKPGQAPRLLIY

SEQ ID NO: 2055 - protein, 36 aa, synthetic construct [sequence omitted]

SEQ ID NO: 2056 - protein, 10 aa, synthetic construct
FGQGTKVEIK

SEQ ID NO: 2057 - protein, 25 aa, synthetic construct
EVQLVESGGGLTQPGGSLRLSCAAS

SEQ ID NO: 2058 - protein, 17 aa, synthetic construct
MNWVRQAPGKGLEWVSA

SEQ ID NO: 2059 - protein, 38 aa, synthetic construct; identical to SEQ ID NO: 2043

SEQ ID NO: 2060 - protein, 11 aa, synthetic construct
WGKGTTVTVSS

SEQ ID NO: 2061 - protein, 25 aa, synthetic construct
QSVLTQPPSASGTPGQRVTISCSGS

SEQ ID NO: 2062 - protein, 17 aa, synthetic construct
VNWYQQLPGTAPKLLIY

SEQ ID NO: 2063 - protein, 36 aa, synthetic construct
QRPSGVPDRFSGSKSGTSASLAISGLQSEDEADYYC

SEQ ID NO: 2064 - protein, 10 aa, synthetic construct
FGTGTKVTVL

SEQ ID NO: 2065 - protein, 25 aa, synthetic construct
EVQLVESGGGLTQPGGSLRLSCAAS

SEQ ID NO: 2066 - protein, 17 aa, synthetic construct
MNWVRQAPGKGLEWVSA

SEQ ID NO: 2067 - protein, 38 aa, synthetic construct; identical to SEQ ID NO: 2043

SEQ ID NO: 2068 - protein, 11 aa, synthetic construct
WGKGTTVTVSS

SEQ ID NO: 2069 - protein, 26 aa, synthetic construct
DIQMTQSPSSLSASVGDRVTITCQAS

SEQ ID NO: 2070 - protein, 17 aa, synthetic construct
LNWYQQKPGKAPKLLIY

SEQ ID NO: 2071 - protein, 36 aa, synthetic construct
NLETGVPSRFSGSGSGTDFTFTISSLQPEDIATYYC

SEQ ID NO: 2072 - protein, 10 aa, synthetic construct
FGGGTKVEIK

SEQ ID NO: 2073 - protein, 25 aa, synthetic construct
QVQLVESGGGVVQPGRSLRLSCATS

SEQ ID NO: 2074 - protein, 17 aa, synthetic construct
MHWVRQAPGKGLEWVAV

SEQ ID NO: 2075 - protein, 38 aa, synthetic construct
YYADSVKGRFTISRDNSENTLYLQMNSLRAQDTAVYFC

SEQ ID NO: 2076 - protein, 11 aa, synthetic construct
WGRGTTVTVSS

SEQ ID NO: 2077 - protein, 25 aa, synthetic construct
QSVLTQPPSASGTPGQRVTISCSGS

SEQ ID NO: 2078 - protein, 17 aa, synthetic construct
VNWYQQLPGTAPKLLIY

SEQ ID NO: 2079 - protein, 36 aa, synthetic construct; identical to SEQ ID NO: 2063

SEQ ID NO: 2080 - protein, 10 aa, synthetic construct
FGGGTKLTVL

SEQ ID NO: 2081 - protein, 3780 aa, SARS-CoV-2
METPHEVALPHELEUVALLEULEUPROLEUVALSERSERGLNCYSVALASNLEUTHRTHRARGTHRGLNLEUPROPROALATYRTHRASNSERPHETHRARGGLYVALTYRTYRPROASPLYSVALPHEARGSERSERVALLEUHISSERTHRGLNASPLEUPHELEUPROPHEPHESERASNVALTHRTRPPHEHISALAILEHISVALSERGLYTHRASNGLYTHRLYSARGPHEASPASNPROVALLEUPROPHEASNASPGLYVALTYRPHEALASERTHRGLULYSSERASNILEILEARGGLYTRPILEPHEGLYTHRTHRLEUASPSERLYSTHRGLNSERLEULEUILEVALASNASNALATHRASNVALVALILELYSVALCYSGLUPHEGLNPHECYSASNASPPROPHELEUGLYVALTYRTYRHISLYSASNASNLYSSERTRPMETGLUSERGLUPHEARGVALTYRSERSERALAASNASNCYSTHRPHEGLUTYRVALSERGLNPROPHELEUMETASPLEUGLUGLYLYSGLNGLYASNPHELYSASNLEUARGGLUPHEVALPHELYSASNILEASPGLYTYRPHELYSILETYRSERLYSHISTHRPROILEASNLEUVALARGASPLEUPROGLNGLYPHESERALALEUGLUPROLEUVALASPLEUPROILEGLYILEASNILETHRARGPHEGLNTHRLEULEUALALEUHISARGSERTYRLEUTHRPROGLYASPSERSERSERGLYTRPTHRALAGLYALAALAALATYRTYRVALGLYTYRLEUGLNPROARGTHRPHELEULEULYSTYRASNGLUASNGLYTHRILETHRASPALAVALASPCYSALALEUASPPROLEUSERGLUTHRLYSCYSTHRLEULYSSERPHETHRVALGLULYSGLYILETYRGLNTHRSERASNPHEARGVALGLNPROTHRGLUSERILEVALARGPHEPROASNILETHRASNLEUCYSPROPHEGLYGLUVALPHEASNALATHRARGPHEALASERVALTYRALATRPASNARGLYSARGILESERASNCYSVALALAASPTYRSERVALLEUTYRASNSERALASERPHESERTHRPHELYSCYSTYRGLYVALSERPROTHRLYSLEUASNASPLEUCYSPHETHRASNVALTYRALAASPSERPHEVALILEARGGLYASPGLUVALARGGLNILEALAPROGLYGLNTHRGLYLYSILEALAASPTYRASNTYRLYSLEUPROASPASPPHETHRGLYCYSVALILEALATRPASNSERASNASNLEUASPSERLYSVALGLYGLYASNTYRASNTYRLEUTYRARGLEUPHEARGLYSSERASNLEULYSPROPHEGLUARGASPILESERTHRGLUILETYRGLNALAGLYSERTHRPROCYSASNGLYVALGLUGLYPHEASNCYSTYRPHEPROLEUGLNSERTYRGLYPHEGLNPROTHRASNGLYVALGLYTYRGLNPROTYRARGVALVALVALLEUSERPHEGLULEULEUHISALAPROALATHRVALCYSGLYPROLYSLYSSERTHRASNLEUVALLYSASNLYSCYSVALASNPHEASNPHEASNGLYLEUTHRGLYTHRGLYVALLEUTHRGLUSERASNLYSLYSPHELEUPROPHEGLNGLNPHEGLYARGASPILEALAASPTHRTHRASPALAVALARGASPPROGLNTHRLEUGLUILELEUASPILETHRPROCYSSERPHEGLYGLYVALSERVALILETHRPROGLYTHRASNTHRSERASNGLNVALALAVALLEUTYRGLNASPVALASNCYSTHRGLUVALPROVALALAILEHISALAASPGLNLEUTHRPROTHRTRPARGVALTYRSERTHRGLYSERASNVALPHEGLNTHRARGALAGLYCYSLEUILEGLYALAGLUHISVALASNASNSERTYRGLUCYSASPILEPROILEGLYALAGLYILECYSALASERTYRGLNTHRGLNTHRASNSERPROARGARGALAARGSERVALALASERGLNSERILEILEALATYRTHRMETSERLEUGLYALAGLUASNSERVALALATYRSERASNASNSERILEALAILEPROTHRASNPHETHRILESERVALTHRTHRGLUILELEUPROVALSERMETTHRLYSTHRSERVALASPCYSTHRMETTYRILECYSGLYASPSERTHRGLUCYSSERASNLEULEULEUGLNTYRGLYSERPHECYSTHRGLNLEUASNARGALALEUTHRGLYILEALAVALGLUGLNASPLYSASNTHRGLNGLUVALPHEALAGLNVALLYSGLNILETYRLYSTHRPROPROILELYSASPPHEGLYGLYPHEASNPHESERGLNILELEUPROASPPROSERLYSPROSERLYSARGSERPHEILEGLUASPLEULEUPHEASNLYSVALTHRLEUALAASPALAGLYPHEILELYSGLNTYRGLYASPCYSLEUGLYASPILEALAALAARGASPLEUILECYSALAGLNLYSPHEASNGLYLEUTHRVALLEUPROPROLEULEUTHRASPGLUMETILEALAGLNTYRTHRSERALALEULEUALAGLYTHRILETHRSERGLYTRPTHRPHEGLYALAGLYALAALALEUGLNILEPROPHEALAMETGLNMETALATYRARGPHEASNGLYILEGLYVALTHRGLNASNVALLEUTYRGLUASNGLNLYSLEUILEALAASNGLNPHEASNSERALAILEGLYLYSILEGLNASPSERLEUSERSERTHRALASERALALEUGLYLYSLEUGLNASPVALVALASNGLNASNALAGLNALALEUASNTHRLEUVALLYSGLNLEUSERSERASNPHEGLYALAILESERSERVALLEUASNASPILELEUSERARGLEUASPLYSVALGLUALAGLUVALGLNILEASPARGLEUILETHRGLYARGLEUGLNSERLEUGLNTHRTYRVALTHRGLNGLNLEUILEARGALAALAGLUILEARGALASERALAASNLEUALAALATHRLYSMETSERGLUCYSVALLEUGLYGLNSERLYSARGVALASPPHECYSGLYLYSGLYTYRHISLEUMETSERPHEPROGLNSERALAPROHISGLYVALVALPHELEUHISVALTHRTYRVALPROALAGLNGLULYSASNPHETHRTHRALAPROALAILECYSHISASPGLYLYSALAHISPHEPROARGGLUGLYVALPHEVALSERASNGLYTHRHISTRPPHEVALTHRGLNARGASNPHETYRGLUPROGLNILEILETHRTHRASPASNTHRPHEVALSERGLYASNCYSASPVALVALILEGLYILEVALASNASNTHRVALTYRASPPROLEUGLNPROGLULEUASPSERPHELYSGLUGLULEUASPLYSTYRPHELYSASNHISTHRSERPROASPVALASPLEUGLYASPILESERGLYILEASNALASERVALVALASNILEGLNLYSGLUILEASPARGLEUASNGLUVALALALYSASNLEUASNGLUSERLEUILEASPLEUGLNGLULEUGLYLYSTYRGLUGLNTYRILELYSTRPPROTRPTYRILETRPLEUGLYPHEILEALAGLYLEUILEALAILEVALMETVALTHRILEMETLEUCYSCYSMETTHRSERCYSCYSSERCYSLEULYSGLYCYSCYSSERCYSGLYSERCYSCYSLYSPHEASPGLUASPASP

SEQ ID NO: 2082 - DNA, 324 bp, synthetic construct
  source 1..324: mol_type = other DNA
gacatccagatgacacagagccccagcagcctgtctgcctctgtgggagacagagtgaccatcacctgtcaggccagccaggacatcagcaactacctgaactggtatcagcagaaggccggcaaggcccctaagctgctgatctacgatgccagcaacctgcagatcggcgtgcccagcagattttctggcagcggctctggcaccgacttcaccttcagcataagcagcctgcagcctgaggatatcgccacctactactgccagcagtacgacaacctgcctccattcacctttggcggaggcaccaaggtggaaatcaaa

SEQ ID NO: 2083 - DNA, 11974 bp, synthetic construct
  source 1..11974: mol_type = other DNA
agatctcccgatcccctatggtgcactctcagtacaatctgctctgatgccgcatagttaagccagtatctgctccctgcttgtgtgttggaggtcgctgagtagtgcgcgagcaaaatttaagctacaacaaggcaaggcttgaccgacaattaattgcatgaagaatctgcttagggttaggcgttttgcgctgcttcgcgatgtacgggccagatatacgcgttgacattgattattgactagttattaatagtaatcaattacggggtcattagttcatagcccatatatggagttccgcgttacataacttacggtaaatggcccgcctggctgaccgcccaacgacccccgcccattgacgtcaataatgacgtatgttcccatagtaacgccaatagggactttccattgacgtcaatgggtggagtatttacggtaaactgcccacttggcagtacatcaagtgtatcatatgccaagtacgccccctattgacgtcaatgacggtaaatggcccgcctggcattatgcccagtacatgaccttatgggactttcctacttggcagtacatctacgtattagtcatcgctattaccatggtgatgcggttttggcagtacatcaatgggcgtggatagcggtttgactcacggggatttccaagtctccaccccattgacgtcaatgggagtttgttttggcaccaaaatcaacgggactttccaaaatgtcgtaacaactccgccccattgacgcaaatgggcggtaggcgtgtacggtgggaggtctatataagcagagctctctggctaactagagaacccactgcttactggcttatcgaaattaatacgactcactatagggagacccaagctagcttggtaccgggccgacctcaccatgggatggagctgtatcatcctcttcttggtagcaacagctacaggtaaggggctcacagtagcaggcttgaggtctggacatatatatgggtgacaatgacatccactttgcctttctctccacaggtgtgcattccgacatccagatgacacagagccccagcagcctgtctgcctctgtgggagacagagtgaccatcacctgtcaggccagccaggacatcagcaactacctgaactggtatcagcagaaggccggcaaggcccctaagctgctgatctacgatgccagcaacctgcagatcggcgtgcccagcagattttctggcagcggctctggcaccgacttcaccttcagcataagcagcctgcagcctgaggatatcgccacctactactgccagcagtacgacaacctgcctccattcacctttggcggaggcaccaaggtggaaatcaaacgtgagtcgtacgctagcaagcttgatatcgaattctaaactctgagggggtcggatgacgtggccattctttgcctaaagcattgagtttactgcaaggtcagaaaagcatgcaaagccctcagaatggctgcaaagagctccaacaaaacaatttagaactttattaaggaatagggggaagctaggaagaaactcaaaacatcaagattttaaatacgcttcttggtctccttgctataattatctgggataagcatgctgttttctgtctgtccctaacatgccctgtgattatccgcaaacaacacacccaagggcagaactttgttacttaaacaccatcctgtttgcttctttcctcaggaactgtggctgcaccatctgtcttcatcttcccgccatctgatgagcagttgaaatctggaactgcctctgttgtgtgcctgctgaataacttctatcccagagaggccaaagtacagtggaaggtggataacgccctccaatcgggtaactcccaggagagtgtcacagagcaggacagcaaggacagcacctacagcctcagcagcaccctgacgctgagcaaagcagactacgagaaacacaaagtctacgcctgcgaagtcacccatcagggcctgagctcgcccgtcacaaagagcttcaacaggggagagtgttagagggagaagtgcccccacctgctcctcagttccagcctgaccccctcccatcctttggcctctgaccctttttccacaggggacctacccctattgcggtcctccagctcatctttcacctcacccccctcctcctccttggctttaattatgctaatgttggaggagaatgaataaataaagtgaatctttgcacctgtggtttctctctttcctcatttaataattattatctgttgttttaccaactactcaatttctcttataagggactaaatatgtagtcatcctaaggcgcataaccatttataaaaatcatccttcattctattttaccctatcatcctctgcaagacagtcctccctcaaacccacaagccttctgtcctcacagtcccctgggccatggtaggagagacttgcttccttgttttcccctcctcagcaagccctcatagtcctttttaagggtgacaggtcttacagtcatatatcctttgattcaattccctgagaatcaaccaaggcaaattcctgcagcccgggggatccagacatgataagatacattgatgagtttggacaaaccacaactacaatgcagtgaaaaaaatgctttatttgtgaaatttgtgatgctattgctttatttgtaaccattataagctgcaataaacaagttaacaacaacaattccattcattttatgtttcaggttcagggggaggtgtgggaggttttttaaagcaagtaaaacctctacaaatgtggtatggctgattatgatccggctgcctcgcgcgtttcggtgatgacggtgaaaacctctgacacatgcagctcccggagacggtcacagcttgtctgtaagcggatgccgggagcagacaagcccgtcaggcgtcagcgggtgttggcgggtgtcggggcgcagccatgaggtcgactctagaggatcgatccccgccccggacgaactaaacctgactacgacatctctgccccttcttcgcggggcagtgcatgtaatcccttcagttggttggtacaacttgccaactgggccctgttccacatgtgacacggggggggaccaaacacaaaggggttctctgactgtagttgacatccttataaatggatgtgcacatttgccaacactgagtggctttcatcctggagcagactttgcagtctgtggactgcaacacaacattgcctttatgtgtaactcttggctgaagctcttacaccaatgctgggggacatgtacctcccaggggcccaggaagactacgggaggctacaccaacgtcaatcagaggggcctgtgtagctaccgataagcggaccctcaagagggcattagcaatagtgtttataaggcccccttgttaaccctaaacgggtagcatatgcttcccgggtagtagtatatactatccagactaaccctaattcaatagcatatgttacccaacgggaagcatatgctatcgaattagggttagtaaaagggtcctaaggaacagcgatatctcccaccccatgagctgtcacggttttatttacatggggtcaggattccacgagggtagtgaaccattttagtcacaagggcagtggctgaagatcaaggagcgggcagtgaactctcctgaatcttcgcctgcttcttcattctccttcgtttagctaatagaataactgctgagttgtgaacagtaaggtgtatgtgaggtgctcgaaaacaaggtttcaggtgacgcccccagaataaaatttggacggggggttcagtggtggcattgtgctatgacaccaatataaccctcacaaaccccttgggcaataaatactagtgtaggaatgaaacattctgaatatctttaacaatagaaatccatggggtggggacaagccgtaaagactggatgtccatctcacacgaatttatggctatgggcaacacataatcctagtgcaatatgatactggggttattaagatgtgtcccaggcagggaccaagacaggtgaaccatgttgttacactctatttgtaacaaggggaaagagagtggacgccgacagcagcggactccactggttgtctctaacacccccgaaaattaaacggggctccacgccaatggggcccataaacaaagacaagtggccactcttttttttgaaattgtggagtgggggcacgcgtcagcccccacacgccgccctgcggttttggactgtaaaataagggtgtaataacttggctgattgtaaccccgctaaccactgcggtcaaaccacttgcccacaaaaccactaatggcaccccggggaatacctgcataagtaggtgggcgggccaagataggggcgcgattgctgcgatctggaggacaaattacacacacttgcgcctgagcgccaagcacagggttgttggtcctcatattcacgaggtcgctgagagcacggtgggctaatgttgccatgggtagcatatactacccaaatatctggatagcatatgctatcctaatctatatctgggtagcataggctatcctaatctatatctgggtagcatatgctatcctaatctatatctgggtagtatatgctatcctaatttatatctgggtagcataggctatcctaatctatatctgggtagcatatgctatcctaatctatatctgggtagtatatgctatcctaatctgtatccgggtagcatatgctatcctaatagagattagggtagtatatgctatcctaatttatatctgggtagcatatactacccaaatatctggatagcatatgctatcctaatctatatctgggtagcatatgctatcctaatctatatctgggtagcataggctatcctaatctatatctgggtagcatatgctatcctaatctatatctgggtagtatatgctatcctaatttatatctgggtagcataggctatcctaatctatatctgggtagcatatgctatcctaatctatatctgggtagtatatgctatcctaatctgtatccgggtagcatatgctatcctcatgcatatacagtcagcatatgatacccagtagtagagtgggagtgctatcctttgcatatgccgccacctcccaagggggcgtgaattttcgctgcttgtccttttcctgctggttgctcccattcttaggtgaatttaaggaggccaggctaaagccgtcgcatgtctgattgctcaccaggtaaatgtcgctaatgttttccaacgcgagaaggtgttgagcgcggagctgagtgacgtgacaacatgggtatgcccaattgccccatgttgggaggacgaaaatggtgacaagacagatggccagaaatacaccaacagcacgcatgatgtctactggggatttattctttagtgcgggggaatacacggcttttaatacgattgagggcgtctcctaacaagttacatcactcctgcccttcctcaccctcatctccatcacctccttcatctccgtcatctccgtcatcaccctccgcggcagccccttccaccataggtggaaaccagggaggcaaatctactccatcgtcaaagctgcacacagtcaccctgatattgcaggtaggagcgggctttgtcataacaaggtccttaatcgcatccttcaaaacctcagcaaatatatgagtttgtaaaaagaccatgaaataacagacaatggactcccttagcgggccaggttgtgggccgggtccaggggccattccaaaggggagacgactcaatggtgtaagacgacattgtggaatagcaagggcagttcctcgccttaggttgtaaagggaggtcttactacctccatatacgaacacaccggcgacccaagttccttcgtcggtagtcctttctacgtgactcctagccaggagagctcttaaaccttctgcaatgttctcaaatttcgggttggaacctccttgaccacgatgctttccaaaccaccctccttttttgcgcctgcctccatcaccctgaccccggggtccagtgcttgggccttctcctgggtcatctgcggggccctgctctatcgctcccgggggcacgtcaggctcaccatctgggccaccttcttggtggtattcaaaataatcggcttcccctacagggtggaaaaatggccttctacctggagggggcctgcgcggtggagacccggatgatgatgactgactactgggactcctgggcctcttttctccacgtccacgacctctccccctggctctttcacgacttccccccctggctctttcacgtcctctaccccggcggcctccactacctcctcgaccccggcctccactacctcctcgaccccggcctccactgcctcctcgaccccggcctccacctcctgctcctgcccctcctgctcctgcccctcctcctgctcctgcccctcctgcccctcctgctcctgcccctcctgcccctcctgctcctgcccctcctgcccctcctgctcctgcccctcctgcccctcctcctgctcctgcccctcctgcccctcctcctgctcctgcccctcctgcccctcctgctcctgcccctcctgcccctcctgctcctgcccctcctgcccctcctgctcctgcccctcctgctcctgcccctcctgctcctgcccctcctgctcctgcccctcctgcccctcctgcccctcctcctgctcctgcccctcctgctcctgcccctcctgcccctcctgcccctcctgctcctgcccctcctcctgctcctgcccctcctgcccctcctgcccctcctcctgctcctgcccctcctgcccctcctcctgctcctgcccctcctcctgctcctgcccctcctgcccctcctgcccctcctcctgctcctgcccctcctgcccctcctcctgctcctgcccctcctcctgctcctgcccctcctgcccctcctgcccctcctcctgctcctgcccctcctcctgctcctgcccctcctgcccctcctgcccctcctgcccctcctcctgctcctgcccctcctcctgctcctgcccctcctgctcctgcccctcccgctcctgctcctgctcctgttccaccgtgggtccctttgcagccaatgcaacttggacgtttttggggtctccggacaccatctctatgtcttggccctgatcctgagccgcccggggctcctggtcttccgcctcctcgtcctcgtcctcttccccgtcctcgtccatggttatcaccccctcttctttgaggtccactgccgccggagccttctggtccagatgtgtctcccttctctcctaggccatttccaggtcctgtacctggcccctcgtcagacatgattcacactaaaagagatcaatagacatctttattagacgacgctcagtgaatacagggagtgcagactcctgccccctccaacagcccccccaccctcatccccttcatggtcgctgtcagacagatccaggtctgaaaattccccatcctccgaaccatcctcgtcctcatcaccaattactcgcagcccggaaaactcccgctgaacatcctcaagatttgcgtcctgagcctcaagccaggcctcaaattcctcgtccccctttttgctggacggtagggatggggattctcgggacccctcctcttcctcttcaaggtcaccagacagagatgctactggggcaacggaagaaaagctgggtgcggcctgtgaggatcagcttatcgatgataagctgtcaaacatgagaattcttgaagacgaaagggcctcgtgatacgcctatttttataggttaatgtcatgataataatggtttcttagacgtcaggtggcacttttcggggaaatgtgcgcggaacccctatttgtttatttttctaaatacattcaaatatgtatccgctcatgagacaataaccctgataaatgcttcaataatattgaaaaaggaagagtatgagtattcaacatttccgtgtcgcccttattcccttttttgcggcattttgccttcctgtttttgctcacccagaaacgctggtgaaagtaaaagatgctgaagatcagttgggtgcacgagtgggttacatcgaactggatctcaacagcggtaagatccttgagagttttcgccccgaagaacgttttccaatgatgagcacttttaaagttctgctatgtggcgcggtattatcccgtgttgacgccgggcaagagcaactcggtcgccgcatacactattctcagaatgacttggttgagtactcaccagtcacagaaaagcatcttacggatggcatgacagtaagagaattatgcagtgctgccataaccatgagtgataacactgcggccaacttacttctgacaacgatcggaggaccgaaggagctaaccgcttttttgcacaacatgggggatcatgtaactcgccttgatcgttgggaaccggagctgaatgaagccataccaaacgacgagcgtgacaccacgatgcctgcagcaatggcaacaacgttgcgcaaactattaactggcgaactacttactctagcttcccggcaacaattaatagactggatggaggcggataaagttgcaggaccacttctgcgctcggcccttccggctggctggtttattgctgataaatctggagccggtgagcgtgggtctcgcggtatcattgcagcactggggccagatggtaagccctcccgtatcgtagttatctacacgacggggagtcaggcaactatggatgaacgaaatagacagatcgctgagataggtgcctcactgattaagcattggtaactgtcagaccaagtttactcatatatactttagattgatttaaaacttcatttttaatttaaaaggatctaggtgaagatcctttttgataatctcatgaccaaaatcccttaacgtgagttttcgttccactgagcgtcagaccccgtagaaaagatcaaaggatcttcttgagatcctttttttctgcgcgtaatctgctgcttgcaaacaaaaaaaccaccgctaccagcggtggtttgtttgccggatcaagagctaccaactctttttccgaaggtaactggcttcagcagagcgcagataccaaatactgtccttctagtgtagccgtagttaggccaccacttcaagaactctgtagcaccgcctacatacctcgctctgctaatcctgttaccagtggctgctgccagtggcgataagtcgtgtcttaccgggttggactcaagacgatagttaccggataaggcgcagcggtcgggctgaacggggggttcgtgcacacagcccagcttggagcgaacgacctacaccgaactgagatacctacagcgtgagctatgagaaagcgccacgcttcccgaagggagaaaggcggacaggtatccggtaagcggcagggtcggaacaggagagcgcacgagggagcttccagggggaaacgcctggtatctttatagtcctgtcgggtttcgccacctctgacttgagcgtcgatttttgtgatgctcgtcaggggggcggagcctatggaaaaacgccagcaacgcggcctttttacggttcctggccttttgctggccttgaagctgtccctgatggtcgtcatctacctgcctggacagcatggcctgcaacgcgggcatcccgatgccgccggaagcgagaagaatcataatggggaaggccatccagcctcgcgtcgcgaacgccagcaagacgtagcccagcgcgtcggccccgagatgcgccgcgtgcggctgctggagatggcggacgcgatggatatgttctgccaagggttggtttgcccattcacagttctccgcaagaattgattggctccaattcttggagtggtgaatccgttagcgaggtgccgccctgcttcatccccgtggcccgttgctcgcgtttgctggcggtgtccccggaagaaatatatttgcatgtctttagttctatgatgacacaaaccccgcccagcgtcttgtcattggcgaattcgaacacgcagatgcagtcggggcggcgcggtccgaggtccacttcgcatattaaggtgacgcgtgtggcctcgaacaccgagcgaccctgcagcgacccgcttaacagcgtcaacagcgtgccgcagatcccggggggcaatgagatatgaaaaagcctgaactcaccgcgacgtctgtcgagaagtttctgatcgaaaagttcgacagcgtctccgacctgatgcagctctcggagggcgaagaatctcgtgctttcagcttcgatgtaggagggcgtggatatgtcctgcgggtaaatagctgcgccgatggtttctacaaagatcgttatgtttatcggcactttgcatcggccgcgctcccgattccggaagtgcttgacattggggaattcagcgagagcctgacctattgcatctcccgccgtgcacagggtgtcacgttgcaagacctgcctgaaaccgaactgcccgctgttctgcagccggtcgcggaggccatggatgcgatcgctgcggccgatcttagccagacgagcgggttcggcccattcggaccgcaaggaatcggtcaatacactacatggcgtgatttcatatgcgcgattgctgatccccatgtgtatcactggcaaactgtgatggacgacaccgtcagtgcgtccgtcgcgcaggctctcgatgagctgatgctttgggccgaggactgccccgaagtccggcacctcgtgcacgcggatttcggctccaacaatgtcctgacggacaatggccgcataacagcggtcattgactggagcgaggcgatgttcggggattcccaatacgaggtcgccaacatcttcttctggaggccgtggttggcttgtatggagcagcagacgcgctacttcgagcggaggcatccggagcttgcaggatcgccgcggctccgggcgtatatgctccgcattggtcttgaccaactctatcagagcttggttgacggcaatttcgatgatgcagcttgggcgcagggtcgatgcgacgcaatcgtccgatccggagccgggactgtcgggcgtacacaaatcgcccgcagaagcgcggccgtctggaccgatggctgtgtagaagtactcgccgatagtggaaaccgacgccccagcactcgtccggatcgggagatgggggaggctaactgaaacacggaaggagacaataccggaaggaacccgcgctatgacggcaataaaaagacagaataaaacgcacgggtgttgggtcgtttgttcataaacgcggggttcggtcccagggctggcactctgtcgataccccaccgagaccccattggggccaatacgcccgcgtttcttccttttccccaccccaccccccaagttcgggtgaaggcccagggctcgcagccaacgtcggggcggcaggccctgccatagccactggccccgtgggttagggacggggtcccccatggggaatggtttatggttcgtgggggttattattttgggcgttgcgtggggtcaggtccacgactggactgagcagacagacccatggtttttggatggcctgggcatggaccgcatgtactggcgcgacacgaacaccgggcgtctgtggctgccaaacacccccgacccccaaaaaccaccgcgcggatttctggcgtgccaagctagtcgaccaattctcatgtttgacagcttatcatcgcagatccgggcaacgttgttgccattgctgcaggcgcagaactggtaggtatgga

SEQ ID NO: 2084 - DNA, 387 bp, synthetic construct
  source 1..387: mol_type = other DNA
gaagtgcagctgctggaatctggcggcggacttgtgaaacctggcggctctctgagactgagctgtgccgcttccggcttcaccttcaccaattacgccatgggctgggtccgacaggcccctggaaaaggacttgagtgggtgtccaccatcaacgacagcggcggcagcacctactacaccgagtctgtcagaggccggttcaccatcagccgggacaacagcaagaataccctgttcctgcagatgggcagcctgagagccgaagataccgccgtgtactactgcgccaaggatgatggcggaagcagactgcctaactgtggcggcgactgcagcagagcctttgattattggggccagggcaccctggtcaccgtttcttca

SEQ ID NO: 2085 - DNA, 13450 bp, synthetic construct
  source 1..13450: mol_type = other DNA
gcttcgcgatgtacgggccagatatacgcgttgacattgattattgactagttattaatagtaatcaattacggggtcattagttcatagcccatatatggagttccgcgttacataacttacggtaaatggcccgcctggctgaccgcccaacgacccccgcccattgacgtcaataatgacgtatgttcccatagtaacgccaatagggactttccattgacgtcaatgggtggagtatttacggtaaactgcccacttggcagtacatcaagtgtatcatatgccaagtacgccccctattgacgtcaatgacggtaaatggcccgcctggcattatgcccagtacatgaccttatgggactttcctacttggcagtacatctacgtattagtcatcgctattaccatggtgatgcggttttggcagtacatcaatgggcgtggatagcggtttgactcacggggatttccaagtctccaccccattgacgtcaatgggagtttgttttggcaccaaaatcaacgggactttccaaaatgtcgtaacaactccgccccattgacgcaaatgggcggtaggcgtgtacggtgggaggtctatataagcagagctctctggctaactagagaacccactgcttactggcttatcgaaattaatacgactcactatagggagacccaagctagcttggtaccgggccgacctcaccatgggatggagctgtatcatcctcttcttggtagcaacagctacaggtaaggggctcacagtagcaggcttgaggtctggacatatatatgggtgacaatgacatccactttgcctttctctccacaggtgtgcattccgaagtgcagctgctggaatctggcggcggacttgtgaaacctggcggctctctgagactgagctgtgccgcttccggcttcaccttcaccaattacgccatgggctgggtccgacaggcccctggaaaaggacttgagtgggtgtccaccatcaacgacagcggcggcagcacctactacaccgagtctgtcagaggccggttcaccatcagccgggacaacagcaagaataccctgttcctgcagatgggcagcctgagagccgaagataccgccgtgtactactgcgccaaggatgatggcggaagcagactgcctaactgtggcggcgactgcagcagagcctttgattattggggccagggcaccctggtcaccgtttcttcaggtgagtcgtacgctagcaagctttctggggcaggccaggcctgaccttggctttggggcagggagggggctaaggtgaggcaggtggcgccagccaggtgcacacccaatgcccatgagcccagacactggacgctgaacctcgcggacagttaagaacccaggggcctctgcgccctgggcccagctctgtcccacaccgcggtcacatggcaccacctctcttgcagcctccaccaagggcccatcggtcttccccctggcaccctcctccaagagcacctctgggggcacagcggccctgggctgcctggtcaaggactacttccccgaaccggtgacggtgtcgtggaactcaggcgccctgaccagcggcgtgcacaccttcccggctgtcctacagtcctcaggactctactccctcagcagcgtggtgaccgtgccctccagcagcttgggcacccagacctacatctgcaacgtgaatcacaagcccagcaacaccaaggtggacaagaaagttggtgagaggccagcacagggagggagggtgtctgctggaagccaggctcagcgctcctgcctggacgcatcccggctatgcagccccagtccagggcagcaaggcaggccccgtctgcctcttcacccggaggcctctgcccgccccactcatgctcagggagagggtcttctggctttttccccaggctctgggcaggcacaggctaggtgcccctaacccaggccctgcacacaaaggggcaggtgctgggctcagacctgccaagagccatatccgggaggaccctgcccctgacctaagcccaccccaaaggccaaactctccactccctcagctcggacaccttctctcctcccagattccagtaactcccaatcttctctctgcagagcccaaatcttgtgacaaaactcacacatgcccaccgtgcccaggtaagccagcccaggcctcgccctccagctcaaggcgggacaggtgccctagagtagcctgcatccagggacaggccccagccgggtgctgacacgtccacctccatctcttcctcagcacctgaactcctggggggaccgtcagtcttcctcttccccccaaaacccaaggacaccctcatgatctcccggacccctgaggtcacatgcgtggtggtggacgtgagccacgaagaccctgaggtcaagttcaactggtacgtggacggcgtggaggtgcataatgccaagacaaagccgcgggaggagcagtacaacagcacgtaccgtgtggtcagcgtcctcaccgtcctgcaccaggactggctgaatggcaaggagtacaagtgcaaggtctccaacaaagccctcccagcccccatcgagaaaaccatctccaaagccaaaggtgggacccgtggggtgcgagggccacatggacagaggccggctcggcccaccctctgccctgagagtgaccgctgtaccaacctctgtccctacagggcagccccgagaaccacaggtgtacaccctgcccccatcccgggatgagctgaccaagaaccaggtcagcctgacctgcctggtcaaaggcttctatcccagcgacatcgccgtggagtgggagagcaatgggcagccggagaacaactacaagaccacgcctcccgtgctggactccgacggctccttcttcctctacagcaagctcaccgtggacaagagcaggtggcagcaggggaacgtcttctcatgctccgtgatgcatgaggctctgcacaaccactacacgcagaagagcctctccctgtctccgggtaaatgagatcgatggccggcaagcccccgctccccgggctctcgcggtcgcacgaggatgcttggcacgtaccccctgtacatacttcccgggcgcccagcatggaaataaagcacccagcgctgccctgggcccctgcgagactgtgatggttctttccacgggtcaggccgagtctgaggcctgagtggcatgagggaggcagagcgggtcccactgtccccacactggcccaggctgtgcaggtgtgcctgggccgcctagggtggggctcagccaggggctgccctcggcagggtgggggatttgccagcgtggccctccctccagcagcacctgccctgggctgggccacgggaagccctaggagcccctggggacagacacacagcccctgcctctgtaggagactgtcctgttctgtgagcgccctgtcctccgacctccatgcccactcgggggcatgcctgcaggtcgactctagaggatccactagtaacggccgccagtgtgctggaattctgcagatatccatcacactggcggccgctcgagcatgcatctagagggccctattctatagtgtcacctaaatgctagagctcgctgatcagcctcgactgtgccttctagttgccagccatctgttgtttgcccctcccccgtgccttccttgaccctggaaggtgccactcccactgtcctttcctaataaaatgaggaaattgcatcgcattgtctgagtaggtgtcattctattctggggggtggggtggggcaggacagcaagggggaggattgggaagacaatagcaggcatgctggggatgcggtgggctctatggcttctgaggcggaaagaaccagctggggctctagggggtatccccacgcgccctgtagcggcgcattaagcgcggcgggtgtggtggttacgcgcagcgtgaccgctacacttgccagcgccctagcgcccgctcctttcgctttcttcccttcctttctcgccacgttcgccggctttccccgtcaagctctaaatcgggggctccctttagggttccgatttagtgctttacggcacctcgaccccaaaaaacttgattagggtgatggttcacgtagtgggccatcgccctgatagacggtttttcgccctttgacgttggagtccacgttctttaatagtggactcttgttccaaactggaacaacactcaaccctatctcggtctattcttttgatttataagggattttgccgatttcggcctattggttaaaaaatgagctgatttaacaaaaatttaacgcgaattaattctgtggaatgtgtgtcagttagggtgtggaaagtccccaggctccccagcaggcagaagtatgcaaagcatgcatctcaattagtcagcaaccaggtgtggaaagtccccaggctccccagcaggcagaagtatgcaaagcatgcatctcaattagtcagcaaccatagtcccgcccctaactccgcccatcccgcccctaactccgcccagttccgcccattctccgccccatggctgactaattttttttatttatgcagaggccgaggccgcctctgcctctgagctattccagaagtagtgaggaggcttttttggaggcctaggcttttgcaaaaagctcccgggagcttgtatatccattttcggatctgatcaagagacaggatgaggatcgtttcgcatgattgaacaagatggattgcacgcaggttctccggccgcttgggtggagaggctattcggctatgactgggcacaacagacaatcggctgctctgatgccgccgtgttccggctgtcagcgcaggggcgcccggttctttttgtcaagaccgacctgtccggtgccctgaatgaactgcaggacgaggcagcgcggctatcgtggctggccacgacgggcgttccttgcgcagctgtgctcgacgttgtcactgaagcgggaagggactggctgctattgggcgaagtgccggggcaggatctcctgtcatctcaccttgctcctgccgagaaagtatccatcatggctgatgcaatgcggcggctgcatacgcttgatccggctacctgcccattcgaccaccaagcgaaacatcgcatcgagcgagcacgtactcggatggaagccggtcttgtcgatcaggatgatctggacgaagagcatcaggggctcgcgccagccgaactgttcgccaggctcaaggcgcgcatgcccgacggcgaggatctcgtcgtgacccatggcgatgcctgcttgccgaatatcatggtggaaaatggccgcttttctggattcatcgactgtggccggctgggtgtggcggaccgctatcaggacatagcgttggctacccgtgatattgctgaagagcttggcggcgaatgggctgaccgcttcctcgtgctttacggtatcgccgctcccgattcgcagcgcatcgccttctatcgccttcttgacgagttcttctgagcgggactctggggttcgaattcgccaatgacaagacgctgggcggggtttgtgtcatcatagaactaaagacatgcaaatatatttcttccggggacaccgccagcaaacgcgagcaacgggccacggggatgaagcagggcggcacctcgctaacggattcaccactccaagaattggagccaatcaattcttgcggagaactgtgaatgggcaaaccaacccttggcagaacatatccatcgcgtccgccatctccagcagccgcacgcggcgcatctcggggccgacgcgctgggctacgtcttgctggcgttcgcgacgcgaggctggatggccttccccattatgattcttctcgcttccggcggcatcgggatgcccgcgttgcaggccatgctgtccaggcaggtagatgacgaccatcagggacagcttcaaggccagcaaaaggccaggaaccgtaaaaaggccgcgttgctggcgtttttccataggctccgcccccctgacgagcatcacaaaaatcgacgctcaagtcagaggtggcgaaacccgacaggactataaagataccaggcgtttccccctggaagctccctcgtgcgctctcctgttccgaccctgccgcttaccggatacctgtccgcctttctcccttcgggaagcgtggcgctttctcatagctcacgctgtaggtatctcagttcggtgtaggtcgttcgctccaagctgggctgtgtgcacgaaccccccgttcagcccgaccgctgcgccttatccggtaactatcgtcttgagtccaacccggtaagacacgacttatcgccactggcagcagccactggtaacaggattagcagagcgaggtatgtaggcggtgctacagagttcttgaagtggtggcctaactacggctacactagaaggacagtatttggtatctgcgctctgctgaagccagttaccttcggaaaaagagttggtagctcttgatccggcaaacaaaccaccgctggtagcggtggtttttttgtttgcaagcagcagattacgcgcagaaaaaaaggatctcaagaagatcctttgatcttttctacggggtctgacgctcagtggaacgaaaactcacgttaagggattttggtcatgagattatcaaaaaggatcttcacctagatccttttaaattaaaaatgaagttttaaatcaatctaaagtatatatgagtaaacttggtctgacagttaccaatgcttaatcagtgaggcacctatctcagcgatctgtctatttcgttcatccatagttgcctgactccccgtcgtgtagataactacgatacgggagggcttaccatctggccccagtgctgcaatgataccgcgagacccacgctcaccggctccagatttatcagcaataaaccagccagccggaagggccgagcgcagaagtggtcctgcaactttatccgcctccatccagtctattaattgttgccgggaagctagagtaagtagttcgccagttaatagtttgcgcaacgttgttgccattgctgcaggcatcgtggtgtcacgctcgtcgtttggtatggcttcattcagctccggttcccaacgatcaaggcgagttacatgatcccccatgttgtgcaaaaaagcggttagctccttcggtcctccgatcgttgtcagaagtaagttggccgcagtgttatcactcatggttatggcagcactgcataattctcttactgtcatgccatccgtaagatgcttttctgtgactggtgagtactcaaccaagtcattctgagaatagtgtatgcggcgaccgagttgctcttgcccggcgtcaacacgggataataccgcgccacatagcagaactttaaaagtgctcatcattggaaaacgttcttcggggcgaaaactctcaaggatcttaccgctgttgagatccagttcgatgtaacccactcgtgcacccaactgatcttcagcatcttttactttcaccagcgtttctgggtgagcaaaaacaggaaggcaaaatgccgcaaaaaagggaataagggcgacacggaaatgttgaatactcatactcttcctttttcaatattattgaagcatttatcagggttattgtctcatgagcggatacatatttgaatgtatttagaaaaataaacaaataggggttccgcgcacatttccccgaaaagtgccacctgacgtctaagaaccattattatcatgacattaacctataaaaataggcgtatcacgaggccctttcgtcttcaagaattctcatgtttgacagcttatcatcgataagctgatcctcacaggccgcacccagcttttcttccgttgccccagtagcatctctgtctggtgaccttgaagaggaagaggaggggtcccgagaatccccatccctaccgtccagcaaaaagggggacgaggaatttgaggcctggcttgaggctcaggacgcaaatcttgaggatgttcagcgggagttttccgggctgcgagtaattggtgatgaggacgaggatggttcggaggatggggaattttcagacctggatctgtctgacagcgaccatgaaggggatgagggtgggggggctgttggagggggcaggagtctgcactccctgtattcactgagcgtcgtctaataaagatgtctattgatctcttttagtgtgaatcatgtctgacgaggggccaggtacaggacctggaaatggcctaggagagaagggagacacatctggaccagaaggctccggcggcagtggacctcaaagaagagggggtgataaccatggacgaggacggggaagaggacgaggacgaggaggcggaagaccaggagccccgggcggctcaggatcagggccaagacatagagatggtgtccggagaccccaaaaacgtccaagttgcattggctgcaaagggacccacggtggaacaggagcaggagcaggagcgggaggggcaggagcaggaggggcaggagcaggaggaggggcaggagcaggaggaggggcaggaggggcaggaggggcaggaggggcaggagcaggaggaggggcaggagcaggaggaggggcaggaggggcaggaggggcaggagcaggaggaggggcaggagcaggaggaggggcaggaggggcaggagcaggaggaggggcaggaggggcaggaggggcaggagcaggaggaggggcaggagcaggaggaggggcaggaggggcaggagcaggaggaggggcaggaggggcaggaggggcaggagcaggaggaggggcaggagcaggaggggcaggaggggcaggaggggcaggagcaggaggggcaggagcaggaggaggggcaggaggggcaggaggggcaggagcaggaggggcaggagcaggaggggcaggagcaggaggggcaggagcaggaggggcaggaggggcaggagcaggaggggcaggaggggcaggagcaggaggggcaggaggggcaggagcaggaggaggggcaggaggggcaggagcaggaggaggggcaggaggggcaggagcaggaggggcaggaggggcaggagcaggaggggcaggaggggcaggagcaggaggggcaggaggggcaggagcaggaggaggggcaggagcaggaggggcaggagcaggaggtggaggccggggtcgaggaggcagtggaggccggggtcgaggaggtagtggaggccggggtcgaggaggtagtggaggccgccggggtagaggacgtgaaagagccagggggggaagtcgtgaaagagccagggggagaggtcgtggacgtggagaaaagaggcccaggagtcccagtagtcagtcatcatcatccgggtctccaccgcgcaggccccctccaggtagaaggccatttttccaccctgtaggggaagccgattattttgaataccaccaagaaggtggcccagatggtgagcctgacgtgcccccgggagcgatagagcagggccccgcagatgacccaggagaaggcccaagcactggaccccggggtcagggtgatggaggcaggcgcaaaaaaggagggtggtttggaaagcatcgtggtcaaggaggttccaacccgaaatttgagaacattgcagaaggtttaagagctctcctggctaggagtcacgtagaaaggactaccgacgaaggaacttgggtcgccggtgtgttcgtatatggaggtagtaagacctccctttacaacctaaggcgaggaactgcccttgctattccacaatgtcgtcttacaccattgagtcgtctcccctttggaatggcccctggacccggcccacaacctggcccgctaagggagtccattgtctgttatttcatggtctttttacaaactcatatatttgctgaggttttgaaggatgcgattaaggaccttgttatgacaaagcccgctcctacctgcaatatcagggtgactgtgtgcagctttgacgatggagtagatttgcctccctggtttccacctatggtggaaggggctgccgcggagggtgatgacggagatgacggagatgaaggaggtgatggagatgagggtgaggaagggcaggagtgatgtaacttgttaggagacgccctcaatcgtattaaaagccgtgtattcccccgcactaaagaataaatccccagtagacatcatgcgtgctgttggtgtatttctggccatctgtcttgtcaccattttcgtcctcccaacatggggcaattgggcatacccatgttgtcacgtcactcagctccgcgctcaacaccttctcgcgttggaaaacattagcgacatttacctggtgagcaatcagacatgcgacggctttagcctggcctccttaaattcacctaagaatgggagcaaccagcaggaaaaggacaagcagcgaaaattcacgcccccttgggaggtggcggcatatgcaaaggatagcactcccactctactactgggtatcatatgctgactgtatatgcatgaggatagcatatgctacccggatacagattaggatagcatatactacccagatatagattaggatagcatatgctacccagatatagattaggatagcctatgctacccagatataaattaggatagcatatactacccagatatagattaggatagcatatgctacccagatatagattaggatagcctatgctacccagatatagattaggatagcatatgctacccagatatagattaggatagcatatgctatccagatatttgggtagtatatgctacccagatataaattaggatagcatatactaccctaatctctattaggatagcatatgctacccggatacagattaggatagcatatactacccagatatagattaggatagcatatgctacccagatatagattaggatagcctatgctacccagatataaattaggatagcatatactacccagatatagattaggatagcatatgctacccagatatagattaggatagcctatgctacccagatatagattaggatagcatatgctatccagatatttgggtagtatatgctacccatggcaacattagcccaccgtgctctcagcgacctcgtgaatatgaggaccaacaaccctgtgcttggcgctcaggcgcaagtgtgtgtaatttgtcctccagatcgcagcaatcgcgcccctatcttggcccgcccacctacttatgcaggtattccccggggtgccattagtggttttgtgggcaagtggtttgaccgcagtggttagcggggttacaatcagccaagttattacacccttattttacagtccaaaaccgcagggcggcgtgtgggggctgacgcgtgcccccactccacaatttcaaaaaaaagagtggccacttgtctttgtttatgggccccattggcgtggagccccgtttaattttcgggggtgttagagacaaccagtggagtccgctgctgtcggcgtccactctctttccccttgttacaaatagagtgtaacaacatggttcacctgtcttggtccctgcctgggacacatcttaataaccccagtatcatattgcactaggattatgtgttgcccatagccataaattcgtgtgagatggacatccagtctttacggcttgtccccaccccatggatttctattgttaaagatattcagaatgtttcattcctacactagtatttattgcccaaggggtttgtgagggttatattggtgtcatagcacaatgccaccactgaaccccccgtccaaattttattctgggggcgtcacctgaaaccttgttttcgagcacctcacatacaccttactgttcacaactcagcagttattctattagctaaacgaaggagaatgaagaagcaggcgaagattcaggagagttcactgcccgctccttgatcttcagccactgcccttgtgactaaaatggttcactaccctcgtggaatcctgaccccatgtaaataaaaccgtgacagctcatggggtgggagatatcgctgttccttaggacccttttactaaccctaattcgatagcatatgcttcccgttgggtaacatatgctattgaattagggttagtctggatagtatatactactacccgggaagcatatgctacccgtttagggttaacaagggggccttataaacactattgctaatgccctcttgagggtccgcttatcggtagctacacaggcccctctgattgacgttggtgtagcctcccgtagtcttcctgggcccctgggaggtacatgtcccccagcattggtgtaagagcttcagccaagagttacacataaaggcaatgttgtgttgcagtccacagactgcaaagtctgctccaggatgaaagccactcagtgttggcaaatgtgcacatccatttataaggatgtcaactacagtcagagaacccctttgtgtttggtccccccccgtgtcacatgaggaacagggcccagttggcaagttgtaccaaccaactgaagggattacatgcactgccccgcgaagaaggggcagagatgtcgtagtcaggtttagttcgtccggggcggggcatcgatcctctagagtcgacctcatggctgcgccccgacacccgccaacacccgctgacgcctgacgggcttgtctgctcccggcatccgcttacagacaagctgtgaccgtctccgggagctgcatgtgtcagaggttttcaccgtcatcaccgaaacgcgcgaggcagccggatcataatcagccataccacatttgtagaggttttacttgctttaaaaaacctcccacacctccccctgaacctgaaacataaaatcaatgcaattgttgttgttaacttgtttattgcagcttataatggttacaaataaagcaatagcatcacaaatttcacaaataaagcatttttttcactgcattgtagttgtggtttgtccaaactcatcaatgtatcttatcatgtctggatccggccttgccggcctcgagcggccgctagcaagcttgctagcagctggtacccagcttctagagatctcccgatcccctatggtgcactctcagtacaatctgctctgatgccgcatagttaagccagtatctgctccctgcttgtgtgttggaggtcgctgagtagtgcgcgagcaaaatttaagctacaacaaggcaaggcttgaccgacaattaattgcatgaagaatctgcttagggttaggcgttttgcgct

SEQ ID NO: 2086 - DNA, 369 bp, synthetic construct
  source 1..369: mol_type = other DNA
cagagacagctggtgcagtctggccccgaagtgaagaaacctggcaccagcgtgaaggtgtcctgcaaggccagcggcttcacctttagcatctctgccgtgcagtgggtccgacaggctagaggacaacggctggaatggatcggatggatcgctcctggcagcggcgatacagattacgcccagaaagtgcagcagcgcgtgaccatcaccagagacaccagcaccgataccgcctacatggaactgagcagcctgagagccgaggacaccgccgtgtactattgtgccgctccttactgtacaggcggcgtgtgtagcgacggcttcgatatttggggccagggcaccacagtgaccgtttcttca

SEQ ID NO: 2087 - DNA, 324 bp, synthetic construct
  source 1..324: mol_type = other DNA
gagatcgtgctgacacagagccccggcacactgtcactttctccaggcgaaagagccacactgagctgcagagccagccagagcgtcagaagcagctacttcgcctggtatcagcagaagcctggacaggcccctcggctgttgatctatggcgcctcttctagagccacaggcatccccgatagattcagcggctctggcagcggcaccgatttcaccctgacaatcagcagactggaacccgaggacttcgccgtgtaccactgtcagcagttcggcaacagcccttggacatttggccagggcaccaaggtggaaatcaaa

SEQ ID NO: 2088 - DNA, 375 bp, synthetic construct
  source 1..375: mol_type = other DNA
caagtgcagctggtggaatctggcggcggacttgtgaaacctggcggctctctgagactgagctgtgccgcttccggcttcaccttcagcgacttcagcatgaactggatccggcaggcccctggcagaggactggaatggatcagctacatcagcgacagcggcagcaccatgaagtacaccgacagcgtgaagggcagattcaccatcagccgggacaacgccaagaagtccctgagcctgcagatgaacagcctgagagatgaggacaccgccgtgtactactgcgccagagatagaagcacctgggagagatacaccacctcttggtgcgtggactcttggggccagggaacactggttacagtgtcctca

SEQ ID NO: 2089 - DNA, 330 bp, synthetic construct
  source 1..330: mol_type = other DNA
cagagcgttctgacacagcctccaagcgttagcgctgcccctggccagaaagtgacaatcgcctgtagcggcagcagcagcaacatcggcaacaacttcgtgacctggtatcagcagctgcccggcacagctcccaaactgctgatctacgacaacaacaagcggcccagcggaatccctgtgcggtttagcggaagcaagagcgccacatctgccagcctgggaatcacaggactgcagacaggcgacgaggccgactactactgtgtgacctgggacgatagcctgagcgtggtggtttttggcggaggcaccaagctgacagtgcta

SEQ ID NO: 2090 - DNA, 12344 bp, synthetic construct
  source 1..12344: mol_type = other DNA
agatctcccgatcccctatggtgcactctcagtacaatctgctctgatgccgcatagttaagccagtatctgctccctgcttgtgtgttggaggtcgctgagtagtgcgcgagcaaaatttaagctacaacaaggcaaggcttgaccgacaattaattgcatgaagaatctgcttagggttaggcgttttgcgctgcttcgcgatgtacgggccagatatacgcgttgacattgattattgactagttattaatagtaatcaattacggggtcattagttcatagcccatatatggagttccgcgttacataacttacggtaaatggcccgcctggctgaccgcccaacgacccccgcccattgacgtcaataatgacgtatgttcccatagtaacgccaatagggactttccattgacgtcaatgggtggagtatttacggtaaactgcccacttggcagtacatcaagtgtatcatatgccaagtacgccccctattgacgtcaatgacggtaaatggcccgcctggcattatgcccagtacatgaccttatgggactttcctacttggcagtacatctacgtattagtcatcgctattaccatggtgatgcggttttggcagtacatcaatgggcgtggatagcggtttgactcacggggatttccaagtctccaccccattgacgtcaatgggagtttgttttggcaccaaaatcaacgggactttccaaaatgtcgtaacaactccgccccattgacgcaaatgggcggtaggcgtgtacggtgggaggtctatataagcagagctctctggctaactagagaacccactgcttactggcttatcgaaattaatacgactcactatagggagacccaagctagcttggtaccgggccgacctcaccatgggatggagctgtatcatcctcttcttggtagcaacagctacaggtaaggggctcacagtagcaggcttgaggtctggacatatatatgggtgacaatgacatccactttgcctttctctccacaggtgtgcattcccagagcgttctgacacagcctccaagcgttagcgctgcccctggccagaaagtgacaatcgcctgtagcggcagcagcagcaacatcggcaacaacttcgtgacctggtatcagcagctgcccggcacagctcccaaactgctgatctacgacaacaacaagcggcccagcggaatccctgtgcggtttagcggaagcaagagcgccacatctgccagcctgggaatcacaggactgcagacaggcgacgaggccgactactactgtgtgacctgggacgatagcctgagcgtggtggtttttggcggaggcaccaagctgacagtgctaggtgagtcgtacgctagcaagcttggacccacgatcctgagcaaggacctctgccctccctgttcagacccttgcttgcctcagcaggtcattacaaccacttcacctctgaccgcaggggcaggggactagatagaatgacctactgagcctcgtctgtctgtctgtctgtctctctgtttgtctgtctgtctctctgtttgtctctctgtctgtctgacaggcgcaggctgggtctctaagccttgttctgttctggcctcctcagtctgggttcttgtcggaacagctttgcccttgggttacctgggttccatctcctggggaattgggaacaaggggtctgagggaggcacctcctgggagactttagaaggacccagtgccctcggggctgatgctcgggaatcacagagctgggacccagagccaggacccagacccagaatgaggtaggaggtggaggggctgccctgggcgtctgggggcgctgccagggactgagccctgagccagcctgagactcaggaaaccccgtcaggagggagaagggagaagcagactctggacaccagaaagccaggggaagggtcacaaaaggagtggatgtgacggaagggcgggctcctgggtctcttcagaacatatccctgtgcccagggggatcagaggggcagagtcacctgcgtgaaagccccactgctatgaccaggtagccgggacgtggggtggatgccagaaaagactccatggaataagagagagcccaggacagcaggcaggctctccgatccccccaggcccttgccccatacacgggctccagaacacacatttgctggaacagcctgagggaccaaaaggccccagtatcccacagagctgaggagccaggccagaaaagtaaccccagagttcgctgtgcaggagagacacagagctctctttatctgtcaggatggcaggaggggacagggtcagggccctgagggtcagatgtcggtgttgggggccaaggcgcagagatctcaggacaggtggtcaggtgtctaaggtaaaacagctccccgtgcagatcaggacatagtggaaaacaccctgacccctctgcctggcatagaccttcagacacagagcccctgaacaagggcaccccaacacctcatcatatactgaggtcaggggctccccaggtggacaccaggactctgaccccctgcccctcatccaccccgcaggtcagcctaaagccgcccctagcgtgaccctgttcccaccctctagcgaggaactgcaggccaacaaggccaccctcgtgtgcctgatcagcgacttctatcctggcgccgtgaccgtggcctggaaggccgatagctctcctgtgaaggccggcgtggaaaccaccacccctagcaagcagagcaacaacaaatacgccgccagcagctacctgagcctgacccccgagcagtggaagtcccacagatcctacagctgccaagtgacccacgagggcagcaccgtggaaaagacagtggcccctaccgagtgcagctgagttctcaaccctcacccccaccacgggagactagagctgcaggatccagacatgataagatacattgatgagtttggacaaaccacaactacaatgcagtgaaaaaaatgctttatttgtgaaatttgtgatgctattgctttatttgtaaccattataagctgcaataaacaagttaacaacaacaattccattcattttatgtttcaggttcagggggaggtgtgggaggttttttaaagcaagtaaaacctctacaaatgtggtatggctgattatgatccggctgcctcgcgcgtttcggtgatgacggtgaaaacctctgacacatgcagctcccggagacggtcacagcttgtctgtaagcggatgccgggagcagacaagcccgtcaggcgtcagcgggtgttggcgggtgtcggggcgcagccatgaggtcgactctagaggatcgatccccgccccggacgaactaaacctgactacgacatctctgccccttcttcgcggggcagtgcatgtaatcccttcagttggttggtacaacttgccaactgggccctgttccacatgtgacacggggggggaccaaacacaaaggggttctctgactgtagttgacatccttataaatggatgtgcacatttgccaacactgagtggctttcatcctggagcagactttgcagtctgtggactgcaacacaacattgcctttatgtgtaactcttggctgaagctcttacaccaatgctgggggacatgtacctcccaggggcccaggaagactacgggaggctacaccaacgtcaatcagaggggcctgtgtagctaccgataagcggaccctcaagagggcattagcaatagtgtttataaggcccccttgttaaccctaaacgggtagcatatgcttcccgggtagtagtatatactatccagactaaccctaattcaatagcatatgttacccaacgggaagcatatgctatcgaattagggttagtaaaagggtcctaaggaacagcgatatctcccaccccatgagctgtcacggttttatttacatggggtcaggattccacgagggtagtgaaccattttagtcacaagggcagtggctgaagatcaaggagcgggcagtgaactctcctgaatcttcgcctgcttcttcattctccttcgtttagctaatagaataactgctgagttgtgaacagtaaggtgtatgtgaggtgctcgaaaacaaggtttcaggtgacgcccccagaataaaatttggacggggggttcagtggtggcattgtgctatgacaccaatataaccctcacaaaccccttgggcaataaatactagtgtaggaatgaaacattctgaatatctttaacaatagaaatccatggggtggggacaagccgtaaagactggatgtccatctcacacgaatttatggctatgggcaacacataatcctagtgcaatatgatactggggttattaagatgtgtcccaggcagggaccaagacaggtgaaccatgttgttacactctatttgtaacaaggggaaagagagtggacgccgacagcagcggactccactggttgtctctaacacccccgaaaattaaacggggctccacgccaatggggcccataaacaaagacaagtggccactcttttttttgaaattgtggagtgggggcacgcgtcagcccccacacgccgccctgcggttttggactgtaaaataagggtgtaataacttggctgattgtaaccccgctaaccactgcggtcaaaccacttgcccacaaaaccactaatggcaccccggggaatacctgcataagtaggtgggcgggccaagataggggcgcgattgctgcgatctggaggacaaattacacacacttgcgcctgagcgccaagcacagggttgttggtcctcatattcacgaggtcgctgagagcacggtgggctaatgttgccatgggtagcatatactacccaaatatctggatagcatatgctatcctaatctatatctgggtagcataggctatcctaatctatatctgggtagcatatgctatcctaatctatatctgggtagtatatgctatcctaatttatatctgggtagcataggctatcctaatctatatctgggtagcatatgctatcctaatctatatctgggtagtatatgctatcctaatctgtatccgggtagcatatgctatcctaatagagattagggtagtatatgctatcctaatttatatctgggtagcatatactacccaaatatctggatagcatatgctatcctaatctatatctgggtagcatatgctatcctaatctatatctgggtagcataggctatcctaatctatatctgggtagcatatgctatcctaatctatatctgggtagtatatgctatcctaatttatatctgggtagcataggctatcctaatctatatctgggtagcatatgctatcctaatctatatctgggtagtatatgctatcctaatctgtatccgggtagcatatgctatcctcatgcatatacagtcagcatatgatacccagtagtagagtgggagtgctatcctttgcatatgccgccacctcccaagggggcgtgaattttcgctgcttgtccttttcctgctggttgctcccattcttaggtgaatttaaggaggccaggctaaagccgtcgcatgtctgattgctcaccaggtaaatgtcgctaatgttttccaacgcgagaaggtgttgagcgcggagctgagtgacgtgacaacatgggtatgcccaattgccccatgttgggaggacgaaaatggtgacaagacagatggccagaaatacaccaacagcacgcatgatgtctactggggatttattctttagtgcgggggaatacacggcttttaatacgattgagggcgtctcctaacaagttacatcactcctgcccttcctcaccctcatctccatcacctccttcatctccgtcatctccgtcatcaccctccgcggcagccccttccaccataggtggaaaccagggaggcaaatctactccatcgtcaaagctgcacacagtcaccctgatattgcaggtaggagcgggctttgtcataacaaggtccttaatcgcatccttcaaaacctcagcaaatatatgagtttgtaaaaagaccatgaaataacagacaatggactcccttagcgggccaggttgtgggccgggtccaggggccattccaaaggggagacgactcaatggtgtaagacgacattgtggaatagcaagggcagttcctcgccttaggttgtaaagggaggtcttactacctccatatacgaacacaccggcgacccaagttccttcgtcggtagtcctttctacgtgactcctagccaggagagctcttaaaccttctgcaatgttctcaaatttcgggttggaacctccttgaccacgatgctttccaaaccaccctccttttttgcgcctgcctccatcaccctgaccccggggtccagtgcttgggccttctcctgggtcatctgcggggccctgctctatcgctcccgggggcacgtcaggctcaccatctgggccaccttcttggtggtattcaaaataatcggcttcccctacagggtggaaaaatggccttctacctggagggggcctgcgcggtggagacccggatgatgatgactgactactgggactcctgggcctcttttctccacgtccacgacctctccccctggctctttcacgacttccccccctggctctttcacgtcctctaccccggcggcctccactacctcctcgaccccggcctccactacctcctcgaccccggcctccactgcctcctcgaccccggcctccacctcctgctcctgcccctcctgctcctgcccctcctcctgctcctgcccctcctgcccctcctgctcctgcccctcctgcccctcctgctcctgcccctcctgcccctcctgctcctgcccctcctgcccctcctcctgctcctgcccctcctgcccctcctcctgctcctgcccctcctgcccctcctgctcctgcccctcctgcccctcctgctcctgcccctcctgcccctcctgctcctgcccctcctgctcctgcccctcctgctcctgcccctcctgctcctgcccctcctgcccctcctgcccctcctcctgctcctgcccctcctgctcctgcccctcctgcccctcctgcccctcctgctcctgcccctcctcctgctcctgcccctcctgcccctcctgcccctcctcctgctcctgcccctcctgcccctcctcctgctcctgcccctcctcctgctcctgcccctcctgcccctcctgcccctcctcctgctcctgcccctcctgcccctcctcctgctcctgcccctcctcctgctcctgcccctcctgcccctcctgcccctcctcctgctcctgcccctcctcctgctcctgcccctcctgcccctcctgcccctcctgcccctcctcctgctcctgcccctcctcctgctcctgcccctcctgctcctgcccctcccgctcctgctcctgctcctgttccaccgtgggtccctttgcagccaatgcaacttggacgtttttggggtctccggacaccatctctatgtcttggccctgatcctgagccgcccggggctcctggtcttccgcctcctcgtcctcgtcctcttccccgtcctcgtccatggttatcaccccctcttctttgaggtccactgccgccggagccttctggtccagatgtgtctcccttctctcctaggccatttccaggtcctgtacctggcccctcgtcagacatgattcacactaaaagagatcaatagacatctttattagacgacgctcagtgaatacagggagtgcagactcctgccccctccaacagcccccccaccctcatccccttcatggtcgctgtcagacagatccaggtctgaaaattccccatcctccgaaccatcctcgtcctcatcaccaattactcgcagcccggaaaactcccgctgaacatcctcaagatttgcgtcctgagcctcaagccaggcctcaaattcctcgtccccctttttgctggacggtagggatggggattctcgggacccctcctcttcctcttcaaggtcaccagacagagatgctactggggcaacggaagaaaagctgggtgcggcctgtgaggatcagcttatcgatgataagctgtcaaacatgagaattcttgaagacgaaagggcctcgtgatacgcctatttttataggttaatgtcatgataataatggtttcttagacgtcaggtggcacttttcggggaaatgtgcgcggaacccctatttgtttatttttctaaatacattcaaatatgtatccgctcatgagacaataaccctgataaatgcttcaataatattgaaaaaggaagagtatgagtattcaacatttccgtgtcgcccttattcccttttttgcggcattttgccttcctgtttttgctcacccagaaacgctggtgaaagtaaaagatgctgaagatcagttgggtgcacgagtgggttacatcgaactggatctcaacagcggtaagatccttgagagttttcgccccgaagaacgttttccaatgatgagcacttttaaagttctgctatgtggcgcggtattatcccgtgttgacgccgggcaagagcaactcggtcgccgcatacactattctcagaatgacttggttgagtactcaccagtcacagaaaagcatcttacggatggcatgacagtaagagaattatgcagtgctgccataaccatgagtgataacactgcggccaacttacttctgacaacgatcggaggaccgaaggagctaaccgcttttttgcacaacatgggggatcatgtaactcgccttgatcgttgggaaccggagctgaatgaagccataccaaacgacgagcgtgacaccacgatgcctgcagcaatggcaacaacgttgcgcaaactattaactggcgaactacttactctagcttcccggcaacaattaatagactggatggaggcggataaagttgcaggaccacttctgcgctcggcccttccggctggctggtttattgctgataaatctggagccggtgagcgtgggtctcgcggtatcattgcagcactggggccagatggtaagccctcccgtatcgtagttatctacacgacggggagtcaggcaactatggatgaacgaaatagacagatcgctgagataggtgcctcactgattaagcattggtaactgtcagaccaagtttactcatatatactttagattgatttaaaacttcatttttaatttaaaaggatctaggtgaagatcctttttgataatctcatgaccaaaatcccttaacgtgagttttcgttccactgagcgtcagaccccgtagaaaagatcaaaggatcttcttgagatcctttttttctgcgcgtaatctgctgcttgcaaacaaaaaaaccaccgctaccagcggtggtttgtttgccggatcaagagctaccaactctttttccgaaggtaactggcttcagcagagcgcagataccaaatactgtccttctagtgtagccgtagttaggccaccacttcaagaactctgtagcaccgcctacatacctcgctctgctaatcctgttaccagtggctgctgccagtggcgataagtcgtgtcttaccgggttggactcaagacgatagttaccggataaggcgcagcggtcgggctgaacggggggttcgtgcacacagcccagcttggagcgaacgacctacaccgaactgagatacctacagcgtgagctatgagaaagcgccacgcttcccgaagggagaaaggcggacaggtatccggtaagcggcagggtcggaacaggagagcgcacgagggagcttccagggggaaacgcctggtatctttatagtcctgtcgggtttcgccacctctgacttgagcgtcgatttttgtgatgctcgtcaggggggcggagcctatggaaaaacgccagcaacgcggcctttttacggttcctggccttttgctggccttgaagctgtccctgatggtcgtcatctacctgcctggacagcatggcctgcaacgcgggcatcccgatgccgccggaagcgagaagaatcataatggggaaggccatccagcctcgcgtcgcgaacgccagcaagacgtagcccagcgcgtcggccccgagatgcgccgcgtgcggctgctggagatggcggacgcgatggatatgttctgccaagggttggtttgcccattcacagttctccgcaagaattgattggctccaattcttggagtggtgaatccgttagcgaggtgccgccctgcttcatccccgtggcccgttgctcgcgtttgctggcggtgtccccggaagaaatatatttgcatgtctttagttctatgatgacacaaaccccgcccagcgtcttgtcattggcgaattcgaacacgcagatgcagtcggggcggcgcggtccgaggtccacttcgcatattaaggtgacgcgtgtggcctcgaacaccgagcgaccctgcagcgacccgcttaacagcgtcaacagcgtgccgcagatcccggggggcaatgagatatgaaaaagcctgaactcaccgcgacgtctgtcgagaagtttctgatcgaaaagttcgacagcgtctccgacctgatgcagctctcggagggcgaagaatctcgtgctttcagcttcgatgtaggagggcgtggatatgtcctgcgggtaaatagctgcgccgatggtttctacaaagatcgttatgtttatcggcactttgcatcggccgcgctcccgattccggaagtgcttgacattggggaattcagcgagagcctgacctattgcatctcccgccgtgcacagggtgtcacgttgcaagacctgcctgaaaccgaactgcccgctgttctgcagccggtcgcggaggccatggatgcgatcgctgcggccgatcttagccagacgagcgggttcggcccattcggaccgcaaggaatcggtcaatacactacatggcgtgatttcatatgcgcgattgctgatccccatgtgtatcactggcaaactgtgatggacgacaccgtcagtgcgtccgtcgcgcaggctctcgatgagctgatgctttgggccgaggactgccccgaagtccggcacctcgtgcacgcggatttcggctccaacaatgtcctgacggacaatggccgcataacagcggtcattgactggagcgaggcgatgttcggggattcccaatacgaggtcgccaacatcttcttctggaggccgtggttggcttgtatggagcagcagacgcgctacttcgagcggaggcatccggagcttgcaggatcgccgcggctccgggcgtatatgctccgcattggtcttgaccaactctatcagagcttggttgacggcaatttcgatgatgcagcttgggcgcagggtcgatgcgacgcaatcgtccgatccggagccgggactgtcgggcgtacacaaatcgcccgcagaagcgcggccgtctggaccgatggctgtgtagaagtactcgccgatagtggaaaccgacgccccagcactcgtccggatcgggagatgggggaggctaactgaaacacggaaggagacaataccggaaggaacccgcgctatgacggcaataaaaagacagaataaaacgcacgggtgttgggtcgtttgttcataaacgcggggttcggtcccagggctggcactctgtcgataccccaccgagaccccattggggccaatacgcccgcgtttcttccttttccccaccccaccccccaagttcgggtgaaggcccagggctcgcagccaacgtcggggcggcaggccctgccatagccactggccccgtgggttagggacggggtcccccatggggaatggtttatggttcgtgggggttattattttgggcgttgcgtggggtcaggtccacgactggactgagcagacagacccatggtttttggatggcctgggcatggaccgcatgtactggcgcgacacgaacaccgggcgtctgtggctgccaaacacccccgacccccaaaaaccaccgcgcggatttctggcgtgccaagctagtcgaccaattctcatgtttgacagcttatcatcgcagatccgggcaacgttgttgccattgctgcaggcgcagaactggtaggtatgga

SEQ ID NO: 2091 - DNA, 381 bp, synthetic construct
  source 1..381: mol_type = other DNA
caagtgcagctggttcagtctggcgccgaagtgaagaaacctggcgcctctgtgaaggtgtcctgcaaggtgtccggctatcccttcaccgagctgagcatgcactgggtccgacaagctccaggcgaaggccttgagtggatgggcagcttcgatcccgaggacggcgataccatgtacagccagaagttccagggcagactgaccatgaccgaggacaccagcatcgacaccgtgtacatggaaatgagcagcctgcggcctgaggacaccgccatctactattgtgccacaggcgtgcggttctgcaccaacgccgtgtgtatgcggtggcactacttcgattcttggggccagggcaccaccgtgacagtttcttca

SEQ ID NO: 2092 - DNA, 330 bp, synthetic construct
  source 1..330: mol_type = other DNA
cagagcgttctgacacagcctccaagcgttagcgctgcccctggccagaaagtgaccatcagctgtagcggcagcagcagcaacatcggcagaaacttcgtgtcctggtatcagcagctgcccggcacagctcctagactgctgatcttcgacaaccagaagcggcccagcggcatccccgatagaatcagcggaagcaagagcggcacaagcgccacactgggaatcacaggacttcagcctggcgacgaggccgattactactgtggcacctgggatacaagcctgagcgcctgggttttcggcggaggcacaaaactgacagtgcta

SEQ ID NO: 2093 - DNA, 393 bp, synthetic construct
  source 1..393: mol_type = other DNA
gaggtggaactgctggaatctggcggaggactggttcagcctggcggaagcctgagactgttttgtgccgccagcggcttcacctttagcacagccgctatgagctgggtccgacaggctcctggaaaaggcctggaatgggtgtccgtgatcgataagagcggcggcaacacctactacgccgactctgtgaagggcagattcacaatcgcccgggacaacagcaagaacaccctgtacctgcagatggacagcctgagagccgaggataccgccgtgtactactgcgccaaggacagaggccccagagactacgatttcagatccggcttcatcaagtactactacggcatggacgtgtggggccagggcacaacagtgacagtttcttca

SEQ ID NO: 2094 - DNA, 321 bp, synthetic construct
  source 1..321: mol_type = other DNA
ggcatccagatgacacagagccctagcagcctgtctgccagcctgggagatagagtgaccatcacctgtcaggccagccaggacatctacaactacctgaactggtatcagcagaagcccggcaaggcccctaagctgcttattcacggcgccagcaatctggaaaccggcgtgccatctacctttagcggcggaggaagcggcacccacttcaccttcaccatcaacagcctgcagcctgaggacgtggccacctactactgtcagcagtacgagaacctgcctctgacctttggcggaggcaccaaggtggaaatcaaa

SEQ ID NO: 2095 - DNA, 17 bp, synthetic construct
  source 1..17: mol_type = other DNA
agggagacccaagctag